European Patent Specification EP 4 182 478 B1, published September 10, 2025. Title: Diagnosi in-vitro della Sclerosi Multipla. Applicant: Università di Cagliari. The sequence listing filed with the application follows.

SEQUENCE LISTING (17 sequences)

SEQ ID NO: 1 - DNA, 7978 bp, Homo sapiens
gtaggagatcagtcagggtggtgggaaaaattgtagaaagatgtaaaccttcttggaaggctggaaggttttacaaaagcttcggaaaaagatttggctgaaggcagccagattgtcttatctggtgcctgaaactttaggttaggtaacaaggggatgtaaagaaactcatctaagtaagttagtttacttagaccatggaacctggcctaaatcatctgcatgcaagactagcggggggtgggggtgggcgcagcacgaccatgtgaattccccacaagtgtgttgactcaagacctttgtcattaaatctatactgaataaatgcccgcagcgcaagcacaggcttgtcagggcctcagccgctgactctttatacaccctcctcagtgtctgtgggcggcccagtcccctagcccactctttcactggcttcctgtgtctgagttcatttgttcatctgttgttcagccagggtctgcgggtcggacccggaaggtagagccctgtgtgaggaatgctgcaacagatcacaacagaacccttgaaaatgaaggtgaaaaaactgcggtcagtaagtcactgttgcctgctctgaatttccaagttcgagggaattgctcaggctagggtttcatcaagggacaacagttatcagctcaacagaaacagtatataaaagtatttaaaaagctgcttaaagctagtggagcctgggtttcacaggctcaattaagggacctaatgcaaactgttgtatcccataacccatggttcctggaagaaggtacactagccatagagctctaggaacaagtggggagaaatcttaaacatcatgcacaaggacaacaggtcccagtaacatctttaacattatgggctttagttagggcagctctggccccgttatacacagaagagcctaaaaaggggagggaggaggaaccatcatctaccttactgcctccttatccctcagccccgctatcaccgggccaaaataacaaagaggaaacggaggttttgcctgagccccctcctccaataaactagaagaaaagacaagggatatgctacagctgggggaccctgtcttaagcaagtggcattagaaggggagctcttagcctgcccagtaatgcaagaacgacaatgcaatcaggtacatgaacccatttcttttaatgcttataaaaagctaagaaaaagcattaaagaaaacagagccgctagcccatttccttacgaaaggaatgactgaagccttggcagacaacttccgtatgaccccatgggactggtcagtgctagctaaaacaattttggaggccagccagtacctcctctagagggcagaatacgatgagttgtgcgaacaacaagccaaccagaacgaggtggccgtgcaagatgtaacagctgctatgctccaggggaggcgtccccatgccgatgtacaacaactaattttgatccccaggcctatgcacaagtgtctttgtgcgctctcggggcttgggacagaatttccaaaagcagagatcaacagggatcttttataaatgttcgacaagggcctcaggagccatttgttgaatttatcaatcgtttaacccaggcaattaagagacaaattagtcacacccaggactgatatcttgttacaattggcttataaaaacgctaatgtggatcgccaacaagcaatgcatgcaatcagaggaaaggcagccacagtcagggaacttacacaagcatgtcaactggtggggactgaaacacacaaagccaaaatattggctatggcattaaggcctcctaaagtgaaaagggagggaaacccaaattgttttctatgtggagaggcaggtcatatgaagagggaatgtcccaataatagagaccaaggtaactcaggaaaagaacccccttctatatgactgcaatgtaaaaaggggaaacattgggcaaatcaatgcaagtccaaatttgataaaaacgacaactccgtaagtaaccaggcgggaaacttcatgaggggctgaccccaggccctgctgcaaactggggcaatgtcagtggctttcctctgtcagatggaaagcccacagtcctctctctcagagcaaccaccactgggagcgcaagactggacttactctgccccgatgaattagtgctaaaagaaggagaagacactaaaagggttgcaaccgggatctggggcccactgcctctgggaacagtgggattagtcctagggcaatctagcctatccagtaaaggaatcaatgtgctcactggggtaactgatagtgattattgaggtgagatactagttatgatggaatgtaaaggtctgcatatttcttcccccgggatcaaagacagctctgttactgcttttaccatactgggtccccaatgcccagaaagggggaaagggacgttttggaagcacaggagccacaaaagtacactggaatcaattaatcactaaccagagacccatgatcaccttaaaaattggaaataagaattttactggcttattggacacacggatggatatttcaaacattaatgatcaaaactagccagaaacttgtccttgggtcactcagaaacaaaaaattgttggcattggggaagcgcacacagccaagcagagcacgtgccccctaacctgttgcgattcagaggtaagaaaggcagttatacaacctcaactcatgcccttccctgttaacctttggggacgggacctattagcccaatgggggggtcactctgcagacctctttctaataatggccacagttattcctcccctacccttgacattgctctctcaaaatcctatttgggtagaatagtgatctttaaagggaaagaaattacaaacagcccgtgaattagttgaggggcaactaaaagccagccatacagaaccatcaaacagcccctggaattcacccattttcgtcattcccaaaaggtctggtaaatggagacttttgcacgacttatgtgctatcaatgctaatttgcaacctatggggccccttcagcaggggctcccctcccccacggccattcgacattggcctataatcgttactgacttaaaagactgcttttatactattcccctagcagaagaggacagagaagaatttgcatttacaataccagcaatcaataatgaaaggccagctccctgattccaatggaaagtgcttccccaaggaatgctgaacagtcctaccatgtgtcagtatcatgtaaatcaggctttctccccagtagaaaagaatttcctaatggcaagattattcattttatggatgatattttactagcagccccaacagagccagtgattttaaggttatataactctgtagcaaagaatacacagttaagaggtttaatcatagcacctgaaaaagtacagatgtcttctccttggaaatatcttggatacagactaatttcttgctaagacctcaaaagcttaaattagatactagcaacttacacaccttaaatgattatcagaaattactaggtgatattaactggctttgccccaccctaggcataactactgataagttacaaaacttgttttctatcttaaaaggcaatgctgccctagactctcctaggtatttaactcctacggcacaaagggaaattgaagaagtagagcaatttatctctcaaaggcaattagatcgcacagatccatgatattcagttcagctgtttgtttttcccactaaacactcccctacagggttaacaagacagatgggcccagagctatgctttctagaatgggttttttgctcacataccgggactaaaacactctctctctatgtccagtgagtcaataaagtcatctattcaggcctcagacaatgcaatcagttgctaggttatgaccctgatatcatcaggattcctttaagtaaaaagcaatttgaagcagtattacccttatctatggacctgcaaacagcactctctgattacacaggccttatagggcatacccttcctgctgacaaactccttcagttcttatctcgtacttctgttgttttgcctactaaaatagttcaatcccccatacctaatgctttaacattgtttactaatggctctggtaaacatggaaaagcggctgtctggtggagatcacataattccctcactcattctggatttactagcactcagagagctgagattggagccttaatattagccttagaaactttctccactcagctcatcgatattgttagtgactctgcttactgtttatttattgcagaactttgagacggccttcattaagaccactctggagcccaccctgtgtgcactttttctccgacttcagcaactgctagatcaatgtatacatcttatttttattacacacattcgggcccacagctcactgcctggcccactggcttatggcaatgatcaagcagacctacaggttatgacatcactgcctgaccaagccacccaattgcaacaatttttccaccaaaacttgagaaacttatctaaacaatttcaacttacccagagactagctaaacaaattaccctacaatgcccagattgccagttcacaggcacatcccctccttcaacaggtgttaaccctagaggactagaacctaatcagttttggcaaacagatgttacacgcatccctgaatttggaaaacgtagatatgtacatgtatccattgataccaattctcatttaattagtactcatgctcttcctggagagtccacccgatatgtcattaaacatcttcttttaacttttgcatttatgggacggcccacagaaattaaaactgataatggtctggcttatgccagctcacaatttcaacaattttgtcacacatggaacatccaacattccacaggcatcccgtataactcccaaggacaggccatagaacgtacccaatccagccttaaaaatatgctcagaaaacaaaaaagggggaatatgaataaggaccctgcaacactactagcacaagccttatttacccttaatttttaaaatttaaataaatttcaatcagctgtagaaaagcactttgctaaaacctctcaagaaataaaacctgcagttttatggaaagacgtaaacagtaatgtatggtatggtccaaatgaattgttaacgtgggggagaggatatgcttgtgttcacaccccctcaggtcctctttgtattccagcataatgcatcgaaccataccatggtgtggctaggacccaacccagtaccagaaataaagaaaataaccctatgggacccatagccccgaacaatgtggcttcatcagacaacacaggccccggacaggatgctcaagaagacaagtcagaagactgagtgaatcctgctctggacacagacaccattcactccagataatctgctccttgttatgctttattattatttatttatttatttattttttttttgagacagagtctcactctgtcaccaagctggagtgcagtggtgcgatctgggctcactgcaacctctgcttgccaggttcaagtgattatcctgcctcagcctcccaagtagctgagaccacaggcacatgccaccatatccagctaatttttgtatttttagtagagatggggtttcaccatgttagccaagatggtctcaaactcttgacctcgtgatccacctgcctcagcctcccaaagtgctgggattaattctctcactctgcctgcaactagtacctgctacactctatttggcccatcctctaaatccgcctttcttctgccctgttacttagacaaatacccgaccttcccagcttctaacaacgtgactgcttggctgagagagattaacataaccccagtggggttccttagtaacagcacacaatgaactgaactgctgagtaacaatataggtcactccttgattggaaaaaaaaaaatgttgattatactcaagtttgtcttatgttatttactaatgctaggatgcaaagctggaatatgagcagttaccaccacgcctgacaaacctactgcacatatctgtactctcctatcaacaaaacctgatgctaaaaacagaaaagggagagatgtaggagatcagtcagggtgatgggaaaaactgtaggaagatgcaaaccttcttggaaggctgtaaggtttttacaaaagcttcggaaaaagatttggctgaaggcagccagattctcttatccggtgcctgacagtttaggttgataaaaagggaatgtaaagaaactgatctagataagtttacttagaccttggaacctggcctttaatcatccacgtgcaggactactggggtgggagggtgggaagggggggagcgcaaccatgtgaactgcccaccagtgtgttgactcaaggcctttgtcattaaatctatactgaataaatgccggcagcgcaggcttgtcagggccgcagctgctgactctttacagcaccctccttggtgtctgtgggtggcctggtcccctagcccgctctttcactggtttctggtgtctgagtgcacttgttcatccatcattcagccagggtctgcgggttggacccagcagttccgtacaggggctgctcccatgtgaggtcccaaagtgggacccaaagtaaggatgacaaaaatgttgagctgagcccccagctgaccctcaatgaatacatggtatgagcaaaacatacaccttctgttgttttaagccactgagatattggggtttttgttcacagcctactcagaataatagtctacaactagttaaaaatcatgctgatgctgtgcatggtggctcacacctataatcccagcactttgggagtctgagacaggaggatcgcttgagcccaggtgttcaagaccagcctgagcaatacagagaccctacctctacaaaaatttaaaaattagttgggtataatggtgtgcctgtagtcccagctactcaggaagctgaggtgggaggaatgcttgagtctgggaggtcgaggatgcagtgagcagtgatcctgacactgcactccagcctgaatgatagagcgagatcctgtctcaaaaaaaaaaaagaaatcatactgaaaatacccaatgttcactctattcattttaagaaattaaaataaatactttaactatggacattaaactctcccatattacttctcttagagatcagaaaaatgaacccacttcccataaaatttatttaaaatagacgagtttattgtcatcccactgaaaagtatatgtaatacaaataaagaaataattctagtttactcaaatatttatcagaactctgacttagcaattataaaaaaatgtgggcaattataaaagcaattataaaagctatttagaatagcatctaaatttcagtggtttttttttttttaaactacattggccctagccccagaagattccagtgcacacattcatcacagagaatatatgtattccagtgcgtatagtcattatagagaatgatgaatataatgagaatatgagcaatgtggaggcagtgggaatgttaggaacctttgctctaactggaagagccacacaaaatcccaactgcactatgtgactctgagccttacctgtaaaatcagaaaaatatgatataccatagttattaagtttaaaaatgtaatatgaattttctggcacacagtagacaatcaaatattatctctgcttcctaagatacggtttgaaatttgtagaaaattgtatgatagcttcaatgccagaagacatgtctttataaaacaggaagagaaagccaaatgggaggctaggctgagatgcaagacaaagacaacgtgaaaaaggaaatgggtg

SEQ ID NO: 2 - DNA, 7374 bp, homo sapiens
tgatgaattcctcttcaaagggtttaactgtgtaacgtccttgttctttgttcagaagcccaacctccttatactctcttgtttctggcctgcaaacaaccctcctgctcttgttgtgccctgacatgctcacacaagtccagacataccttgtactgtaacagacagactgctcctatcccctctttctcttacaaatcatgcgtttatcctattcaaaaaagttttaagtcttagccaactgggatcagtttagattgtacagtccaatcctagccaacaggggaaggacaccgacaggaactgcgttagggataaaaaccccttccctcctttgttcagtgtgctcttgcagtcgtaacagatgcaggcggcacccttctgcaaaagtaaattgccttgctgagaaatcctttgtctcagtgctagtttttctcttgagcacagcttacttgttcccaacaatctgggggcccatccaggattcccattctcctctggggaagggtctccagtcctcactcgtgaggagacaggtcccactgcctcgttgtggtggcctcaagggttagggatcgagacccacctggtgtgacgaataaacccggacgcttagcaacgcgggagaaaaaggcctacaaataccacagtgaccaggtaactctgtgcagagacaaaggttaagaaaaaacacaatggcagtgcagtatttccttggtggtcaggacatcctggaggttgaaagtgtgtgaatgagacgcacaattgagtgtggagtccggatctgtggttccgtggtcacctcatacagcttaggacagcttgcctgtcttgcctgtcgggggatcataccgacccaccaacgctaagggggacctgaaaattcccacaaaggaagcagccagagaaggattaagcagaagcaaaagaatgcaagaaatctcaagtaaggggggttgggcctctaaagaaagagtgcaagaggccaggcgcagtggctcatgcctgtaatcccagcactttgggaggctgaggtaggcagatcacaaggtcaggagttcaagaccagcctggccaacatggtgcaaccccatctctaccaaggaaataaataaataaataaaatacaaaaaattagccaggtgtggtggtgtgtgcctgtagtcccagctacttgggaggctgaggcagaagaatcgcttgaacccaggaggcagaggctgcagtgagcggagatcgtgccattgcactcctgcctgggcaacagagcaagactccaccttaaaaaaaaaaaaagaaaaaaagaaagggtgcaagaaatctctagtaagagaggttgagcctcacaaactcaaaaaaacaccttctccaggatgcgaaataccccaagcaagacaatagaatttcccgggacagccccttaggtctcctgctaaaatactggaaagataatgaaaggactaaaaataagaaaaagcaacaaatgataaaatactgttgttttatttggactaaggaaactatcctcaaaccatcagttttctggctacagtttgggtcaaatgaggattggatttgtcaacttttaatagagtatgtgaataacaagagtcctgtccctcaggaggagatacgctatgccctgtgctgacggcaggggcctgtccacctctaccccctcaaagccagtaagaataagccagaaactacttaccctatagaaactaaggcccccacccctaagcaacccacatgggatcctttagaccatctgcctcagccagatacctctcacctccctccccctcaggcagccgccctggacccttcccccgactcacgttgtgccccctctttataatcctaactcctggaatcattcccagcctcagggccctcccccaggaagacttcggtgcgagacagaacaatgtaaaaaggatattcaaaacttccctttccccaccacttctaaagagttagctccaactctcttccccttaagggaagtgcccctcagaggaggctaaatgctccattaactagctcagaggtccgaaacctacaaagggagctcaaaccactcttaagtgacccttatatagtggctgaccagattaatcaatttctcagaccccagatatatacttgggctgagctaatgtctatcctaggtattcgctttttaggagaagacaggagcatgattcgcagggctgctatgacaatttgggaacgtgagcatcccccaggtcagaacgtcccagcagctgagcaaaaacttgcggccacagatcctcaatgggatagtaacaacgcagcctactggaggaatatgcaagaccttggagaactgataattaaaggaactcaaaaatctgtattccgcatccaaaacattcccaaagctttctatatacaacaagggaaggatgaaggacctacagagttcttagaaaggctcaaggagcaagcgaggatatatgcaggtctaggtttagaagaccctcttgggcaggggatgttaaagctccattttgttaccaatagttggccagacatcacaaaacacgttatagaaaatagagaactggaaagataaatctatagagcagcttttgagagacgctcaaaaggtatatgtacgaaaagacgaggaaaagaaaagcaaaaacaaaaagcaaggatcatgctgtccgccccacaacagaacactcaggggccaaaacctataaagaacttaagcccccactttccaggccatataaaggctataaaacagcacagccaaagaacccaaaagtagagagggaaaagggcaaaacaaatgcttcaagtgtggaaaaataggccactttaaaaaggaatgtcccagatgggaaaaagagaaagaagtcattctactcatgaccttggaggaagaatacggcggtcaagggctccactcttttttttacctcaagtcccaccaagagcccttgataaatttagaggtgggacccaaacctgagcttatcacctttttcattgattcaggagctgctcgctcctcagtttgttatcttccccctggtgtaacttgttcacaggaaaaactttttatttcgggagtaaaagaagaggggtttaaagcaaaaatcttagaagaaacagaaattaaatataaggaccgctcagtaaatattaaacttctgttaatcccggaggcaggaacaaacctatttaggaagagatttaatgctaaaattaaacccagacctctatgttaaccaagaaaaattcctcccctccctaaatttgctcactaccctagataaaggatacatccatccagatgtatggtcaaaagaaggaaatcgaggcaagtaataaaagaaaaaaggcataacgggtactcagtagtaaacggagatatcctcacagaaataaaatcgggaagattacctaataacgggtctgcacctgctctgcgcaaacatgtgagctgtttgcattaaatcaagccttaaaatttctgcaaaaccaggaaggaactatttatacagactccaagtatgcttttggagtggtccacaccttggaaaaatttgaacagagcaaggcctcattaacagtaacttagtccacagggacataataattcaagtattagaaaatctatagttgccagaacaaatagctgttgttcacgtcccaggtatcaaagaaatctttcctttagaagctgagggaataatcttgctgaccaaatagccaagcaagctgcctcttccccaacgggaacccattttccatttaactccttgtctccctcccccagccacagtccccgtcttttcccataacaaacaagaaaagttaaatgaaataggagccaaagaaagctcagaagaaaaacgaatattaccagatgagagggaaatgttgcctaaacctctcataagagggatgttgtctcaactccatcaaggaactcactggggtccccaggctatgtgtgatgccgctctcggagtttatgggtgtatagaaatctatacccttgctaggtaaattgtggatagttgtataatatgcaaaaaaaactaataaatcaacaaataagatgcaagcccttgggggaaaaaactcagggttaacgccattccaaaaaattcaaattcattacactgaaatgcccccagtaggccatgttaactatttattaataatagtagatcatctcacccactgggtagaggccatccctttcccaaacacaacagctaaacatgtagttaaaaccttattaaaacaaattatacctaggtttggaattatagaaaacactgattcagacaatagaacccaattcactgccctcgttattaaagggctcactcaagcactaggaataaaatgggaatatcatacaccaaggcatccaccctcatcaggaaaagtagaaagaatgaaccaaactttaaaaaatcatttaacccaactaattttaaaaacccagctacctcggacaaaatgccttcctattgccctgttcagagtccaaacagccccgcaaaaggacactggcctctctccttatgaaatgctttatggactgccttacttaaactctaatactgacattcccacttttgaaacaaaggatgaatttctcaaaaactatgtatcaggtctgtcttccaccctttcctctcttaggactcaaggccttttagcacaaactgcaccccttgaatttgcaggccatcatcaccagcccagagattacgtcctcgtcagaagttggaaagaagaaaagctcaaacctacttgggaagaaccttatttagtacttctaaaaactgaaacggcagtcaggaccaccaaaaacggttgcactcatcacacccaagtcaaaagagcaccatcctctccagagtcatggactgccgttccaggacccaccccaaccagagtcacgttaaaaaagaaagtttaatctgtctcttccttcttagcttcctttccccagctaccacacatcttattattaatataaccagatctagctcccctcaaaccattacttttaatgcttgtcttgttatgccctgtggggatctccaaagccaaagacagctggcctcttcagaaaagtacctttgcccttccaggataaataaaactgcctacagaactgacttttgcatggactgaggccgatcctataactggtagttctgtgatacttagggagatgtaatctataccaccaagtgtcaaggctggacctcctcaataggttgtacctatctaaagccttacattcactttaccaaaggtacaaccccctccacctgtcaactccaacagtgtaaccctgtgcaaatctctattaatgtccccacctctaccgacaccaagcctaccctaggtcacttctatggcccaggagctaatattcctggaaaggaccccaaaggatcctttgaaatgcacttcattactcctcaacccccttcaccttcttctccttctaaaccctcttccaatcaaacagctgttctttccataccccatgacgaaactatagtaggcactgtaaaggttaaagatttaaaacaaactttagtgcttagaacaggataccaagatgcgaatgcctggctggaatggattaaatattctgctcgcacattaaacaaaattgactgttaggcttgtgcggcaggcaggccagaggcccagatagtccccttcccacttggatggtcttctgactgaccgggcataagctgcatggtaagtctctttcaaaatctcacagcctgggagagagcatgcaagactctctcattgctattcccccaagttaaagaccccgcaggtcagcccccgagggccatctggcctccagcttctgatttaattttacctcgtgtcttctctcatggcaaggggaaagattaacgtccctcggagacctaacagggtgtagtcaaaccaagccttcccaagagcttaccagtcaagctgccttttgtctattctcaagcaaatgtatggtggtactgcggtaaactattaggcactctgctgagaaactggagcggcacgtgagccctagtccaactggccctttcactctggcattccgtcaacataacaggacagaggatcacaaaaaaaaaaaaaaaaaaaaaaaaaaaaaagatgctcctcacgggtcttttgaccctcacatttatgtagctgctactggggtcccacaagaggtaccagataaatttaaaccccgaaaccaaatagctgcaggattcagattcaaatctgcactgttctggtggtcaactataaacaaaaatgtagactggataaattacatttactataatcaacagcggtttgtcaattatgcagacgatgccattaaagggatagctgaacaattaggcccaccagccaaatgccctgggaaaatagaagagcccttaacataatgttagcaaaaaaaggcaaagtctgtgtcaagaccagagtccaatgctgtactttcagccctaacaacacagctcccaatggaacaattatgaaggctttacaaggccttacctccatatcagataagttagccaaaaattccagaataaatgaccccatcacaagtctcatggaaaagtggtttggtgaatggaaagggattatgacttcaatattaacctctcttgcaattgttacaggtgtactcatatgtaggatgctgcatcataccctgtatccatgggttaatgcaaggacttatagaaacagctctcacaaaacctcccctacctctcctcctctatactcaaataggctcttgttcctaggtgatcgagaagaacagcagagccaaatcatgttaaaaaaatgtgaagaggaagaattatcaaaagacaaagggggaaattgccagagatgatgaattcctcttcaaagggtttaactgtgtaacgttcttgctctttgttcagaagcccaacctccttatactcccttgtttctagcctccgaacaaccctcccacgcttgtggcccgacatgccccgtaccgtaatggacagaccactcctaccccctccttctcttacaaatcacgcatttacctattagaaaaagtttaagtcttagccaactggcatcagtttagattgtatggtccaaccctagccaacaggggaaggacacagggacaggaactgcattagggataaaaaccccttccctcctttgctcggtgtactcttgcggttgtaacaggcagcacctttctgcagaagtaaattgccttgctgagaaataatttgtctcaatactggtttttctcttcagcaccgcttacttgttcccaac

SEQ ID NO: 3 - DNA, 5643 bp, Homo sapiens
ggcaaccccctttgggtcccctcccattttatgggagctcttttttcactctattaaatcttgcaactgcacactcttctggtccgtgtttgttacggctcaagctgagctttcactcggcatccaccactgctatttggcgccatcgcagacctgccactgacttccatccctctggatccagcaggctgtctgctgcgctcctgatccagcgaggtgcccgttgcccctcccaattgggctaaaggctcaccattgttcctgcgtggctaagtgcccaggttcattctaatcgagctgaacactagtcgttgggttccacggctctcttccgtgacccacggcttctaatagagctataacactcaccacatagcccaagattccatccttggaatccatgaggccaagaaccccaggtcagagaacaagaggcttgccaccatcttggaagcagcccaccaccatcttgggagctctaagaacaaggagcccccgccacccccggtaacattttagcgaccatgaagggacctccaaagcggtaatattggaccactttagcttactatcctcccttagaattggaggaaaataccaggcacctgtcggctggttaaaaatgattagcatggctgctggacttaagactcacgtgtgaggctgtctgggaaagggctttctaacaacccaacccttctgggttgggagcattgttctgcctggaaccagcttccgctttcaattttcctggggaagccgagggccaactagaggcagaaagctgttgtcccgaactcccagcattagccagttgagatcatggtgcagccagaactctctactcaacagttgcccatgcatgcacccctacctttctttctgacccatacatcctgggtcccaaccacaactttcttgaaagtgtagccccaaaattctctttacctctgaatctacttcctccaatccctgcctcctaggtactaatggttcagactttcatttcctctcccaagtattagagcaagttgtatctccaaagggatctaaggaagctctacactgtgtccttaggcatctaggctatgaacccagggagtcttgtccctggtgtccctcccaatttaggcatatagctctcgacatgggcagttatgtgggacccgttccccaccacccttgccagggccccaagtttgtaaatggctatgaggattgctctcccattgtgtaagatgctctcttcccccaatttctacccagcttacccctctgcaatacaatctccaagtcttagctccttggccagggccttagaactgatgacccagtactttaacaactggaactgggtctacaacaacataacagatcaggatgaaagcgacttgagtaagtcaaggagagaagagacagagagagagaaaagagagggagagagaaaagagagatagaagtagtaaagaaaaaacagtgtgccctattcctttaaaagccagggtaaatttaaaacctataattgataattgaagagcttctccatgaccctataacacttcaatactaccttgttgtcagtgtaaacaagggcattgcctgaaaacactgagaccactgacaaacagtaaccttcctgtcaaaaatccttaacccaggaacccgcggatgacccaaatgcattcaatctgtagcagcaactgctttgctaacagaagaaagtagaaaagtaacttttagaggaaacctcattgtgagcacacctcgccagttcagaattattctaagtcaaaaaagcaaaaaggtagcttactaactcaaaaatcttgaagtatagggatagtcggttaaaaaaaaaacaacataacattaaccactgaaaattcccttaacccagcagatttcctaacaggggatttaaatatcaattaccatacaaaggcccagccagacctagaaggaactcccttcaggacaggacaatagatggttcctcccaggtgattgagggaaaaaaaaaaacacaatgggtattcagtaattgatagggagactcttgtggaaacagagttaggaaaattgcctaataattgatctgctcaaactgggagctgtttgcactcagccaagccttaaagtacttacagaatcaaaaaaaaaaattctatctcaatcctgactcaaaaggttacctacaccctctgaaatgaatttccataagaactgttgtttataggaatgcatcttaatggggcagctgggttgttatgaaatactcaggaacccagcccagctttaggactcacccctgagcacaaaggcaatgttgggcacgctggtaaaggaccactagaatccagcagcctggacccctttctttgtggtcaagaaaggcaggaaaacaggtgcaggactgctacattggtgagcgtaactactccaataagcagaagtccatgggtgattacgcacactggaaaggaataagcattaggaccatagaggatgctctaggactaatgctcattggaaaatgactaggggtgctgacatccctatgtttttttttttctcagatgggaaacgttccccacaaggcaaaaacgcccctaagatgtattctggagaattcggcccagtcagagtgtatgtacctttttccctgtcagactcgaagcaaattaaaatagacctaggtaaattatcagataaccctgatggctatattgatgtttaacaagggttaggacaatcctttgatctgacatggagagatataacgttactgctagatcagacactaaccccaaatgacagaagtgccatcataactgcagccctagagtttggagatctctggtatctcagtcaggtcaatgatagggtgacaatagaggaaagagaacaattccccacagaccagcaggcagttcccagcatagaccctcactgggacgcagaatcagaacatggagattggtgccgcagacatttactaacttgtgtgctagaaggactaaggaaaactaggaaggagcctataaattattcaatgatatccactataacacagggaaaggaagaaaatcctactgcctttctggagagactaagggaggcatcgaggaagcatacctccctgtcacctgactctattgaaggccaactaatcttaaaggataagtttatcactcagtcagctgcagacattagaaaaaaaaaaacttcaaaagtccgctttaggcctggagcaaaacttagaaaccctattgaacttggcaaccttggttttttataatagagatcaggaggagcaggcagaacaggacaaacgagataagaaaaaggccactgctttagtcatgaccctcaggcaagcggactttggaggctctggaacacggaacagctgggcaaatgaaatgcctaatagggcttgcttccagtgcggtcgatgaggacactttaaaaaagattgtctgaatagaaataagccaccccctcatccatgccccttatgtcaagggaatcactggaaggcccactgccccaggggatgaaggtcctctgaatcagaagccactaaccagatgatccagcagcaggactgagggggcctggggcaggtgccagcccatgccatcaccctcacagagccccgggtatgcctgaccattgaaagctaggaggttaactgtctcctggacactggcacggccttctcagtcttactcttctgtcctggacaactgtcttccagatctgtcgctatccgaggggtcctaggacaggcagtcactaggtacttctcccagctgccaagctgtgactggggacctttactcttttcacatgcctttctaattatgcctgaaagccccactcctttcttagggagagacatcctagcaaaagcaagggccattatacactagaattaggagaaggaaaatgggtaaatatatatacagactctaagtatgcttacctagtcctccatgctcacgcagcaatatggagagaaagggaattcctaacttctgaaggaacacctatcaaacatcaggaagccattaggagattattattggctgtacagaaacctaaagaggtggcagtcttacactgccggggtcatcagaaaagaaaggaaagggaaatagaagggaaccgccaagtggatattgaagccgaaagagccacaaggcgggaccctccattagaaatgcttatagaagtatccctagtatggggtagtcccctctgggaaaccaagccccactactcagcaggagaaatagatgggtttcactcgcatccacctctgtgggaagagaccaccaaacaggcttggtgtgagcaacaaggctatttatttcacctgggtgcaggcgggctgaatccgaaaagagagtcagcgaagggagatggggtggggccgttttataagatttgggtaggtaaaggaaaattacagtcaaaggggggttgttctccggcgggcaggggtgggggtcacaaggtgctcagtgggggagcttttgagccaggatgagccaggagaaggaatttcacaaggtaatgtcatcagttaaggcagagacaggccattttcacttcttttgtggtggaatgtcatcagttaaggcaggaacaggccattttcacttctgtgattcttcacttgcttcaggccatttggatgtatacgtgcaggtcacaggagatacgatggcttagcttgggctcagaggcctgacaatggggaacctcatgaggacatagtttcctcccctcaggatggttagccaccaaagaaggaaaaatacttttgcctgcagctaaccaatggaaattacttaaaactcttcaccaaacctttcacttaggcattgatagcactcatcagatggctgaatctttatttactggaccaggccttttcaaaactaacaagcagatagtcagggcctgtgaagtgtgccaaagaaataatcccctgcactgcaggccatacatttcaatccctgtatctttttaacctccttgttaagtttgtctcttccagaatcgaagctgtaaaactacaaatcgttcttcaaatggagccccaggtgcagtcgaggactaagatctaccgcagccccctggaccagcctgctagcccatgcttcgatgttgatgacatcaaaggcacccctcccgaggaaatctcaactgcatgacccctactgcgccctagttcagaaggaagcagttagagcagtcgctggcccgcctccccaacagcacttgggttttcctgttgagaggagggactgagagacaggactagctgcgtttcctaggccggctaagaatccctaagcctagctgggaaggtgactgtatccacctttaaacacagggcttgcaacttagctcacacccgaccaatcaggtagtaaagagagctcactaaaatgctaattaggcaaaaacaggaggtaaagaaatagctaatatctatcacctgagagtacagggggagggacaatgattgggatagaaacccaggcattcgagccggcaacggcaaccccctttgggtctccttccattttatgggagctctgttttcactctattaaatcttgcacctgc

SEQ ID NO: 4 - DNA, 8995 bp, Homo sapiens
tgagaaaacattttaaatggtccattttcaagtcataataaacctaaggactggcagccagcctgcggatgtaacaaactgcacagctcatgcacctagaaggtcatgataagtgaacagactgtagaagaggggtcagcccataaaaggaaagaaagtttcgttattgggaaatcgaaacttaagtggggaaggggacgaggatataaccttctaagggtgataataaaacttacacatctgggaagattgtaactccacagtactcaaccaatgaagaactgggggagggacttgtgtgctaggagataaattgcctgtcgtaactgccccaggtgtgcctgcctaccacacacgggatggtgtctccaagtccattttttgggtttgcatgggtgaatgtgtgtttctcacaaacctgggggcccaaccaggatctctgtgcctgcatggagtggaactccggtcaagggggagacacatcccatcaatttaggtggcctgctctgtctgggtattccagcacccggcagaggccatagacaaacccaagactgttattccagaggcagcagagacaacacagggagaaaagcacacactgcagcaaccaggcaaccttgtgcaggagcccaggtaggaaaattagactgtaagtactgccttagtggttgggcattttcagaggtcaagtgtgtgcaactgagatgtatcttagatatgaagcaagtgcggagtcccaatccacggttccgttctcctgcgacgcaaacagccagagacggacaaaccgatgctcagggtgtgcaagaaacctctagtagcgcgggtcgagtacacagggaagaaagctcagacatagaggctgatcaaaaatgggaaacagaaatcctaaacctagggtacaaagcaaagagggagccaaagagactccctctgacattcccccagatagtcctttggggagaatgctgaaggtttgaagggacaacccttgaaccaggcaaaaggaaaagcaaaagataaggcatcgctgttttatctggcccaaagaccctattcataagccttcgatcttttttggcctaagtttggctcagatgaggattgggtgtgccaagctttaattctctatgtaaatgataaaactccatcctcacaagaagaggtaggttacactctgctggatcaaaaaattagctcccatgttccccctcaaagaagaagaaaaagaacctaataaaaagccctcacccagtgaaaggccctggaaccacctatcacgcatgccccctccatacatctcacaaaatagtggacaggaaaatcaaggggcagcaggagggttagaggaagatagacctggagaccacaggagagccaaaccaactgctcctttaaatccttatccaaatttaagaaaagaattagaacagtgtaagagggatactgagaacttccctatcccttccacacagcaggcatctagcaatgttccctcttagggaagctcccatgggacacagagatattggctttgtaaatgctcctcttacaagtactgaagttaagaatttcaagaaggaaatgaaatcactcctagaggatgccctcagtttagcagtccagctggaccaattcgtaggacccagcttttacacctgggctgaaatgatatctatcatgaatagcctattcacaggagaagaaaggggaatgattaagagagcagccatgaccatctgggagaggcaacaccctcctgggcaagaagtcttgccagctgaacaaaaatctccaaacgttgaccccaaatgggataataataatcccagggaccaagcccaaatgcaggacctcagagaataattaaagggatcaaagagtccactcctaggacacaaaatgtcttaaaggcattcgagattcaacaagaaaaagagaaaattccctccgcattcctgtagaggctcaaaaatcacatgagaaaattagatccggaggacccagtagggcaaggccttttgaaggctaactttgtaacatagagctggcctgacattacaaaaaaattagacaagattgatggatagaataaaaaactgattaaggaattattcagggaagctcagaaggtctttgtaaggacagaggaagagaagcaaaaacaaaaagcaaaaatcatggtttccactgtggaagaggtagtcagaaaaacgttaaatcaaaatccccctcaaaggagagaagggaatgatagattctgacatagagaaagaagggaaacgcaggaaaaagctcctaagagtggatgttacgagtgtggaaagccagggcattttaagagaatgtcctgaatagaaaaaagaagaccccaatagcaaagacttggaaccaacccaaatgtccaacaatgatagaatggattaagaacaccatggaatactatgcagccataaaaaaggatgagttcatgtcctttgcagggacatggatgaagctggaaaccatcattctgagcaaactatcgccaaggacagaaaactaaacactgcatgttctcactcataggtgggaactgaacaatgagaacacctggacacagggtggggaacatcacataccagggcctgtcgtggggtaggaggaggcgggggatagcattaggagatatcctaatgtaaatgaccggttagtgggtgcagcacaccaacatggcacatgtatacatatgtaacaaacctgcatgttgtgcacatgtaccctagaacttaaagtataaatcaaaaaaaaaaagaggaagaaaaggtaatccccctcatgaccattaatgaagactattggggtcagaggttccttctgagtaggtcccactaggaacccttgataaatttgaaggtgggacctgaggaaaaagaagggacatttttggttgatactggggcggcttgctcctccctaattcaccaaggggtactgaaccaaggaaaaattgacagtatcagggattaaaagggagagatttcaggttccaatattcaagaaaatgttaattagattgggaccagaacgaactgagaggtcactcttatatgttcccaaagcagaaactaacctcctgggtggagacctgattgtgagattgggtttagaattaggaatacaggcagaacaattaaaagtcataatgggcctcctaataaaggaggaagaaagacaaaataatccctatgtgtcgattagaaaaaggcaacagcagagggttaaaaatcacacccttacagactgaactaaaacaaccaggagaactagtttgcagaaaacaatatcccatttctactgaagggagaaaaaggctccaaccagtaatagaggaattaattaaagatggactattagaaccctgcatgtcaccatacaatactccaattctcccagtcaaaaagcctgatgggtcgtatagattggtgcaaaatctaaggactataaatcaaattgtccagacctgccaccctgtggtgcccaacccctacaccctccttagtaagataccctatgaacataagtggttcagtgtggtagatctaaaagatgcattctgggcatgtcccctagaccttaggagcagggacctctttgcctttgaatgggaaaatcctacaactgggagaaaacaacaataccactgtactgtgctgcaagaaggcttcacggaagccccaaacttatttggtcaagtcttagaaaaagtcctggaggaattccaaccttccagggaaacccagttgttacaatatgtaaatgatcttttaatttctggggagaggagagccaaggtatcagaaaccactataataatttcctaggagagaggggattgcaagtctctaaaaacaaactgcagtctgtagaaaaagaagttaaatatttaggacacctgattagtgaaggaaagagaataaacccagagagaatatcaggaatagaggggtctaccttttcctaagaccaagagagaactctgaaaatttttaggtttaactggctgttgtaggttatagattaagtcatatgctcaaaagacaaagattgtgtatctgaaactactagaggaggaacctgattccttgcaatggtccccagaagaaattcaggcagtgaaagaactaaaacaggccctcattacagccccggccctagtcctcccatctttagagaaaccattccatctgtttgtaacagtagaccagggcatgccccttgcggtgctcactcaaacctggggagggaagaggcaacatattgcttttgtctccaagcttcttgatcctgtctctctcgggtggcccgaatgtgtacaagcagtagctgccacagccctgctggtagaggagagtcgaaagctatcctttggtggggccctaatagtaagcaccccacaccaggtcaggaatatattaaatcaaaaagccgggagatggttactggattctcagattctaaaatatgaagccatattactagaaaaaaaagatttggtcgtaacaacaaatacttgcctgaatccagccagtttcctatacaaaggagagaacaaagagccatcagaccataactgcttagatatcactgaatacaaaatcaaagctaaacctgaccttagggaagctccacaacatgatgggataaggctgtttgtggatgggttgtcccaagtggatagatggcaaagagagataatggttatgctatcactgatggaaataaacactccttatgtgagaaaggtagattacctaatggttggttggcccaaacctgtgaattatatgcttttaaccaggcgctaaagctccttgaaggccaagaaggcactatattcactaattctaaatatgcctatggggtggtacacacttttggaaaaatctggacagtgcagggcctaataaatagcaggggaaaagaattggtacatggggaactggtcaaacaggttttagaaagcctccagcttccagcagaggttgccatagttcgcataaatggtcatcagaaaggtaacactatagaagctgtaggaaacaagcttgcagataaagctgctatgcaagcctccctggaggaagaaattagactatttagcctgatcccagacatccctaaggtagtattaaggccccagtttaccagaaaggagaaggaagaattaggataggggtcacacaaactgaaaacgggaagtgggtacttcctgatgggagagaaataagtaaacccctgatgagagaactaacgtctgtattacacaaagggagtcaatggggaccccaggctctgtgtaatacaatacataggaatgatgagtgtatagggagttacacttttgctaaacaagtacgtggaagctgtgtaacttgtcaaaggataaacaaaaaggtgattagaaaacaggccacaggaggaagacctcccagactaagaccatttcaaagcattcaaataaatttcacagaaatgcccaaagtaggaaaactaaagtatttactggtgatcagagatcacctttctggctaggtggaagtctttccactcccaacagccactgctgggaatgtggtcaaaataaaattagaacagaatgtacctagatttggcctggtggaaaatattaattcagacaatgggagccactttacctcaagggtattaaggggaattatggaaggtttacaaattagatgggattatcacactccttggtatcccccttcctctagaaaagtagaaagaatgaatcaaactctcaaaaagcatatcaccaaactaatcttagaaactaaaatgccttgaatgaaatgtctcccaatagcactcctcagaattaggacagccccaagaaaagacttgggattgtccccctacgagttattatatgggctcccatatttgggcagagctacagatcttcctactttggaaaccaaggatcaattcttaagaaattatatactggccatatcctctaccctgtcatcccttaggttaaaaggacttctgactcaaactcttcctcttgagttcacagttcaccatttccaccctggtgacttggtgctgattaagacttgttaagaagacaagctccacccaacctgagaaggtccctatgaagtgctcctgaccactaagatggccgtgcaaacggctgaacaggggtggactcactgtactcaagtcaagggactggtaaaagagacctcggaagggaaggaacaagaccagtggaaagtgcatggatcacctgtgctacgggaggacctcaggcacaggtggttccatttcccctaggatgggatactgatcctgaagaagtggattgcacgttggctctataccaggacaaggatgcatggggaaacaagacttataagagtctgtcactgctctttcccacattgcagaggttaactttaagtaacccttaaagttaactctgagaaaaatctaaaaagaaaacatgggctggccccatttctggaagttaatatggctgagatggcctactacgcaaagagcagaaggtcaaaatggaaacttgcaggcaactcctccctacccaatcaggtttgtaatctatgtaaccaagatggtagcaccccagactataagattcgatgcctgccaggtctcaccttgtgggaattttgaaactcagagatagttctcacaagtgaataaacatctttgccctgaaccagatacagattacagtatggcattaccatgccccagctgggatgatgtatggtgaaccacccaattcagggttggacagtaaacacggggtgggtaactccgagctgaagacacttaaagaataaactacatctgtccaagggctccttgccaaataactgccaaaatttagaacgcaaccctatactcattgccattagcaatccagccactctaggccaagaaccaaaagtagtgtctcaggtatatacgtgaggggcagacatcacagggaaagaccccatagggtgatttgttctcaaactaataaaaaactcaacctctcatttgcctggaactactccaactccagaccctaataaacactttagtctgccaaataataaccctaaaaggtaaaaataattgaggtaaaggatttaaggcaaaccttagaaattgagacagggtgcagggatgtaaacgcctgggtcaaatggatcaaattttcggtacaagccttcaacaagagtgactgctatgcgtgtgctacgggaggacctcaggcacaggtggttccatttcccctaggatgggatactgatcctgaagaaatggattgcatgttggctctataccaggacaaggacgcatggggaaacaagacttgtaaagagtctgtcactgctctttcccacattgcagaggtcagatcccaaagcaatcccctcattctctctagggaatatgaaccactcctcttgcctctctagatagggggcagagttcaataagcccgtgggaaaactctcaacttgtacgcacatcctaaacatcactggtaagtcaggcgatggcaatcactcggctctccatataccccaggctaacgtctggtggtactatgggaaaaggaacctccccaacttgttaccatccaactggaccgggacttgtgctttagtctaattggccattcccttcaccctggcattccataagatacctgaaaacacacacggccactgaaagcagagagatttgacaaactcttttaatgtcaatatatatgttgactcaataggagtccctaggggagtgccgaataaatttaaggcccaaaaccaaatagctgctgggtttgagtcagcactcttctgtggtcaactattaataagaatgtgaactagattaactacatctattataatcaacaaagattcatcaattatactcaggacaccctcaaagggatggctagccagttagatgccaccagcccaatggcctggaaaaacaggcttgcactagacgtaataccagaaaaagggggtgtaagtgttatgctgggtgggaaacgttatactttcattcccaacaatactgccccagatgggaccatcacaaaagctttacaaggactgacaactctagccaacgaacaggcagaaaatgctggaattaacaacccatttacgggttggctaaatggttggtttggaaaatggaaaggcatggtggcttcaatccttacatctctcataattgtagcaggagtcttagcagtgggatgtagtattacttgtgtgtgaggggactagcacagagattaattaaaacagctattaataaacaatgccaataagttaccagcaaaataacctgctactattagaaaccaaaataaactcactctcctataaggaagaaagtaaatgacttctaaagcaatttgaggaccaaaagggtttagatgaaaatgagaccaaaggaagtaaatagaaaaggaaggaaatttgtgagaaaacattttaagtggtccattttcgaggcataataaatctaagtactggaagccagcctgtggatgtaataaaccacacagctcatgcacccagaaggtcatgataagtgaacagaatgtagaggaggggtcagcccctaaaaggggagaaagtttcattattgggaaatcgaaactgaagtggggaaagggaccacggtataaccttataagggggataataaaacttaggcaatgtccaggaagattgtaaccccatagtactcaaccaatgaggagctgggggagggacttgcgtgctaggagataaattacctgttgtaactgtccccggtgtgactgcctaccagacaccagatcttgcaagaccgccaataaaagtcttgcttccgctgttcttcatgtctccaagtccattctttgggtttggatgagtaaatgagtgtttctcac

SEQ ID NO: 5 - DNA, 9140 bp, Homo sapiens
tgagcagggcaggagagggcccccagctcaggaatgtcaggcgaccatcaggtgatgatcaggcggttgttacactgtttctctaaaataataataatgggttgcagccagtaccagggaaagacagtctcccaaaagacaggaaacaccggaagctggtgatcagcaacttcctgataagatctccgaagctgggcaagtgggctcaagcatgcgcactaagaagcaaaatgacagtttaaccagtatgtgaccttcctctaggaacacctgactgataagggaaaaatgtctcaagaaagcatgcgcacaacttcagtaaacaaatgcacatgtggctcctcccaagtgctgacaggccactgcacagcagacagcccaccccaaggaaaaaaatccaaggaggagaaatggaaaccccggaaccatgccgatgtataaaaccccaagtcaagggctgaacagggcacttggatctctcaaatggtgcagtgactcggataccttccctagtggtaagacacctctacgccttgccttcttcggctggaggcgttcaaccctcgtacgtggtttcgttctcctctttcactctcctgcttactaacctacccctggaacgattcctctcaaccacagtggctctgctccccctggctgctctctctgctcaccccgaaggatggcttgcaggggtgggaaggaccttggagtctgcactaagtagacctgagacactaatggcccccccagacaggaggctgatgagagcggtagggctaaaacctacaaccatgtagtatctggggtttcctctgctttttcaactaaaatcagctctttcccaaaaacccaccaccacctattttcctttctctgtatgtattccaaaatgacctcgcacacccattggaccaactgccttgggggtaagtctgtcttttctctgttcttactttgcatgccctgcaactttcttctctgccttaaacacacattccctatttgttattcatgcacccgcagctcttgctgtgttagcctggcaaccaagagatggactcccttacggatgtcccttgatatttatacttgttaccctaccagctcggatgacctccaaccctttccctgtctgttggctcactgccgggatagacactaatcagaaccttagctctgtcagctccttatgacttaccatatgcttttcatccctgttatgctccagggccatgtttctccctggcttttgaatggtttgcttgcttgcataggacctcactctgtagcccttaaggaccccacccactcgctttttttctgagttagcacccctttgtggggaaggaaaattctctgccgtttgcagggtcttatcccaaacaccaagtcctccagaggttcctcctttatatcaagagggcaaataaacgttgccctctcaaatccaagggctgctgtttctgcaaacatatgaaggctttccatgagtattcctcttgcttcctcccgctttctcctgtagcagagggattgttctacctcgttaagcatttgttctgcatgttaccctgggaggatgaagaatcccaaatacaaattttcctccattcctctaatcacctccaggcccttctcaatatgtatcaggaccttcaaagttatatttgaagggagagaagtccagcccccttgcagcaattggcagaaaaacaggcttctcgtcttcttaaagaacatgggaaatgagaatctgagaagagataatcattctgttgctagaatgctctgaacaagggtcactataaggtcatggagacaaggatataggacagcccaaggaggcagatgcaagagaccaaagtacccatagaacagagatgaagactagttccaggctacaaacacaaaacagattaccactgcaacacagatgaaggctggtccagaaatgggatgggatcagggtaggggtacccagtaaacactgggttcattccagaaccccttggatgagtgggagggcaccctgttcactgtagtctgccataggcacaggattaagagaacaaggggagatgccctcttctcgcctctgttctttctttacaaacgggtaattgtgcctcaataaaacaagatgggaccaaggttaggggtacctggtaagcactggttcattctggaacccctagaatgaatgggggacactgccatacgcaaaggaaaaatggatgaatggggtaatgccctacccactctggtctgctgtaagttcaggaaaaagacagtagggaaattggaggggttgccttctttttctcttctctcctctgttctctctgtggacaggtaatcaagtctctgtaccacaggacacactactaggatacatcctcaagaactgggaaaagtttgactcccaaaccctaaaaaggaaaaggctaatatttttctgtaatacagcctgggttgaataaaagctctaggaccaggaatcttggccagaaaatagaagcacaaatttaaatatgatccatcaactagatttgttttgctaccaccagggaaaatggacagaaatcccctatgtgctggccttcatggccctaagaaacaaccctgacctttgttgggcttgtaaaacagatccatggccatagtcatgcagccccttcccattggttcagaaggcccctcatcaggtttacccagagctcaagccccattgccccttctacccaattatatcgaagtctcccagaagccttctcctccctacccagggccatcctctggacaccacctccttaagttatgccccattcaggaggtttagtggtcccagtggacccactggagtccagactccattcactgtgcaagacctgagccaaattaaaatggaactagggaagtttatggaggaccctgacaaatatatcaaagtgttttataaactgggcttaacatctgaactcaccaggagggacctctcagtcatactagggcaaactctgcctaagggagaatgtgactccattatggtggcggtccaacaatttgcaaacacaatgcacatgcctgacactggtggctaccctgtgggggccaccatagttccccaggtcaaccccaattgggattacaatatccaggggagtacatgagcaaggacccacatgttcctctatctgatagaaggaatgaaagctagcagagcaaagcctgtgaactgtaataaattgggcttgacagatcaagggccttatgaaaacctcaccattttcttagacaggctagaagaggccctagtgaaacacactaacctagacccagacccactagaaggacaactgttcataaaggatcatttccctaactcaaacaacaccagatattaggaggaaacaccagaaactagcactggatcccagtacccctatgcctgacatctgcaaagtaggttccttggtcttttacaaccaaaaccaggaggagtaggaaagggctcaagaaaaggagaggcaaaaggaaaagcaacagctccaactactgactgccctgcaaacctgccagccacctctggcaggccccagggagatccctttgcccaaatgctacttctgtggggagccaggccacacaagaaggcagtgcccaaactgatggggacacccacccccagctctccatgctccaattgccacaatcttggccactgggaaacaggactaccctgaaagctgaaaggccctcaggacatcccaactggatgaccttcagctccttgagctgaagggggccctacgctccacttggctcctggattaaataacactattgaagggacagagccaagggctgccttggatgtgcccagtaggactgtaagttttcttttggacatgagggctgcctgctcaatgcttacctcttttcccaggcaattatcctcctgggaggatatgaagtgcccgtaacctggaggtttactcctcctctgtgctgtctctgggggaaaaccgtcttttctcattcatttttagtgatgccagaataccctacataccttttgggtagagatattttgctcagactaggggctcagttaacctttcctccagggccaacaccccctttttcaaatgcaatcttatgcctcaaggaaaccatacacaaggatgaactgttcacagaccttcccatttatccagaggtctgggcctcaggaataacaggaaaggccataatggcaatgcctatagtaattcagcccaagaatccttctagctatccttgtagaaggcagtttcctcttcagctggaggccaaagagggatttcagcttctgactgaaaaatttcaaaaacatggattattaataccctataacaccccatcttacctgttaaaaagagcaatgaaaaatacaggctagtccaggacctgagaatcataaatgaggcagtagtcccaatacacccaatgatccccaactcatatgtaattcttccccaacctccagatgctcagtggtttccagtcttagaccttaaagactctttcttttgtatctccccctcgacccatcctcccaatttctatttgcatttgagtgggagaatgaaaaggaaggagtcaacagctcacctgcacagtgcttcaacagggtttcagagacagtccccattggtctgggcaagccctggctagagatttgcaggacctaagtcttgagaggagagagtgtctcctacaatacatggatgacctgttaatctgctccccaacaagagaactgggaatccaacatctagtccaaacaccaaacttccttgcagacagagaatacaacgtgtctgaaaacagactcctaaagtaccaagtcttgttgttagaaaacccataggtaacagttgagcagtgttccacccttaactcagtttccttactgccactaccaggagaccataacaccacatttgtgttgtgagatacttaaccaaatttatgccagccaggaagatttaaaagatcagctcctagataatccacatgacatacggttttcaggtgggaatagctttgtcagggatagagctagatatgcagagtatggtacaatgtcccttcaacaaattacagaggttaaagctctgtccccggggacctctgtgcaattagccaaactcactgtgctgacgaaagccctaaactaggggaaagaaaaggagtatatacaaattccaaatacacgtttctggttcttcacactcacacagctatctggaaggagagggtgtacctaacagctccagatactcaaattaaatatgggcctcaaatcttagagctattagaagctgttcatttgccccaggaggtgacaatagtgcacagtaaaggacaccaaaggggctctaatgaaactgcatagggaaataggttagctaactaaacagctaaagagacaggcatctcaaaagataccttcatgggggccttgctcatctctctccccagtgaactgctctctctccaatacattaaggaagaaacagattgggccacccaacatgggtattgaaaagaaaccaatggatgatataggttgggagaacttctccgtctacctaaagcctaccaatggaaaccatcaagagtttacaggactcccgccactttagaagagacagtctaaggcaaatttgtaaaccagtgttcagtgggggagggactaaataaaactattcaacaggtttgtcaagcctgcactttgtgcactataaataatccccagacggggaagccctctccatcagtaagtccaatccaaaggagaggtacataccctgcggaggactggcagatggacttcactcagctccctgcataccacaggtttaagtacctcgtggtctgtgtagacaccttcacaggatgggtagaagcctgcctcacaaggactgaaaaggcacaggaggtagctaaattcctcctaaaggaactcattcctcagttcagccaacccaggtcattgcagaatgacaatggtccatccttcatttcccaattaactcaacaggttagtagtgccctggacataaagcttcactctgccaggagactgtaatcttcaggaaaagtggaaataaccaaaccctcaaacacatccccaacaaactctgccaggaaacagcacagccatgggtgtacctcttagctttagccctccttctgatttgctgcccctaaggctcccttgcaattaagccccttcaaggctttatatggtaggccattcctatattctgtcattactagatgaagaaactgctaaaatcacccactatgtttcttctttagcaggcttctaacaggctctctgggaatatggtttacaaacaaacctgaaatctgaaggggaaaaatccccacctctataccccataggctcacaacttctcattaacgcctggaaggatggaaccccaaattcccaacaaactcctatttgaaagggccccttcaccattctattatctacccctacagccattacagtactggagactgccagctagatccatcacacccaagtgaagctgtggaaaagcccttaaactccagagccagaaccagcaacctcagctccggaatacacttgcaaggcactggaagatctaaaattcctctttaaacaaaaagataagtaatgccccaccaacatcctttcacctcaaagtaaggtgatcccaatactagaaattttactggcaattgctctgattgttatcactattttaaccctaacttgtacaccaccaggagttccattggcagctcgttttgtgaccagtttctcttaggtcaccatgggcctgctcctgctggttctcattctcacgccttcactagcagcctaccgccatcctgatttcccgttattggaaaaagctcagcaactgctccaaagtacaggatccccttactccaccaattgctggttatgtactagctcttccactgaaacaccagggacagcttatccagcctcgcccagagaatggacaagcatagaggcggaattacatatttcctatcgatgggaccctaatctgaaaggactgatgaggcctgcaaatagtcttctttcaacagtaaagcaagatttccctgatatccgccagaaacctcccattttcggacccatctttactaatatcaacctaatgggaatagcccctatttgtgttatggccaaaaggaaaaatggaacaaatgtaggcactcttccaagtacagtctgtaatgttactttcactgtagattctaaccaacagacttaccaaacatacacccacaaccaattccgccatcaaccaagattccccaaacctccaaatattacttttcctcagggaactttgctagataaatccagccggttttgccagggacgcccaagctcatgcagtactcgaaacttctggttccggcctgctgattataaccaatgtctgcaaatttccaacctcagctctacagcggaatgggttctattggaccaaactcgaaattctcttttttgggaaaataaaaccaagggagctaaccagagccaaacaccctgcgtccaagtcttagcaggcatgactatagccaccagctacctgggcatatcagcagtctcagaattttttggaacctccctcacccccttatttcatttccatatctctacatgccttaaaactcaaggagccttttatatttgtggccagtcgattcaccaatgcctccccagtaactggactggaacttgtaccataggctatgtaaccccagacatcttcatagcccctggcaatctctctcttccaataccaatctatgggaattccccgttgcccagggtgaggagggcaatccatttcattccccttctcgcgggactcggcattctagctggtacgggaaccggaattgctggaatcacaaaagcttccctcacctatagccagctctcaaaggaaatagccaacaacattgacaccatggctaaagccttaacgaccatgcaagaacaaatcgactctttagcagccgtagtccttcaaaatcgtcgaggactagacatgttaacggcagcacagggaggaatttgtttggccttagatgaaaaatgttgcttttgggtaaatcaatcaggaaaagtacaagacaacatcagacaactcctaaatcaagcctccagtttacgggaacgagccactcagggttggttaaattgggaaggaacttggaaatggttctcttgggttcttccccttacaggcccacttgttagtctcctacttttgctcctttttggtccatgtctcctaaatctaataacccaatttgtctcctctcgccttcaggccataaagctccagacgaatctcagtgcaggacgccatcctcgcaatattcaagagtcacccttctaaggaggacccctagactgctcgctagtggaacacgacagaggcgaaatcctgccccgtctcccgtggacctggctggatatggtttttgccaatccacagagccatcctgccctgacagctagcaagaggccaagacccacagaacaaccactacagcccctctgtcagcaggaagcagttaaagaagactgaccttcgtccattttcccagataattgggtcttggactcttgagggggggaaatgttggagcaggtagctagtcagacatgagcagggcaggggagggccccctcaccaggaatgtcaggcaaccatcaggtgatggtgaggcagttgttaagctgtgtctctaacataataatgagtggcagctggcgccagggaacgatggcctcccaatagataggaaacacctgaagctggtgatcagccacttcctgataagatctcaggagttgggtgcgcaggctcaagcatgcaccctaagaggcaaaatagtggcatttaactcatatatgaccttcctttaggaaggcttgactggtaagggaaaaactcctccagtgaacacgtgcacaacttcagtaaaaacactgcacatgcgtcccctcccaagtgctggcaggccactgtgcatgc

SEQ ID NO: 6 - DNA, 12239 bp, Homo sapiens
gaacaagcccctcattctaaaattcaccttaataagaaactgcctaaatccaaagggcatccccctaatggctaaggtcagcatgaccataaaccacaaacaacatcaccaacctgaaacattccaaactcctcccagatcagagacatactagcctcaaaataaacccctctctgggccggaaagatgtctgccccaagataacctcccctcctcccaaagagattccaaccccgccataaaattctccacacacataaatattccaagcttgtgataagccccctcgccctaaaaccaatatatattcttagtctgtaaaaggaaacacttcttaacgaaatcggccaggagtgcctctcaggttttgtctaaaataaacctgtctttaactgccagccgcgttttgtgtttctttcctttctttaactcttacatttggtgcccaaacccgggatgagtgctgggggcagaggctctcttgcaacccaggaagcagtgggcaacagcagctcatcttgagttaattcctggatcctgagggtctctggccacatgccccatcttttctctcacttcacttttccctcatcctccctttttttttcttcctctctctctctccctcgtgcggctgcagtccaggaggccctttgccaaatccaaccggaacatccaacattggacactaatccagccaactggtaagatctgccgtcccctggctttcttgcagtacccaggaaaagtcaggtcagccatcccggtcctcagaggaccagcaggactaagctagaggaaatcttggggatgcccagtttcttctcagcttgatgactgtcctcttcagaaagacgattccggacttctgtcttttgtctggggatgcctagaacaaaaacagacaccctcggcttcttctcaccagtccacatgggtgccaaacaattccacattcctacggtctctccactgtgctgtctccttcatgacctcgccaaagttggcttaagtgtttagtcttttactgtaacacagcctggccccaaaacacattagataatggcagcccatggtccgaaaatggcatctttaacttgcaaattctcaggaacttcacaactttatgaccaggaatggcaaatggcaagaggttctctatattcaggccttcttctacttctaccttaaatcccaaccctacctgtgtcaagcttgtacctcttataaaatctttcttcttattaaaaaccctctccgggtctctccttcctccgaaactccttttgaccctgcagatgaaccctctctgtattcttatccccctgcatctgctcctagcctgtccaaaccctccaccctggtggccctacctgcctccaagccttcagccccaaaccccactcctcctcctcctccacctgttacccattcaaaaaccacctctgccattctccctctctgggaagtggctggagttaaaggcactgctcatgttcatgtctctttctccatgtctgacttgtcacagatcaaaactatgagtatattcaaaaggtctttatagttttctcttcatcaatcttattttcctggaaaaggttttcccccagttaactcaattacttttcttcactgtgtcttgcaactcttggtgcatatgtaaaaaaccctaaaatgacttctggtgccctgggattcctttggaaaagagaaaaggcaccacaaatcccattttggggaaaaatctgttttccttatggaaaccgtggaattagaggtaaataagtacctctcaaaatctttgtatttgtcttccagctatacctgtttattagaccctggaaactgttttcctagtcctgttcttcaagggcctcacctgaaggtcaataatccaattgggaaattagcagagagaaaaaaaaaacgttatagctactgaatcttcttctggttgtctgtgtggctatatatgtgttgtctgtgcaatgtctattaaaagagctctaattaattggcctaagaaaactaagcacttaaatcaaatatttttaagggaaaagtaaaagctgtgggacctttcagttcacgtgaccttaatctttaaatcttactggtacactaaagttagaagtatcttaaaagttgccagcatacctttttgtttgcatttgttaatcaggcaaattcatacttttctcggccaaatactgtaaggtgtcaacattttgcatagaggctgcaaaactaactcagcccaaacaaaatcatctttgcttgtgtcatttttttttttaagacagagtttcgctcttgttgcccaggctgaagtacaatagcacaatctcagctcaccacaacctctgcctcatgggttcaagccattctcctgcctctgcctcccaagtagctgggattacaggcatgtgccaccacgcccggggaattttttgtatttttagtagagatggggtttctccaagttggtcaggctagtctcaaactcccaacctcaggtaacccacccgtcttggcctcccaaagtgctggcattacaggcgtgagacaccgcacccagccttgtgtaattttttaataaatgaaatattaatattggtttaatgaagatagctgtatcttaaactatttagtaaaatatcttagcttctaatcttgtggcttaggcagtctagtccacaaacatgaaggaagtttgctttgggaaagaatggttatcatctgtgacattaaagaaaggagaagttatggaaaaagaatcttatatggtaaattcttgtcctaagttaactggttgtttaaagaaagagatgtttacaagtcagaaagttgaggcatgtcaaggattgtctgtgaaagtcatgaaaaatgttataaaagggaatttatacaagaaatgttgtataatttaaaagtaattaggcctcctgaatgctttataaaatgtcactgtaactcttagctggacaactggcctgctttgcagctaggtaaaacctacgacacgtggagttaaatgctagaacatttaactgcacttctttctaggtcctgggctctacacctagcacataattaaaatcccaaacttacaaggttttcaacaaaagtaaagtttactaaaagttaacagcgtagccaagatggccgaataggaacagctcctgtctgcagctcccagcatgatcgacgcagaagacggctaatttctgtatttccaactgaggtacctggttcatctcattgggaatggttggacagtgggtgcagcccatggagggcaagctgaagcagggtggggcgttgcatcacccacaaagcgcaaggagtcgggggtttccctttcctagccaagggaagccatgacagactacctggaaaaatgggaaactacccacccaaatactgcacttttcccaaggtcttagcacccgctgacaagatgattctctcccgtgcctggctcggcgggtcccacgcccacggagccttgctcactgctagcgcagtagtctgagatcgatctgtcaggcggcagcctggctggggaagggtgtctgccattgctgaggcttgagtaggtaaaaaaagtggccgggaagctcgaactgggcagagcccaccacagctcaacaacacctacagcctctagactccacctctgtgggcaaggcatagctgaataaaaggcagcagacaacttctgcagacataaacgtccctatctgacagctctgaagagagcagtggttcctcccagcacggcatttgagctctgagaacagacagactgcctccacaagtgggtccctgacccccgtatagcctaactgggagatacctcccagtaggggccaacagacacctcatataggcagctgccccgctgtgacgaagcttccagaggaagatcaggcagcaatatttgctgttctgcagtatttgttgttctgcagcctctgctggtgatacacaggcaaccagggtctggagtggaactccagcaaactccaacagacctgcagctgagggatctgttagaaggaaaacaaacaaacagaaaggaatagcatcaacatcaacaaaaaggacatctacaccaaaaccccatctgtaggtcaccaacatcaaagaacgaaggtagataaaaccacaaagatgaggagaaccagagcagaaaagctgaaaattctaaaatcagagcacctcttcacctccaaaggatggcagctcctcgccagcaacagaaaaaaagctggaaggagaatgactttgacgagttgacagaagtaggcttcataaggtcggtaataacagacttctccgagttaaaggagaatgttcaaacccatcgcaaggaagctaataaccttgaaaaaagattagactaatggctaactagaataaacagtgtagagaagacattaaataaactgatggagctgaaaatcatggcacaagaacgtcatgacatatgcacaagcttcaatagctgattcgatcaagtggaagaaagggtatcagtcactgaagatcatattaatgaaataaagcgagaaggttagagaaaaaagactgaaaagaaatgaataaagcctccaagaaatatgggactatgtgaaaagaccaaatctacgtttgattggtgtagaaagtgatggggagaagggaaccaagttggaaaacactctgcaggatattatccaggagaacttccctaacctaggaaggcaggccaacatccaaattcaggaaatagagagaacaccacaaagatactccaagagaagagcaaccccaagacacataattgacagattcaccaaggttgaaatgaaggaaaaactgttaagggcagccatagagaaaggtcgagttaatcacaatcggaaggccatcagactaacagtggatctctcggcagaaaccctacaagccagaagaaagtggaggccaatattcaaaattcttaaagaagaattttcaacccagaatctcatatccagccaaactaagcttcataagtgaaggagaaataaaatcctttacagacaagcaaatgctgagagactttgtcaccaccaggcctgccttacaagagctcctgaaggaggaactaaacatggaaaggaacaactggtaccagctactgcaaaaacatgccaaattgtaaagaccactgatgctatgaagaaactgcatcaattaatgggcaaaataaccagcgaacatcataatgacaggaacaaattcatatatagcaatattaaccttaaatgtaaacaggctaaatgccccaattaaaagacacagattggcaaattggataaagagtcaagacccatcagtgtgctgtattcaggagacccatctcatatgcaaagacgcacacagactcaaaataaagagatggaggaagatttaccaagcaaatggagagaaaaaaaaaaaagcaggggttgcaatcctagtctctgataaaacagactttaaaccaacaaagatcaaagagacaaagaaagccattacatgatggtaaaggagtcaattcaacaagaagagctaactatcctaaagatatatgcacccaatacaggagcacccagattcataaagcaagtccttggagacctacaaagagacttagactcctacacaataataatgggagactttaacaccccactgtcaacattagaaagatcaactacaaaaggttaacaagcatatccaggacctgaactcagctctgcaacaagcagacctaatagacatctacagaactctccacccaaaatcaacagaatatacattcttctcagcaccacactgcacttattctacaactgaccacataattggaagtaaagcactcctcagcaaatgtaaaaggacagaaagcacaacaaactgtctcatagaccacagtgcaataaaattagaactcaggattaagaaactcactcaaaactgcacaactgcatggaaactgaacaacttgctcctgaatgactactgggtacataataaaatgaaggcagaaataaagatattctctgaaaccaatgagaacaaagacacaacataccagaatctctggaacacatttaaagcagtgtgtagagggaaatttatagcactaaatggccacaagataaagcagcaaagatctaaaattgacaccctaacatcacaattaaaagaactagacaagcaaaagcaaacaaattcaaaagctagcaaaaggcaagaaataactaagatcagagcagaactgaaggagatagagacacagaaaaaccttaaaaaaaaaaaaaaatcaatgaatccaggagctggttttttgaaaagatcaacaaaattgatagaccggtagcaagattaataaagaagaaaagagagaagaatcaaatatacgcaataaaaaatgataaaggggatatcaccaccgatcccacagaaatacaaactaccatcagagaatactataaacacctctatgcaaataaactagaaaatcaagaagaaacagataaattcctggacacatacaccctcccaagaataaaccaggaagaagttgaatctctgaatagaccaataacaggctctgaaattgaggcaatgattaatagtctaccaaccaaaaaaagtccaggaccagaggtacaaagaggagctggcaccattccttctgaaactatttcaatcaatagaaaaagaggggatccaccctgactcattttatgaggccaacatcatcctgataccaaaacctggcagagacacaacaaaaaaaggagaattttagaccaatatccctgatgaacattgatgcaaaaatcctcaataaaatattggcaaattgaatccagcagcacatcaaaaagcttatccaccacgatccagcaggcttcatccctggaatgcaaggctggttcaacatatgcaaatcaacaaacgtaatccatcacataaacagaaccaaagacaaaaaccacatgattatctcaatagatgcagaaaaggccttcgacaaaattcaacagcccctcatgctaaaattctcaataaacgaggtattgatggaacgtatctcaaaataagagctatttatgacaaactcacaatcaatatcatactgaatgggcaaaaactggaagcattccctttgaaaaccaacacaagacaaggatgccctctctcaccagtcctattcaacatagtgttggaagttctggtcagggcaatcaggcaagagaaagaaataaagggcattcaattaggaaacaaggaagtcaaattgtccctgtttgcagatgacatgattgtatatttggaaaactccaccgtctcagcccaaaatctcaagctgataaccaacttcagcaaagtctcaggatacaaaatcaacgtgcaaaaatcacaagcattcctagacaccaataacagaccaacagagagccaaatcatgagtgaactcccattcacaattgctacaaagagaattaaatacctaggaatacaacttacaaagaatgtgaaggacctcttcaagaataactacaaaccactgctcaacgaaataaaagaggacataaacaaatggaagaatattccatgctcatggataggaaaaatcaatatggtgaaaacggccatactgcccaaagtaatttatagattcaatgtcatccccatgaagctaccaatgactttcttcacagaattggaaaaaactactttaaacttcatattgaatcaaaaaagagcctgaattgccaatacaatcctaagcaaaaagaacaaagctagaggcatcatgctacctgacttcaaactatactacaaggctacagtcaccaaaacagcatagtactggtaccaaaacagatatatagaccaatggaacagaagagagccctcagaaataataccacacatctacaaccatctgatctttgacaaacctgagaaaaacaagaaatggggaaaggattccctatttaataaatggtgctgggaaaactagctagccatatgcagaaaactgaaactggaccccttccttacaccttatagaaaaattaattcatgatggataaaagacttaaatattagacctaaaaccataaaaaccctagaagaaaacctaggcaatatcattcaggacatagttatgggcaaggacttcatgactaaaataccaaaagcaatggcaacaaaagccaaaatagacaaatgggatcaattaaactgaagaacttctgcacggtgaaagaaactaccatcagaatgaacaggcaacctacagaatgggagaaaatttttgcaatctatccatctgacaaagggctaatatccagaatctacaaataactcaaacaaatttacaaaaaaaaaaacaacccccatcataaagtgggcaacagatatgaacagaaacttgtcaaaagaagacatctatgcagccaacagacacacgaaaaaatgctcatcatcactggtcatcagagaaacacaaatcaaaaccacaatgagataccatctcacgccagttagaatggcggtcgttaaaaagtcaggaaacaacagatgctggagaggatgtggagaaactggaatgcttatacactgttggtggcagtgtaaattggtttaaccattgtggaagacagtatggggattcctcaaggatctagaactagaattaccatttgacccagcaatcccattactgggtatatacccaaaggattataaatcatgctactataaagacacatgcacacgtttgtttattgtggcactattcacaagacttggaaccaacgcaaatgtccatcaatgatagactggattaagaaaatgtggcacatatacagcatggaatactatgcagccataaaaaaggatgagttcctgtcctttgcagggacacagatgaagctagaaaccatccttctcagcaaactatcacaaggacctaaaaccaaagaccgcatgttctcactcacaggtgggaattgaacaatgagatcacttggacacagggcagggaacatcacacactggggactgtaaggggatgagggactgcggggagggatagcattaggagaaatacctaatgtaaatgatgagttgatgggtgcagcaaaccaacatggcacatgtatacctatgtatcaaacctgtacgttgtgcacatgtaccctagaacttaaagtataataataaaagttaatggtgtaacatgtatttaaagctattgaaaaaacagtttatatgcaaggtgtgtaaggaaagtaaaatatacttttcgtaaaaggattataaggaggcataagaatgtggatttttacctacattaaaaagttaaaaaattgttttgaaggtttaagcaagttttgaaacgttaattataaaggaaattctgtgtgtaaacatattggtaaagttaaaggggtatcatccagtttttctgtaaattgggcattaaaacaaaagcacaatgggtttttcttaaagcactaacctgttctttaacaaaacttataaagcattaaaaaaagtctataaaaatcttaccttatggtcagatattaaaattggataaatatgcctacaaggtcttattaaaattgagtttaacattaatagcacactaatagaaaggtgaaatttagcttatctggtataaaatcatacaagaagcattgtcaaatataaaacggtatttggctttctttggtctatatttgtatgttactcatatgtgttccaaagttatggaagactcctataattctgatatatattagtgtacattttcagtaataattacaatcgttatgttaaaattattgtgtgtcatccttgtcaattgtgtctttatggctaccctaaaactttttgtcatccataaacaattgttgccttgttttggtcctctttaaaaggtggttttataatcagctataaagctctaacaggtgctcttaaatgcaggtttctgataacactggagactgtaacatcagaatagaggaaaaacgttcaggacttttgaagagataaaatgttaatattgagcatgacaggaattaattccatgaactaaactaacaggagaccaatctttttaatgttttaacatattgctaatcctttgttttgcttttcaaagtcaaagaaatttttcttttgagctattaacagcttttaacaatttactatactaccatgaacaaaatttggaacatacttgtttctctctacctgattttctccataattttgaaactatctgtgagtattcttaagttacagtacttgcataagtgcactaaaaatctgttttcttttgtaacaggacagaattggaaaaactggttatttttacaaaggctttaactggaataatatgctttcctttaaggaaccatacttacaaaggcaaaaatgcccttggaaaactggcctcatattttgtgtacacagtccctgtacagggtttctggtctatggtaagtaaagaatgtcactttctagcagaccaggaataccaagttatcttgggacctcaagaggaaagaaattcaccaactcatagatatttgatagtacaaatccagggctgggcttggctaaaacggttttctctcagattccttctacagaacaaagttccatcaaagccaatttaaaaggcctatgtaacaaataattattcttgctgcactgtatgcaaataattaagccaagtataataaagcaaaccattcctaccatgatttgtcttttaataaaaatgggaaactggaaaaagaaaattatatttaaaaaaccatagcacacctgttgttaaattctagtgttgcctaacatttttcagtttttattattttctactgcttaaattaaattctaatttttctggctacaagtttccaaaataagtcgggctttcttaaagccctataaactgaaaactagatgtttcagcagacgctgcctctaagctccccgaccatcacagaaggaaatctcttcactgctggtgctgacaactaataactgagggtgcccagaatccttcacccccatgtctagtgaatccacggaacccagggtaattaaaatggtacctgttacaggaatcaactcctaaatacatcacactcaagtcaaagcctggaaagctaaggaagcaacccctgacagcccccaaaagtcataaatatcaatgtaaagaaataagaaatcttgctaggtgaagtagctcacgcctgtaatcccagcattttgggaggctgaggcacatgtatcacctgaagccaggagttcaagaccaccctgaccaacaaggtgaaaccccatctctacttaaaaaatacaaaaattagccgggcgtacaggcaggcgcctgtagtcccaagctactcgggggctgagacaggagaactgcttgaacctgggagttggaggttgcattgagctgagattgcgccactgtactccagtctgggtgacggagcaagagtctgactccaaaaaaaaaaaaaaggaaataaaaagctaaggaaatatctaaacaaccaaacagattcttggtttggaaacaaaatcatagcatgtgtcatcccattcctgagcccccttctaataatatgcctgggactaatgttcttaccctgcccaattaacctttttcaaagatttttatctgacaggatcatggccatttcacagacaactacccaaaaacatctacagatgtcattgctcctacagtcaacctgagaccagaaaactctccatcccctagtcagcaggaagtagccagaagaacacgccgtccctcctcaaattatagggtctggattgacagagtaggagcatcgccatcttggacaagcccctcattctaaaattcaccttaataaaaaactgcctaaattcaaagggcatcagcctaatggctaaggtcagcatgaccataaaccacaaataacatctccaaccagaaacattccaaactcctccctgaccagagacatgctagccccgaaataaaccccgctccagttggaaagatgctagccccgagataacacccctcctggccggaaagatgtctgccccaagataacctcccctcctcccagagagattctaaccccaccataaacttctccacacacataaacattcca

SEQ ID NO: 7 - DNA, 5800 bp, Homo sapiens
gtgccaactgtcaggcctctgagcccaagctaagccatcatatcccctgtgacctgcacgtacacatccagatggccagttcctgccttaactgatgacattccaccacaaaagaaatgaaaatggcctgttcctgccttaactgatgacattatcttgtgaaattccttctcctggctcatcctggctcaagagctcccctactgagcaccttgtgacccccactcctgcccgccagagaacccccctttgactgtaattttcctttacctacccaaatcctacaaaatggccccacccccatctcccttcgctgactcttttcggactcagcccacctgcacccaggtgaaataaacagctttattgctcacagaaagcctgtttggtggtctcttcacacggacgtgagtgaaatttggtgccatgactaggatcgggggacctcccttgggagatcaatcccctgtcctcctgctctttgctctgtgagaaagatccacctacaacctcaggtcctcagaccgaccagcccaagaaacatctcaccaatttcaagtccggtaagcggcctctttttactctcttctccaacctccctcactatccctcaacctctttctcctttcaatcttggcaccacacttcaatctctcccttctcttaatttcaattcctttcattttctggtagagacaaaggagacacattttatccatggacccaaaactccggtgctggtcatggactagggaaggcagccttcccttcgtgtttaatcattgcagggatgcctgtatgattattcacccaggtttcagaggtgtcagaccacgcagggacgcctgccttggtacttcacccttagcggcaagtcccacttttctgggggaggggcaggaaacctaatcccctatctctgtgccccagtccttatttctgcaccccaacctcttatatctgcgccccaaccccttatttccatgccccaaccccttctctgcttttatggagggcaagaactccccaccccttctccgcttttatggagggcaagaaccccccaccccttctccgtgtctctactcttttctctaggcttgcctccttcactatgggcaagcttccaccttccattcctccttcttctcccttagcctgtgttcttaagaacttaaaacctcttcaaccctcacctgacctaaaatctaagtgtcttattttcttctgcaatgctgcttgaccccaatacacactcaacagtagttccaaatagctggaaaatggcactttcaatttttccatcctacaaggtctaaataattctgtcgtaaaataggcaaacggtctgaggtgcctgacgtccaggcattcttttacacatcagtccctccctagtctctgttcccaatgcaacttgtcccaaatcttccttctttccctcctacctgtcccctcagtcccaaccccaagtgtccctgagtctttctaatcttccttttctacagacccatctgacctctcccctccttgccaggctgagctaggtcccaattcttcctcagcctccgctcctccaccctataatccttttatcacctcccctcctcacacccggtccagcttacagttttgttccgtgactagccctcccccacctgcccagcaatttactcttaaaaaggtgcctggagctaaaggcatagtcaaggttaatgctcctttttctttatcccaaatcagatagcgtttaggctccttttcatcaaatataaaaatccagcctagttcatggctcatttggcagcaaccctgagatgctttacagccctagaccctaaaaggtcaaaaggatgtcttattctcaatatacattgtattacccaatctgctcccgacattaaataaaactccaaaaattaaattctggccctcaaaccccacaacacgacttaattaacctcgccttcaaggtgtacaataatagagtagaggcagccaagtagcaacatatttctgagttgcaattccttgcctccactgtgagacaaaccccagccacatctccagcacacaagaacttccaaacgcctaaagcacagtggccaggcattcctccagaaccgcctcccccaggagcttgctacaagtgccagaaatctggccacaaggccaaggaatgcctgcagcccaggatacctcctaagccatgtcccatctgtgtgggaccccactggaaactggtctgttcaacttacctggcagccactcccagagaccctggaactctggcccaaggctctctgactggctccttctcagatcttcttggcttagtggctgaagacggacactgcccgattgccttggaagccctgtagaccatctcagacactgagctttaggtaactctcacagtgaagggtaagtccatccccttcttaatcaatatggaggctacccactccacattaccttcttttcaagggcctgttcccttgccttcataactgttgtgggtattgaaagccaggcttctaaacctcttaaaactccccaactctggtgccaacttagacaatactcttttaagcactcctttttaattatccccacctgcccagttcccttattaggccgagacactttaactaaattatctgcttccctgactattcctggattacagctacatctcgttgccgcccttcttcccaatccaaagcctcctttgtgttctcctcttgtatgcccccaccttaacccacaagtataagatacctctactccctcctttgcgaccgatcatgcaccccttaccatctcattaaaacctaatcacccttaccccgctcaatggcaatatcccatcccacagcatgctttgaaaggattaaagcctgttatcacctgcctgctacagcatggccttttaaagcctataaactctccttacaattcctccattttacctgtcctaaaaccagacaaggcttacaagttagttcaggatctatgccttgccaaccaaatcgttttgcctatccaccccatggtgccaaaaccatatactctcctatcctcaataccaccctccacaacccattattctgttctggatctcaaacatgctttctttactattcctttgcacccttcatcccagcctctctttgctttcacttggactgaccctgacacccatcaggctcagcaaattacctgggctgtactgctgcaaagcttcacagacagcccccattacttcagtcaagcccaaatgtcttccttatctgttacctatctcagcataattctcataaaaacacacgtgctctccctgctgatcatgtccaactaatctctcaaaccccaaccccttctacaaaacaactcctttccttcctgggcatggttgaatacttttgcctttggatacctggttttgccatcctaacaaaaccattatataaactcacaaaaggaaacctagctgaccccatagatcctaaatcctttccccactcctctttctgttccttcaagacagctttagagactgcccccatcctatctctccctgactcatcccaaccctttttattacacacagccgaagtgcagggctgtgcagttggaattcttacacaaggaccggaatcgcgtcctgtagcctttttgtccaaacaacttgaccttactgttttaggctggccatcatgtctccgtgcagtggctgctgccgccctaatacttttagaggcccttaaaatctcaaactatgctcaactcactctctagagctctcataatttccaaaatctattttcttcctcacacctgacacatatactttctgctccccggctccttcagctgtactcactctttgttaagtctcccacaattaccattgttcctggcccggacttcaatccggcctcccacattattcctgataccacacctgacccccatgactgcatctctgatccacctgaccttcaccccatttccccacatttccttcttccctgtttctcaccctgatcacacttggtttattgatggcagttccatcaggcctaatcgccacacaccagcaaaggcaggctatgctatagtataagccactaacccgcctcttagaacctctcatttcctttccatcgtggaaatctgtcctcaaggaaataacttctcagtgttccatctgctattctactactcctcagggattcttcaggccccctcgcttccctacacatcaagctcagggatttgccccctcccaggactggcaaattagctttactcaacatgccccgagtcaggaaactaaaatacctcttggtctaggtagacactttcactggataggtagaggcctttcccacagggtctaagaaggccaccacggtcatttcttcccttctgtcagacataattcctcggtttggccttcccacctctatacagtccaacagcagaccggcctttattagtcaaatcagccaagcattttttcaggctcttggtattcagtgaaacctttatatcccttacagtcctcagtcttcaagaaaggtagaacagactaatggtcttttaaaaacacacctcaccaagctcagccaccaacttaaaaaggactagacaatacttttaccactttcccttctcacaattcaggcctgtccttggagtgctacagggtgcagcccatttaagctcctgtgtggatgctcctttttatcaggcctcagtctcattccagacaccagaccaacttggactgtgccccaaaaaacttgtcatccctactatcttctgtctagtcatactcctattcaccgttctcaactactcatacatgccctgctcttgtttacactgccggtttacactgtttctccaagccatcacagctgatatctccttgtgctatccccaaactgccactgttaactcttaaataaataatctttgctggcaggactatgctgaatctccttaggcactctctaattagatgtcctgggtcctcccaattattagtcctttaatacctgtttttctccttctcttattccatttagtttttcaattcatacaaaaccgtacccaggccatgaccaataattctaaatgacaaatatttcttctaacagtcccacaatatcaccccttaccacaaaatcttccttcagcttaacctctcccactctaggttcccacgccgcccctaatccggctcaaagcagccctgacaaacatcgcccattatctctccataccatcccctcaaaattttcgccgtcccaacactttaccactatttcattttatttttcttattaatataagaagacaggaatgtcaggcctctgagcccaagctaagccatcatatcccctgtgacctgcacgtacacatccagatggccagttcctgccttaactgatgacattccaccacaaaagaaatgaaaatggcctgttcctgccttaactgatgacattaacttgtgaaattccttctcctggctcatcctggctcaaaagcttccctactgagcgccttgtgacccccactcctgtccgccagagaacaacccccctttgactgtaattttcctttacctacccaaatcctataaaatggccccacccctatctccctttgctgactctctttttggactcagcccgcctgcacccgggtgaaataaacagctttattgctcacacaaagcctgtttggtggtctcttcacacggacgccagtgaaaccgacctcc

SEQ ID NO: 8 - DNA, 6762 bp, Homo sapiens
gtcaggcctctgagcccaagctgagccatcatatcccctgtgacctgcaggtatacatccagatggcttgaagcaactgaagaaccacaaaagataacattccaccattgtgatatgttcctgccccaccctaactgatcaactgaccttatgacaatacaccctccctgcccttgtgataatgcactttgtgatattcccctgctcttaacaaggtactttataatattctccctgcccttgagaatgtactttgtgagatccacccctggcccacctatcccaaacctataagaactaatgataatcccaccacaatttgctgactcctttttcagactcagccaacctgcacccaggtgaaataaacagccttgttgctcacacaaagcctgttggtggactctcttcaaatggacgtgcatgacatttggtgccgaagacccgggacagggggactcctttgggagaccagccccctgtccttgccctcactccgtgaggagatccacctatgacctcaggtcctcagaccaaccagcccaaggaacatctcaccaattttaaatcgggtaagcagtcttttcactctcttctccaacctctctcgctatccctccacccttcaatctctcccttccttaattttggttcctttccctttctggtagagacagaggagacgcgttttatccgtgatctcaaaactctggtgccggttacggactgaggaagacagtcttcccttggtgtttaatcactgcggggatgcctgcctgattattcacccacatttcagaggtgtctgatcaccgtggggatgcctgccttgaaccttcacgttggtggcaagtaccaccttccctgggaggcaagcaccaccctcccgcccatgtctctaccctctcttttctctgggcttgcctctttcactatgggcaatctttcaacctccattcctccttcttctcccttagcctgtgcaagaacttaaaacctcttcaattcttgcctgacctaaaaacctaagcatcttattttcttctgcaacactgcttggccccaaaacaaacttgataatggctctaaatggccagaaaacggcacttttgatttctccatcctacaagatctagataattactgtcgtaaaaatgggcaaatggtctgaggtgcccgacgtccaggcattcttttacacatcggtccctccctagtctctgctcgcaatgcgactcgtcgcaaatctttcttctttctctcctgtctgttccttcagtttccaccccaagctctgagtcctttgaatcctcctcttctacggacccatctgacctctcccctcctccccaggctgctcctcgccaggctgagccaggtcccaattcttccttggcctctgctcccccaccctataatctttctatcacctcccctcctcacacccggtctagattacagttttgttccatgactagccctcccctacctgcccaacaatttcctctcaaagaagtggctggtgctaaaggcataatcaaggttaatattcctttttctctatcagaccttcagaccttccccaaatcagttagcatttggactttttcatcaaatatgaaaacccagcccagttcatggcccatttgttaacaacccttagacgttttaccaccctagacccagaggggccagaagtccgtcttattctcaacatacattttattacccaatctgctcccaacgcacatcaggacttaattaacctcgccttcaaagtgtacaataatagagaagagttgcaattacttgcctccgctgtgagacaaaccccagccacatctccagcacacaagaacttcaaaacgcctgaactgcagcagccaggcattcctccaggacctcctcccccaggatcttgcttcaagtgccgaaaatgtggccactgggccaaggaatgcccgcagcccgggattcctcgtaagctgttgtcccatctgtgtggggccccactggaaatcggactgtccaacttgcccggcagccactcccagagccctggaactctggcccaaggctctctgactcctttccagatcttcttagcttagtggctgaaatctgacgctgcctgatctcctcaaaagcctcttggaccatcacagacactttgggtaactcttacagtggagggtaagttcatccccttcttaatcaatacagaggctacccactccccattaccttcttttcaacggcctgtttcccttgtctccataactgttgtgggtattgatggccaggcttctaaacctcttaaaactccccaactctggtgccagcttggacaacattcctttatgcactccttttttagttaccctcacctgcccagttcccttattaggtcgaggcattttaactaaattatctgcttccctgactattcctgggctacagccacacctcactgctgcccttttccccagttcaaagcctcctttgcatcttcctattgtatccccccaccttaacccacaagtgataggacacctttactccctccatggcaaccaatcacatgcccattactatcccattaaaatctaatcagccttacccggctcaacgccagtatgccatcccacaacaggctttgaagggaataaagcctgtccaggatcttcgccttattaatcaaatcatccttcccatccatcctatggtgccaaacccatatactttcctatcctcaataccttcctccacaacccattattctgttctggatctcaaacatgctttctttattattcctttacacccttcatcccagcctttttttgctttcacttggactgacccagacacccatcagtctcagcaacttacctgagctgtactgccggaaggcttcagggacagtccccattactttagtcaagccctttttcatgatttactttctttccatccatctgcttctcaacttattaagcattttgataaccttctactttatagcccctcctacaaatcttcccaacaggacaccctcctgctcctccaacatctattctcaaaaggacatcgcacatccccctccaaagctcaaatttcttccccaaccgttacctacctcggcataattcttcatgaaaacatgcatgctctccctgctgatcatgtccagctaatctcccaaacctcaaccccttctacaaagcaagaactcctttccttcctaggcatggttaggtactttcgcctttagatacctagttttgccatcctgacaaaaccattatataaattcacaaaggaaacctagctgaccccataaatcctcaatcctttccccactcccctttccattctttaaaaaacagccctaaaagctgctccccactagctctccctaactcatcccaaccctttttcattacacacagccaaagcgcagggctgtgtggtcaggattcttacacaagagctgggaccgtaccttgtggcctttctgtccaaacaacttgaccttactgtttcaggctggcccccacgttattcctgataccacacatgacccccatgactgcatctctctgatctacccagcattcacttcatttccccatatttccttctttcctgttcctcaccctgatcacacttggtttattgatggtagttcttccaggcccaatcgccaatcactggcaaaggcaggctatgctatagtgtcttccccatctatcactgagtctaccgctctgcccccctccactacctctcagcaagccgaactcactgtcttaactcaggccctcactcttgcaaaagaactgtgcgtcaatatttatgttgactctaaatatgccttccatatcctgcaccaccatgctgttacatgggcagaaagaggtttcctcactacacaaggatcctccattattaatgcctctttaataaaaactcttctcaaggccgctttacttccaaaggccactttacttcaaaaggaagctggaatcattcactgcaagggccatcaaaaggcatcacatcccagtgctcagggcaacgcttctgctgataaggtagctaaagaagcagctagcgttccaacttctgtccctcatggccagtttttctccttctcaccggtcactcccacctactctcccactgaaacttccacctaccaatcttttcccacataaggcaaatggttcttggaacaaggaaaatatctccttccagactcacaggcccattctattctgtcatcatttcataacctcgtccatgaaggttacaggctgctagcccatctcttagaacctctcatttcctttccatcatggaaatctatcctcagggaaatcacttctcagtgttccatccactattctactactcctcagggattgttcaggccccctcccttccctatacatcaagctcggggatttgcccctgcccaggactggcaaattgactttactcacatgcctcgagtcaggaaactataatacctcttggtctgggtaaacactttcactggatgggtagaggcctttcccacacggtctgagaaggctaccacagttatttcttccattctctcagacatacttcctcggtttggcctttccacctctatacaatctgataacagaccggcctttattaatcaagtcattcaggcagtctcccagtccctgggcattcaatggaaacttcgtgctccttatcgccctcaatcctcaggaaaggtagaaagaactaatggtcttttaaagacacacctcaccaaactcagcctccaacttaaaaaggactggacagtacttttaccacttgcccttctcagaattcgggcctgtcctcgggatgctacagggtacagcccatttgagctcctgtatggacgctctttttcattaggccccagtctcattccagacaccagccctctaggtgactatcttccagtcctccagcaagctacacaggaaatttgccaagctgctaatcttctcttgcctactccagattcccagtcatatgaagacaccctagctggatgatcagttcttgttaagaatctgacccctcaaattctacaacctcgatggaccagaccctacttagtcatctatagtaccccaactgccgtccgcctacaggaccctccccattgggttcaccattccagaataaagctgtgtccatcggacagccagcctgaagtctcaagtactctcccctacttcccttaaactcacttgcatttctgaataacagtaataaaccttatgagcctaatacatcccttcattctattaggtctattcgtccttaccctactttttgcaacagggctttacgcagtcactcccactacttggactgtgccccaaaaccttgtcatccctcctatcttctgtctagccatactcctattcaccattctcaactactcgtaaataccctgcccttgtttacattgctggtttacacttttcctccaaaccatcatagcggatatctcctggtactatccccaatcagccactcttgactccctcttggagtgaacagatgatctttgctgacagggcacactccaatactttcgccctgacgaagtcctattctttacttttatactcactcttattttcattctcgtcttatgccaccctctacctctccccggctatctccaccacactatcaatctcactcactctctcctagccatttctaatccttccttaacaaacagttactggctttgcatttctctttcctccagaaccaccgaggcctcgaccttactcactgctaaaaaaaaaaaaaaaagagcagactctatatttttaaatgaagagtgttgtttttacctaaatcaatctggcctggtatatgacaacataaagaactcaaggctagagccccaaaactccccaaccaaataattatgctgaacccccttgggcactctctaattggatgtcctgggtactcccagttcttagtcctttaatacctgttttcctcttccttttattcagaccttgtatcttccatttagtttctcaattcatacaaaactgcatccaggccatcaccaatcattctatataacaaatgttccttctaataaccccacaatatcaccccttaccccaaaagctttcttcagtttaatctctcccactataggttcccacgctgcccctaattccgctcgaagcagccctgagaaacattgcccatgatctctccataccacccccaaaaatttttgccaccccaacacttcaccaccattttgttttgtttttcttattaatataaaaagacaggaatgtcaggcctctgagcccaagctaagccatcatatcccctgtgacctgcaggtatacatccagatggcctgaagcaactgaagaaccacaaaagatgacattcctccattgtgatcttttcctgccccaccctaactgatcaattgaccttatgacaatacaccctccccacccttgtgataatgcactttgtgatattcccctgcccttaagaaggtactttgtaatattctctacgcccttgagaatgcacttggtgagatccacccgctgcctgcctatcccaaacctataagaactaatgataatcccaccacccgttgctgactccattttcagactcagcccaactgcacccaggtgaaataaacagccttgttgctca

SEQ ID NO: 9 - DNA, 13377 bp, Homo sapiens
tggcctgagaaggactccatacttctatatttgtgttcttgtggacaaaccataacctagcacaataggcagacaaaatggaaaacctgagtagtatgcatctgtaataatagctgagtgttggccaatcccagtggccatacttcaagcactaatagactgctaagtgttcaaactgcattcaattctggaggctgcctgatttgcaaagtgtttattttccttgcttaattaaactccatcaaatttaacttgtctgaagttttcttttaacagatctggtgtcagaagtgggatttgaagaaaaactctggcaaccccctggaacaccaggtgacctggtgaggtacccactgaggccgttgctctcactggtctcttgattgtaactggaggtcatgggtgagttttctctcagattccgagctccactaacttgtgttttgagctctccgagtttactcaagcaatacttagcctggactggatccaagatcaaattggatttgataattaactggattggattcagttagaggcctcagacctctgataagtaccttatttaataatgggatcatctcaatccaaggagtctgggactccatcttcagggactccagctaattttacgtataaaaattatgggcccagaacatgtgcattttcagtaaaatgggttaacctcactaaagaaaacttagaattaaaatggccacaatggagaagttttaatttggataaaattgtttgcaaggcatattagaaaaaggggatcaaagcccccacaaatacagtgggatgtattgtctcatggatacgcaaaggcctccaaaagactaagtgaatcaaaaagtgcctccttaaaagattctttgcaaaaaccaaatgaaaagcttaagcaacagaccaaggacatgaagaaagaggactgtactttgactgatctaactcggactgttccttctttgtccatctctacctacatactctgagtccactaaactttttgttaaattacactttcaccctgaagatgatttaaaaaaaaaaaaaaaaaaaaaaggaagttagacagatgtcttacaaagtgagaccttatatcagccaggcctgcctgctgtaactactttcactccatggtctaaaactgagcttagccccattgtgaaggacttccctggtccaagggaaaagtctcaaaaatttactgaggaatttagaatcctaataggagcttacgatccaggacttcatgaatttaccaatttattcatatgatactgggggctggtgaagctcagaaatggatggcagcagcagaatgggacaaacctgaggaggacattttaaagggccctctaagagctcctcacaagaaggaccaaaaatagctagaaaaatcgctgaaaaccttttaacattcagttcctaaaatttttccacaaaaaattggtccatcatacaatcttgtaagcaaaaaaaaaagaaaagaaaagatgaaccagtttcagattacagaagtcgcttagaaatatttgtgaaacatcctgggctcaaagtacagcaaggagtattccctgcaggggctgaaacagcattaactgctttacttataaatggactccatcctgaacttagcagtttaactaaaaaacataagttgcaatgggaagttagagatgtgactgaattggtggccttagctgaactttttttttttttttttttttttttgaggtggagtcttgctctgtcacccaggctagagtgtagtggcgcaatctcggctcactgcaacctctgcctcccaggttcaagcaattctcttgcctcagcctcccgagtagctgcgactacaggcgtgtgccaccatgcccagctaatctgtgtatttttagtagagatgggatttcaccatcttagccaggatggtcttgatctcctgacctcgtgatcctcccaccttggccttccaaagtgctgggattacaggcgtgagccatcgtgcccaacctagctaagcattttgagaagactctagagcaaaaaaaacctcaaaaggctaataagcttatgccccttcaattgcaacagttacagggaccaggaaccaaagggaccatctcgttctcattttaaatcacaatcgggcggttccaagatggccaaataggaacagctccagtctacagctcccagcttgagcgacgcagaaaacgggtgatttctgcatttccaactgaggtactgggttcatctcactggggattgtcagacagtgggtgcaggacagtgggtgcagcgcaccgagcatgagccaaagcagggcgaggcatcgcctcacccaggaagcacaaggggtcagggaattccctttcctagccaaggaaaggggtgacagacagcacctggaaaattgggtcactcccaccctaatactgcgcttttccgatggtcttagcaaacagcacaccaggagactatatcccgcgcctggctcagcgggtcctatgcccatggagcctcgctcattgctagcacagcagtctgagatcaaactgcaaggtggcagcgaggctgggggaggggtgcccgccattgcggaggcttgagcaggtaaaaaaagcagctgggaagctcgaactgggtggagcccactgcagctcaaggaggcctgccttcctctgtagactccacctctgcaggcagggcatagccgaacaaaaggcagcagaaacctctgcagacttaaatgtccctgtctgacagcttggaagagagcagtggttctcccagcacacagcttgagatctgagaacagacagactgcctcctcaagtgggtccctgacccccgaatagcctaactgggaggcaccccccagtaggggcagactgacacctcacatggccgggtacccctctgagacaaaacttccagaggaacgatcaggcagcaacatctgctgttcaccaatattcgttgttctgcagcctccgctgctgatacccaggcaaacatggtctggagtggacctccagcaaactccaatagacctgcagctgagggtcctgactgttagaaggaaaactaacaaacagaaaggacatccacaccaaaaacccatctgtacatcaccatcatcaaagaccaaaggtagacaaaaccacaaagatggggaagaaacagagcaaaaatactgaaaattctaaaaatcagagcacctctcctcctccaaaggaatgcagctcctcaccagcaacggaacaaagctggacagagaatgactttgacgagctgagagaagaagacttcagacaatcaaactatccaagctaaaggaggaagttcgaacccatggcaaagaagttaaaaaccttgaaaaaaattcgacgaacggctaactagaataactaatgcagagaagtccttaaaggacctgatggagctgaaaaccaaggcacgagaactacgtgacggatgcacaagcctcagtagccgattcgatcaactggaagaaagggtatcagtgatggaagatcaaatcaatgaaatgaagcgggaagagaagtttagagaaaaaagaataaaaagaaacgaacaaagcctccaagaaatatgggactatgtgaaaagaccaaatctacgtctgattggtgtacctgaaagtgacgggaagaatggaaccaagttggaaaacactctgcaggatattatccaggagaacttccccaatctagcaaggcaggccaacattcaaattcaggaaacacagagaatgccacaaagatactcctcgaaaagagcaactccaagacacataattgtcagattcaccaaagttgaaatgaaggaaaaaatgttaatggcagctagagagaaaggtcaggttacccacaaagggaagcccatcagaccaacagctgatctctcggcagaaactctacacgccagaagagagtggaggccaatattcaacattcttaaagaaaagaattttcaacccagaatttcatatccagccaaactaagcttcataagtgaaggagaaataaaatcctttacagacaagcaaatgttgagagaatgacaggatcaaattcacacataacaatattaaccttaaatgtaaatgggctaaatgctccaattaaaagacacggactggcaaattggataaagagtcaagacccatcagtgtgctgtattcaggaaacccatctcacgtgcagagtcacacataggctcaaaataaagggatggaggaagatctaccaagcaaatggaaaacaaaaaaaggcaggggtttcaatcctagtctctggtaaaacagactttaaaccaacaaagatcaaaagagacaaagaaggccattacataatggtaaagggatcaattcaacaagaagagctaactatcctaaatatatatgcaaccaatacaggagcacccagattcataaagcaagccctgagtgacctacaaagagactcagactcccacacaacaataatgggagactttaacaccccactgtcaacattagacagaccaacgagacagaaagttaacaaggatatccaggaattcaactcagctctgcaccaagcggacctaatacacatctacagaactctccaccccaaatcaacagaacatacgttcttcttagcaccacactgcacttattccaaaattgaccacatagttggaaataaagctctcctcagaaaatgtaaaagaatacaaattataacaaactgtctctcagaccacagtggaatcaaactagaactcaggattaagaaactcactcaaaactgctcaactacatggaaactgaacaacctgctcctgaatgactactgggtacataacgaaatgaaggcagaagtaaagatgttctttgaaaccaatgagaacaaagacacaacataccagaatctctgggacacattcaaagcagtgtgtagagggaaatttatagcactaaatgcccacaagagaaagtaggaaagatctaaaattgacaccctaacgtcacaattaaaagaactagagaagcaagagcaaacacattcaaaagccagcagaaggcaagaaataaataagaccagagcagaactgaaggagatagagacacaaaaaacccttcaaaaaatcaatgaatccagtaactggtttttcgaaaagatcaacaaaattgatagaccgctagcaagactaacaaagaacaaaagagagcattcttatataccaataacagacaaacagagagccaaatcatgagtgaactctcattcacaattgcttcaaagagaataaaatacctaggaatccaacatacaagggatgtgaaagacctcttcaaggagaactacaaaccactgctcaaggaaataaaagaggatacaaacaaatggaagaacattccatgctcatgggtaggaagaatcaatatcgtgaaaatggccatactgcccagggtaatttatagattcaatgccatccccatcaagctaccaaagactttcttcacagaattggaaaaaactactttaaagttcatatggaaccaaaaaagagcctgcattgccaagtcaatcctaagccaaagaacaaagctggaggcatcacgctacctgacttcaaactatacaaggctacagtcaccaaaacagcatggtactggtaccaaaacagagatataggccaatggaacagaacagagccctcagaaataacgccgcatatctacaactatctgatctttgacaaacctgacaaaaacaagaaacggggaaacgattccctatttaataaatggtgctgggaaaactggctagccatatgtagaaagctgaaactggatcccttccttacaccttatacaaaaattaattcaagatagattaaagacttaatttagacctaaaaccataaaaatcctagaagaaaacctaggcaataccattcaggacataggcatggccaaggacttcatgtctaaaacaccaaaagcaatggcaacaaaagccaaaattgacaaatgggatctcattaaagtaaagagcttctgcacagcaaaagaaactaccatcagagtgaacaggcaacctacagaatgggagaaaatttctgaaacttctcatctgacaaagggctaatatccagaatctacaaagaactcaaacaaacttacaagagaaaaacaaacaaccccatcaacaagtgggtgaaggatatgaacagacacttctcaaaagaagacatttatgcagccaaaagacacatgaaaaaatgctcatcatcactggccatcagagaaatgcaaatcaaaaccacaatgagataccaactcacaccagttagaatggcaatcattaaaaagtcaggaaacaacaggtgctggagaggatgtggagaaataggaacacttttacactgttggtgggactgtaaactagttcaaccattgtggaagtcagtgtggcaattcctcagggatctagaactagaaataccgtttgacccagccatcccattactgggtatatacccaaaggattataaatcatgctgctataaagacacatgcacacgtatgtttattgcagcactattcacaatagcaaagacttggaaccaacacaaatgtccaacaatgatagactggattaagaaaatgtggcatatatacaccatggaatactatggagccataaaaaatgatgagttaatgtcctttgtagggacatggatgaagctggaaaccatcattctcagcaaactatcacaaggacaaaaaaccaaacaccgcatgttctcactcgtaggtgggaactgaacagtgagaacacttggacacaggaaggggaacatcacacactggggcctgttgtggggttgggggaggggggagggatagcattaggagatatacctaatgtaaatgatgagttaatgggtgcagcacaccaacatggcacatgtatacatatgtaacaaacctgcacgttgtgcacatgtaccctaaaacttaaagtataataaaaaaaaatttttttaagtcacactttggaaaatatttttaaaattatatattaaaaaaatcaaatcaagaggtcccagaacaagaatttctttaccccaagatgtctgcctgtattgcaaacaaccagggcactggaaaagggattgtcggctgataaacctccctctaggccaaactgtttcaccactagagggagcccaagagaccttagtcctcctgacaatattcaacttaaaggaggctctaagggattctccagtggattgctccccgtaatacctttaaaggaacatggggaaacagaggttaaaataaatagggagttgtgtatagtccttatggataccagggctactctatctaccataaaccccaccttaataagccaacaaatcccttagagtaaaaaggtcatttctgtgacaggggtttcaaatcaagttccagaggttcccatatctgaacccatccaattaactctgagccccctttcagaaaaacacagttttttactacgtgatactgttccagtaaacttggtagggcaagatttactttcaaagctaaaagggcacctaaaattttcctcagaaacagaaataatcttaagagttttcctgattctcctgaactagaattgttatgctgtctacaggcagaaattgataagatcgaaactcaagcctgtaatacccctgatctttcgaaaacacctaatgtttatgggcctcttcccaactgatataggaagaattaaaagtgtagaacctataaaagtactaacagatcattctaaacctttgcctaattaccacaatatccactaaaacctgaagcaatttaagggctctcaccaattgtagaagatttaattaaacaaggactcataattccatgcaccagcccctgtaacactccaatcctaccagttaaaaaacaaaatggatgagactggagatttgttccagatttacaggcaattaataaaattgtaataccaagatttcctgtagtcccaaatcctaatactttataacctaatgtacccactgattccaagttgtccacagtaatagatcttggctcagccttctctagcattccataaagaaagtcaatacttgtttgcctttacttggaaaaatcagcaatacacctggagtgtaatgccacaagggtttactgaagccccttcatattttccccaggcactgcatcaggagttaatgacactacagtttcctcaaaattctactctcattcagtatgtagataacttattgttatgctctcctattaaggagtgcccggaaattgactcagtttaccttttacagcaacttgcatataaaggtcacagggcttcaatggaaaaacttcaattttttcttttcttttttctttttttttttttttgagatggagtttcactcttgttgcccaggctggagtgcaatggtgtgatactggctcaccacaacctctgcctcctgggttcaagcgattctcctgcctcagcctcccgagtagctgggattacaggcatgcaccaccacgcctggctaattttgtatttttagtagagacagggtttctccatgttggtcaggctgtccttgaactcccgacctcaggtgatccgcctgcctcagcctcccaaagtgctgggattacaggcgttagccaccatgcctggccaaaacttcaattttcaaaagaaaaagtccactatttgggacatgacttggctgctgaagggatttccctcttacctgagaggataaaacctatttaaagttttcctcgacctgcaaccaaaagacaaaaggctttcttaggcttgcaggatattgcagatcctgggttccaaatttttccttaatagcttcaccactgtatgagctcactaaaaatgctgtaccagagcctttaccttgggaagacagtcatgagcaggcttttagccaaatgaagttggccttacaacagcccccagctttaggacttccaaattacactaaacctttcactttgtttgttcatgaatgtaataatcaggaacacggtgctaaacataggaccactgcatactatagcctgcaattaggcccagtctctaaggcatatcctaattgtttaaaagcagtagcagcagccaagctggtagaagcttcatcagatctggttttaggaaatgaacttaatttgcaagtcccacacgctgtggaaagtctattaaattccaatcaaacccagcatttttcagtgagtagactaacatcttatgaattacttctcctatctccttcttatcttcatctaaaaggctgtaatctacttaatgctgctactctgttatctctgcctgatgatggtgaagaccacaacggtgtgagtgtagtatcagaaatagtggcccctcgtgttgctatacaagatactccactggataatcctgaattaacactttttgttgatgggtcctatgccaaaaactcagaaaaaaaaatatcagtcaggatatgctgttaccacccaaaatgagttaatagagaagcgaactcttcaagtcaagtcagcccaacctgcagaactttctgcccttacctgaacatgtcacacagctaaggacaagtcagtaaatatttacggatagtagacatgcttttggagtagtacgtgattttggcatgatatggaaactacgaaggtttctcacctctagtgggatccccatcaaaaatggactccaaacagatgagctcctttctgctatcctgttacaaatgcagattgctgttattaagactgaagctcatacttgtagaaatgaacccaaatatcagtgaaatgctttagcagatttttatgctcaatcagctagtgctggaaccatcaagatacgcaatctgaatgaactccataagattaatccaagccaatttccttacgatgacctatttaataaacagtgcaacgcatctgatttgcaaaaacaaaactggtatctaaaaggatgtaaatttaacgtgaagcaaagactcacaaagggcccggacggccgcctggtccttcctgaatctttgaagcttccattattgaaagctctccacagctcatcatggaacagacaaagtgatccaaattatgaaaaaatactggtggggtgactattctgacattactaaaatggcttataatcaatgtttgacttgtcaaactcataatcccagaaaaactagaggcagtatatttccaccacctgatggaccatttgaacatttacagatggacttcattcagttaccaccctcaatggggtatcagtatgttcttgtaatagtttgcatgttttctggttggataaaggccttcccatgtaggaaagctgatgctgtgaccatagctaagaaattattagaaaatgtttttcctttatgggggatccctctaaaagtctccagtgatagaggaactcattttactgagcaagttataaagcagttaaataaggtgttactgacacagttgcattaccattgtccttattaccctcagtcttcaggaaagcttgaaagaacaaatggcatttgaaaactgaaactgtccaagttaactgaatcaattgagttgccttggccaaaggtactaccttttggttttaatggcaatcagattcaatcctgttggaaaacataaattgaccccttatgaaatagtcactgggaggcccatgtccctaataatagcatctcatgcttctcctgctctcttaaactctgatatgactaaatactgcaaggctttaatgtattacgccaaagtatacttccaccaggtaaaggaagcatttcaagatccaccaactgaggacaatcaaaccctccatggtctggaatttggagactgggccttccggaaatgacatcagaagaagatcactcttgaacctcgttggatgggaccataccaagtccttcttaccacccacagtgcagagaagcttcagggctttgaaccatgggtccacatctcacaattcaaaagggccccctcagactcctggtactatatacccgttggagactttaaggtaaagctgaccagggaaatctcttcccagaagcagacagcatcctggttacagacagctttccctagatcacagatcaagacttctctaccaccatgaaagccttatgtgtttttctgttttccttatttttttccctaatcctttccttttccttacatgaaaatccatgggaccataatcagtggatggcttcagctcaagcttatgctctagcacaaaaccagggtaactgttgggtttgtgggctaatgccaaaaaatcaggaaatgattccaagggtgccagtgcccctccacgtttcccaatgagtcaccctgaaaccccaagggaagaatggaaagctattcttgatactctaaacatcactagtacttgctttcctacactcactaaaaacaacactctttttcaactgataaagtcgatcacaccaaatataaaaaacaaatccaaatgatgcctacaaaacgtatattgtgcttgcaggcatcacatactcaagatttgggaattacttatgttagtacaagtgattgcttgtatatccagtagggtctctttttactagatgtggttatacacccttacaacacactacaaaggggccatagaaaagtaaatttcccactggatgttattcaggagctacagattcatggtcgaacaaacctgaatgatccctgctcaaatacaactaggtggcccccttttccaacccctgagggtctctattgggtctgtggagaatctgcatattctgttctgcctccttggttggtttggttcttgttatctggcctggcctgctcctgcctttcgaattgcttcccctgaaaattctcatgatagcccttatacttggaggccaaaatgatcaataactgaaattagcactagcctcgaaatagacgaggataagctagtttctaccggggaaagattccactggggttcctgggggctcactcttggtggtagtgaagtaccatttgtacggaatttaaaactaatttgtatattgggaaaattcttggatttggtagccaatcagacctcccagggtttcagatgggtagaagctactctcagaaaggcacatgacaacatacatattcaacgaaaacacttaatggaagatcatgcagtcttagatcttctttttgctcaagctggaggcctatgtttggtgttaaacaaaactgaattttgtactaatccctcccctgattctgttactacaaaaagcttaatttaaaaggtggctgatactgctgtttccttagacactgccaccaagtacaataaagaaatctctcaagagaaaggaacccacgatatgtttataggagcaactaacagttggtttgcaggcatcctaagtggtgaatggcaagcttgggttttccaagggtttctaatctttatatctcttctagcaggttttcaagttattatgacttgtattaacaaggtaacaatgaaaacgagcacctctttaagtcaagctactttacagcgaactatgatccttaatcactatcatactccaactgaagactctgaccaatcagaccccaatactgctgaactgcttatattgtctgaaccttaacttggctgatttggttcagttcatttcataagaacttttattaaggagtacaccttagcattttgacggtgtcctcttaacagtcataataatagtccccttggtgcactgtatactctcaagtcttaaatgttttgtatgcagctgtacattgacagttgaatggtcttactccaactggatcagcaagaacataaagaatcatttagctggtacaaagttgcaacttgtgaattccctattaacaccaaagaagatgtgtgagactccatactgaaactaaagacgacttgtgagttccacactgagaccaaataagtctttatgatggtgacagagagtggtgtcaacgcctaaagttttggtcaatctctctaaattgaggggctgaccaaaagggggaattgttaaagcgaactaaatatggcccgaagaggactccgtacttttatatttgagtccttgtggacgaactgtaacctagctcaaataggcagacaaaatcgaaaacctaacttagtagtatgcatctgtaataacagctgagtgttggccaatcccagcggccatacttcaaccactcatagactgctgagtgttcaaactgcgttc

SEQ ID NO: 10 - DNA, 7060 bp, Homo sapiens
tgggtgacaggacaaggttgatatttttccttcctttgcttttctgtaccatctaagttgcacaatctaacaatcacatggctggtgcaggggctcatgcttataatcccagcactttgggaggctgaggtgggaggatcactggagcccagaagttcaagatcagcctgggcaacatagcaagaccctgtctctacaaaaaataaattagccaggcatggtaacacatgtgtgtggtcccagctactcaaggtgggaggactgcttgagcctaggagttcatggctgcagtgtgccgtgatcatgctactgcactccagcctgggcaacaaagcaagaccctgtctcaacaaaataaaacaaaacaatcacagattgcttttttcacataggggcaggaaatctttacatttttacttatttttgttttaacgcaagctctttggagtgtttcctatactgtctctcacacatgggaattatctgtaaatcacggtttaaattaaggttttctttttaattttagaattgcatttttcttttccctctctgttcctcagcctctcatcactatgcccagacctccagagagcacgcctccagtcttttttctgttcacagctgttatttcccagctgcctacagtcacttcacaatgactcacacttcttgaagtattggccctaacacagatgcccagacagcagctgcagtggcagcacaccctcaccacagctggtacccacactgaacttagtgtgggagactctcccaggaacaggatctgaaaaagggcagcaaaggcttttaagctgtaactgttctgacctgggcacaccccagcaagttcactggcttgcaacttgattccaatgggatgacaatggcagatgcgagacctgcctggtaaggcagctggcaaggcagctggccacactgtaccacagtccccagcttggattaggatcaggagcttgacaactcctggttgcaatacacaatctaacagccattggaggaaaaaaaaggcctccttaatgtacttcatttctttgcccagtaataagctattacatagggtaaatctgatttctgctttcatctttgcattgggtcaagacaaaataactctttttgtttttcttcataactagaatgaaaaaaaaaaaacaaaaacaagaattgagcagggtaatgggaggaaagaacaaagtagaggcatttatgatgaaataatacagtttgtctacttgaatccatttctagcgtaaacctctgcttaccccatcttcaacattctccagtaaagctagaaatttttttgttctttttctcttctgataactttccctcaacccatcatattactgtcaggcctctgagcccaagctaagccatcatattcccagtgacctgcacgtatacatccagatggcctgaagcaactaaagatccacaaaagaagtgaaaagagccttaactgatgatattctaccattgtgatttgtttctgccctaccctaactgatcaatatactttgtaatctcccccacccttaagaaggttcttcataatctcccccacccttaagaaggttctttgtaattctccccgcccttgagaatgtgcgagatccaccccctgcccccaaaacattgctcttaactccactgcctatcccaaaacctgtaagaactaatgataatcccaccaccctttgctgactctcttttctgactcagcctgccggcacccaggtgaaataaacagccttgttgctcacacaaagcctgttttgtggtctcttcacatgcacatgtgagacatttggtgccgaagacccaggtcagcgggactccttcgggagaccagtcccctgtcctcaccctcactccgtgaagagatccacctatgacctcaggtcctcagactaaccagcccaaggaacatctccccaattttagatcaggtaagcagcctctttttactctcttctccaacctctctcactatccctcaacctctttctccttttaatcttggcgccacccttcaatctctcccttctcttaatttcaactcctttcattttctggtggagacaaaggagacatattttatccattgacccaaaactccagcgccagtcacggactcgggaaggcagacttcccttggtgtttaatcattgcgaggacgcctctctgattattcacccacgttccactggtgtctgatctccgtggggacgtctgccttggtcattcatccacattcccttggtggcaagtcaagtgcggagacgcctgctttggctgctccccaccccccttctccgtgtctctacccttctctttaaacttgcctccttcactatgggcaaccttccaccctccactcctccttcttctcccttagcctgtgttctcaagaacttaaaacctcttcaactctcacctgacctaaaatctaagcgtcttattttcttctgcaatgccgcttgaccccaatacaaactcgacagtggttccaaatagccagaaaacggcactttcgatttttccatcctacaagatctaaataattcttgtcgtaaaatgggcaaacggtctgaggtgcctgatgtccaggcattcttttacacactggtccctccctagtctctgctcccaatgagagtcgtcccaaatctttcttctttctctcctgtctgttccttcagtcctaaccccaagcgtctctgagtcttttgaatcttccttttctagggacccatctgacctctctcccctcctccccaggctgctccttgccaggccaagccaggtcccaattcttcctcagcctctgcttccccaccctataatccttctatcacctcccttccccacacccagtctggtttacagtttcgttccatgactagccctccccgacctgcccaacaatttcctcttaaagaggtggctggagctaaaggcataatcaaggttaatgctccttttttctttatctgacctctcccaaatcagttagcatttaggttctttttcatcaaatacaaaaactcaacccaattcaaggcctgtttgacaacaacccttagacgctttaccaccctagacccagaggggccagaaggctgccttattttcaatatgcattttattacccaatccgctcccgacattagaaaaagctccaaaaagcccctctgcctggccggccgccccgacggggacggaggtgggggggggtcagccccccgcccggccagccgccccatccgggaggtgaggggcgcctctgcctggccgcccctactgggaagtgaggagcccctctgcccggccaccaccccgtctgggaggtgcgcccaacagctcattgagaacaggccatgatgacagtggcagttttgtggaatagaaaggggggaaaggtggggaaaagactgagaaatcggatggttgccgtgtctgtgtagaaagaggtagacatgggagacttttcattttgttctgtactaagaaaagttcttctgccttgggatcctgttgatctgtgaccttacccccaaccctgtgctctctgaaacatgtgctgtgtccactcagggttaaatggattaagggcggtgcaagatgtgctttgttaaacagacgcttgaaggcagcatgctcgttgagagtcatcaccactccctagtctcaagtgcccagggacacaaacactgcggaaggccacagggtcctctgcctaggaaaaccagagacctttgttcacttgtttgtctgctgaccttccctccactattgtcctgtgaccctgccaaatccccctctacaagaaacacccaagaatgatcaataaaaaaataaataaataaataaataaataaataaataaataaataaaataaaaaagaaaaaaaaaaagaaaaagctccaaaaattagactctggccctcaaaccccacaacaggacttaattaacctcgctttcaaggtgtacagtaatagagtaatggcagccaagtagcaatgtatttctgaggtgcaattccttgcctccactgtgagacaaaccccagccacatctccagcacacaagaactccaaacgcctgaaccacagttgccaggggttcctctagaacttcctcccccaggatcttgcttcaagtgccggaaatctggccactgggccaaggaatgcccgcagcccgggattcctcctaaaccgtgtcccatctgtgcaggaccccactggaaactggactgtccaactggcccaaggctctgattgactccttcccagatcttctcggcttagtggctgaagactgacactgcccaatagcctcggaagccccctggaccatgatggaggccaagcttcgggtaactcttacagtggagggtaaatccgtccccttcttaatcattatggaggctactcactccacattaccttattttcaagggcctgtttcccttgcctccataactgttgtgggtattgacggccaggcttctaaaccccttaaaactccccaattctggtgccaacttggacaatattcttttatgcactcctttttagttatccccacctgcccggctcccttattaggtcgagacttttaactacattatctgcttccctgattattcctgggctacagctgtacctcactgccaccttttgccccagttcaaagcctccttcacatcctctccttgtatctccccttcttagtccacaagcataggacacctctactccctccttgacaacaaatgatgcaccctttaccatcccattaaaacctaatcacccttatcctgctcaatgccaatatcccatcccacagcatgctttaaaaggattaaaacctgttgtcacttgcctgttacagcatggccttttaaagcctgtaaactctccttacaattcccctgttttacctgtccaaaaaccagacaaggcttttacaggttagttcaggatctgcaccttatcaactaaattgtcttgcctatccacccagtggtgccaaagtcatatactctcctatcctcaatacctccctccacaacccctccataactcattattctgttctggatctcaaacatgctttctttactattcctttgcacccttcataccagcctctcttcgctttcacttggactgaccctgatacccatcaggctcagcaaattacctgggctgtactgctgcaaggcttcgtggacagcccctactacttcagtcaagcccaaatttcttcctcatccattacctatcttgacatatttcttcattaaaacatacgtgttctccctgctgattgtgtccaactaatctcccaaaccccaaccccttccacaaaacaacaactcctttccttcctgggcatgtttggatactttcacctttagatagcctcggaagccccctggaccatcacggatgccaagctttgggtaactcttacagtggaaggtaaatccgtccccttcttaatcaataaggagactactcactccacattaccttattttcaagggcctgtttcccttgcctccataactgttgtgggtattgacggccatcctaacaaaaccattatataaactcacaaaaccaaacctagatgactccatagatcctaaatcctttcaccactcctctttctgttccttaaaaacagccctagaagctgcccccacactagctctccctaactcatcccaacccttttcattacacacagccaaagtgcagggctgtgtggtcagaattcttacacaagaaccaggaccacgccctgtagcctttctgtccaaacaacttggccttactgttttagcctagccctcatgtctgtgtgcagtggctgctgccgccctaatacttttagaggccctcaaaatcacaaactatgctcatctcactctctacagttctcataacttccaaaatctattttcttcctcacatctgacacacatactttctgctccctggctccttcagctgtactcactctttgttgagtctcccacacttaccattgttcctggcctggacttcaatccggcctcccacattattccggataccacacctgacccccatgactgtatgtctctgatccacctgacattcactccatttccccatatttccttctttcctgttcctcaccctgatcacatttggtttactgatggcagttccaccaggcctaatcaccactcaccagcaaaggcaggctatgctatagtatctcccacatctatcattgaggctaccgctctgcctccctccactatctctcagcaagccgaactcattgccttaattcaagccctcactcttgcaaagagaccacgtgtcaatatttatattgactccaaatatgccttccatatcctgcatcaccatgctgttatatgggctgaaagaggtttcctcactatgcaagggtcctccatcattaatcctctttaataaaaactcttctcaaggccgctttacttccaaaggaagctggagtcatacactgcaaggaccaccaaaggacatcagatcccatggctcagggcaacgcttatgctggtaaggtagctaaagaagcaggcagaattccaacttctgtccctcacggccagtttttctccttctcatcgatcacttccacctactgccctgctgaaacttccatctatcaatctcttcccacacaaggcaaatggttcttagaccaaggaaaatatctccttccagcctcacaagcccattcttttctgtcgtcatttcataacctcttccatgtaggttacaagccactagcccgtctcttagaacctctcatttcctttccgtcgtggaaatctatcctcaaggaaatcacttctctgtgttccatgtgctattccactacccctcagggattgttcaggccaaccccccccaccccacccttccctacacatcaagctcagggattttcccccgcccaggactggcaaattgactttaccca

SEQ ID NO: 11 - DNA, 6229 bp, Homo sapiens
gtatacatccagatggcctgaagcaactgaagatccacaaaagaactgaaaacagccttaactgatgacattccaccattgtgatttgttcctgccccaccctaagtgataggctatgttctcccccgcccttaagaaggtactttgtaatattctcccccgcccttaagaatgtactttgtacacctatcccaaacgtataaaaactaatgataatcccaccaacctttgctgactcctttctcggactcagcccacctgcacccaggtgaaataaacagccctgttgctcacacaaagcctgttggtggtctcttcacaaggatgcgtgtgacatttggtgccaaaacccaggacaggaggactccttcaggagaccagtcccctgtcttcgccctcactccgtgacctcaggtcctcagaccaaccagcccaaggaacatctcaccaacttcaaattgggtaagcagtcttttcactcttctcatgcctctcttgctacccttcaatcttcctctcttgctacccttcaatctccctgtccttccaattccaattctttttcctctctagtagagacaaggagacggccaggtgcggtggctcacgcctgcaatcccagctctcagggaggctaagaggcgggaggatagcttgagcccaggagttcgagacctgcctgggcaatatagcgagaccccgttctccagaaaaaggaaaaaaaaaaaaaaagagacaaggagacacattttatccgtggacccaaaactctggcgccagtcacggactcgggaagatagtcttcccttggtgtttaatcactgcggagatgcctgcctgattattcacccaccctccactggtgtctgatcactgcggggacacctgccttagtcattcacccacattcccttggtggcaagtcaattgcagggatgcctgctttggctgctcacccacattgcagcccagggctgctcacccacccacttctccatgtctctacctttctctttaaacttacctccttcactatgggcaaccttccactcgccattctcccttcttctcctttagcctgtgttctcaaaaacttaaaacctcttcaactcacacctgacctaaaacctaagcgtcttattttcttctacaacaccgcttggccccaatacaaacttgacaatgattccaaatagccagaaaatgacactttcgatttctccatcctacaagatctagataattcttgtcataaaatgggcaaatggtctgaggtgcctgacgtccaggcattcttttacacatcggtcccttcctaatctctgttcccaatgagattcatcccaaagctttcttctttctctcctgtctgttccttcagtctccaccccaagctctgaatcctgggaatcctccttttctacagacccatctgacctctaccctcctccccaggctgctccttgccaggccgagccagctcccaactcttcttcaacctctgctcccccaccctataacccttctattacctcccctcctcacacccggtctggcttacagtttcattccgtgaccagccctcccccacctgcccaacaatttcctctcagagaggtggctggagctgaaggcatagccaaggttaatcctcctttttctttatccaacctctcccaaatcagttagcgtttaggctctttttcatcaaatatgaaaacccagcccagtccatggcccgtttggcaacaacccttagatgctttaccgccctagacccagaggggccagaaggctgtcttattctcaatacacattttattacccaacccactcctgacattagaaaaatctccaaaaattagattctggccttcaaccccccaacagtacttaattgacctcaccttcaaggggtacagtaatacagaagagttgtaattacttgcctccgctgtgagagaaaccccagctacatctccagcacacaagaacttcaaaacgcctaaacctcaggggtcaggcattcctccaggaccgcctccccaggatcttgcttctagtgctggaaatctggccactgggccaaggaatgcctgcagcctgggattcctcctaagccgtgtcccatctgtgcaggaccccactggaaatcagactgtccaactcacccagcagccactcccagagcccctggaactctggcccaaggctctctgactgactccttcccagatcgtctcagcttagcggctgaagactgacactgcccgatcgcctcggaagcctacaggaccatcacagatgctctggataactcttacagtggagggtaagtccatcctcttctttatcaatacggaagctacacactccacattaccttctttccaagggcgtgtttcccttgcctccataactgttgtgggtattgacagccaggcgtctaaacctcctaaaactccccaactctggtgccaacttggaaaacattcttttatgcactcctttttagttatcctcacctgcccagctcccttattaggttgagacattttaactaaattttctgcttccctgactattcctgggctacagccacacctcattgcctccttttcccccagttcaaagcctccttcacatcctctccttgtatctccccaccttaatccacaagtataggacacctctactccctccttggcaacggatgatgcaccccttaccatcccattaaaacctaatcacccttaccctgctcaatgccaatatcccatcccacagcacgctttaaaaggattaaagcctgttatcactcacctgctacagcatggccttttaaagcctataaactctccttacaattccccattttacctgtccaaaaactacacgagtcttacaggttagttcaggatctgcaccctatcgaccaaattgtcttgcctatccaccctgtggtgccaaagccatatattctcccatcctcaatacctccctccacaacccattattctgttctagataaacctagctgaccccataaatcctaaatcctttccccactcccctttccattccttaaaaaacagccctaaaagatgctcccacactacctctccctaactcatcccaacctttttcattacacacagctgaagtgcagggctgtgtggtcggaattcttacacaagagccgggaccgcgccctggagcctttctgtccaaacaacttgaccttactcttttagcctagcccttacgtctgcgtgtggtggctgccgctgctttaatacttttagaggccctcaaaatcacaagctatgctccacttactctctacagttcccataactttcaaaatctattttcctcctcacacttgacgcatatactttctgccccccagctctttcagctatactcactctttgttgagtctcccacagttactattgttcctggcccagacttcaatccggcctcccacattattccggataccacacctgatccccatgactgtatctctctgatccacctgacattcactccatttccccatatttccttctttcctgttcctcaccctgataacacttggtttattgatggcagttccaccaggcctaatcgccactcaccagcaaagggaggctatgctatagtatctttcacatctatcattgaggctaccactctgaccccctccactacctctcagcaagctaaactcattgccttaacttgggccctcattcttgcaaaaggactacgagtcaatatttatactgactctaaatatgccttccatatcctgcaccaccatgctgttatatgggcagaaagaggtttcctcactactcaagggtcctccatcattaatgcctctttaataaatactcttctcaaggctgttttacttccaaaggaagctggagtcattcactgcaagggccatcaaaaggcatcagatcccactgctcagggcaacgcttatgctgataaggtagttaaagaagcagctagctttccaacttctgtccctcacggccaggactggacagtactttgcccttctcagaattagagcctgtcctcgagatgctacagggtactgtccatttgaacttttatatggacgcactttcttgctcagccctgacctcgtcccagacaccagccctctaggcaactatcttccagtcctccagcaggctagacaggaaattcgctaggctgctcatcttctcttgcctactccagattcccagccatatgaagacaccctagctggatgatcagttcttgttaagaatctgacccctcaaactctacaacctccatggactggaccccacttagtcatctatagtaccccaatggctgttcgtctgcaggatgccccaccattaggttcatcattccagaataaagctgtgcccgtcaaacagccagcctgatctctcctcttcctcctggaagtcacaagtgttcacccctactttccttaaacttatttgcatttctgaagagcagtaataacccttatgagcctaatacaacccttcattctattaggtctattcatccttaccctactttttgcaatagggctttacgcagtcacccccactacttgttctgtgccccaaaaacttgtcatccctatcttctgtctagtcatactcctattcaccattctcaactacttgtaaatgccctgcccttgtttacactgctggtttacgcttttcctccaaaccattgtagcggatatctcctggtactatccccaatccgccactcttgactccctcttagagtggatagatgaactttgctgacagggcaccctccgatacttttaccctgatgaagtcctattctttacttttatactcactcttattctcattcccattcttatgccatcctctacctctccccagctatctccaccacactatcaatctcactcactctctcctagctgtttctaaaccttctttaacaaacaattgctggctttgcatttctctttcctctaaaatcacagaggcctcgacttactcactgctaaaaaaaaaaaaaaagggggactctgggccaggcgcagtggctcatgcctgcaatcccagcactttggaacactgaggtgggcagatcacgaggtcaggagatcgagaccatcctggctaacacagtgaaattctgtctctactaagaatacaaaaacttagctgggcgtggtggcgggtgcctgtagtcccagcttcttgggaggctgaggcaggagaatggtgtgaacccggaaggcggagcttgcagtgagccgagatcacgccactgcactccagcctgggcaacaaagcaagagtctgtctcaaaaaacaaaaacaaaaacaacaaaaaacattttttaaatgaagagtgttgtttttacctaaatcaatctggcctggtatatgacaacataaaaaaactcaaggatagagccccaaaactcgccaaccaatcaaataattacgctgaacccccttggacactctctaattggatatcctgggtcctcccaattcttagtcctttaatacctgtttttctccttctcttattaggaccttgtgtcttccgtttagtttcccaattcttacaaaaccgcatccaggccatcaccaatcattctatatgacaaatgctccttctaacaaccccacaatatcaccccctaccccaaaatctttcttcagtttaatctctcccactgtaggttcccatgccacccctaatcctgctcgaagcagcccagagaaacattgctcattatctctccacatcgcccctaaaaaattttcgccaccccaacacttcaccaccattttgttttgtttttcttattaatataagaagacaggaatgtcaggtctctaagcccaagctaaatcatcatatcctgtgacctgcatgtatacatccagatggcctgaagcaactgaagatccacaaaagaactgaaaatagccttaactgatgacattctaccattgtgatttgttcctgccccaccctaactgataggatatattctacccccccacttaagaaggtgcttcgtaatattctccccgcccttgagaatgtactttgtacacctatcccaaacctataagaactaatgataatcctgccaccctttgctgactcctttttcagactcagccca

SEQ ID NO: 12 - DNA, 7085 bp, Homo sapiens
tgaaaaaaagccagacacaaagtgtcaggcctctgagcccaagctaagccatcatatctcctgtgacctgcacgtacacatccagatggctggttcctgccttaactgatgacattccaccacaaaagaaatgaaaatggcctgttcttgccttaactgatgacattatcttgtgaaattccttctcctggctcatcctggctcaaaagctcccctactgagcaccttgtgacccccactcctgccagagaacaacccccctttgactgtaattttcctttacctacccaaatcttacaaaacggccccaccccatcttccttcactgactctcttttcagactcagcccgcctgcacccaggtgaaataaacagccttgctgctcacacaaagcctgcttgttggtctctttacacagatgcgcatgaaatttggtgctgtgactcggatcggggggacctcccttgggagatcaatcccctgtcctcctgctctttgctccgtgaaaaagatccacctacgacctcgggtcctcagacccaccagcccaaggaacatctcaccaattttaaatcaggtaagccgcctcttcttaatctcttctccaacctctctcactatccctcaaccactttctcctttcaatcttggtaccacccttcaatctctcccttctcttaagttcagttcctttccttttctggtagagacaggagacgcgttttatccgtggacccaaaactccggcgctggtcacagactagggaagacagtcttcccttggtgtttaatcacgtggggacgactgcctgattactcacccacgtttcagaggtgtctgaccacacggggacgcctgccttggtccttcacccttagcagcaagtactgcttttctggggggcaagaacctcccaactccttctctctgtgtctctaccccttctctgctttttcaggggggcaagaaccccccaaccccttctccttcacccttagtggcaagtaccacttttctagggggcaagaaccccctgatcccttatttccatgccccaacctcttatctctgtgccccgatcccttaattccatgccctgacctcttatctttgcaccccaatcccttatttccatgccctgacttcttatctctgcaccccatcccttatttccacgccccaacctcttatctctgcgccctgatcccttatttctgtgccctgacctcttatctctgcaccccaaccccttatatctccatgccccgacccctttcctgcttttctggaaggtaagaacccccaaaccccttccctccgtgtctctactctgttctctgggcttgcttccttcactatgggcaaccttccaccctccattcctccttcttctcccttagcctgtgttctcaagaacttaaaacctcttcaactcacacttgacctaaaacctaaacaacttattttcttctacaatgccgcttgaccccaatacaaactcaacagtggttccaaatagacagaaaacggcactttcgatttttccatcctacaagatctagataattcttgttgtaaaataggcaaatggtctgaggtgcctgacgtccaggcattcttctacacgttgttccctccctagtctctgttcccaatgtgattcctccccaatcctccttctttccctcctggctgtcccctcagtcccaaccccaagcgtcgctgagtctttccagtcttccttttctacagacccatctgacctttcccctcctccccaggctgcttgtcgccaggccgagctaagtcccaattcttcctcagcctcagctcctccaccctataatccttctatcatctcccctcctcacacccagtctggcttacagttttgttccgcgactagccctcccctacctgcccagcaatttcctcttaggaaagtggctggagctaaaggcatagtcaaggttaatgctcctttttctttatccgacctctcccaaatcagttagcctttaggctctttttcatcaaatatgaaaaacccagcccagttcatggctcgtttggcagcaaccctgagacgctttacagccctagaccctaaaaggtcaaaaggccatcttattctcaatatacatttgattacccagtcagctcctgactttaaataaagctccaaaaattaaattccggccctgaaaccccacaacaggacttaattaacctcgccttcaaggtgtacaataatagaaaaaagttgcaattccttgcctccactgtgagacatatcccagccacatcaccagcacacaagaacttccaaacacctgaaccacagcagccaggagttcctccagaacctcctccccaagaagcttgctacaagtgccggacatctggccaccgggacaaggaatgcccgcagcccaggattcctcctaagccgtgtcccatctgtgtaggaccccactgaaaatcagactgttcaactcacctggcagccactcccagagcccctagaactctggcccaaggctctctgagtgactccttcccagatcttctcggcttagcagctgaagactgacactgcccgatcgcctcggaagccccctaaaccatcacggacgccgagcttcaggtaactctcacagtggaaggtaagtccgtccccttcttaatcgatatggaagctacccactccacattaccttcttttcaagggcctgtttcccttgcctccataactgttgcaggtactgacggccaggcttctaaacctcttaaaactccccaactctggtgccaacttagacaatactcttttaagcactcctttttagttatccccacctgcccagttcccttattaggccgacactttaactaaattatctgcttccctgactattcctgggctacagccacacctcatcgctgccttttcccccagttcaaagcctccttcacatcctccccttgtatctccccatcttaacccacaagtataagacacccctactccctccttagtgaccgatcctgcaccccttaccatcccattaaaacctaatcacccttaccctgctcaatgtcaatatcccatcccacagcacgcttcaaaaggattaaagcctgctattactcgcctgctacagcatggccttttaaagcctataaactccccttacaattcccccattttacctgtcctaaaaccagacaaggcttacaggttagttcaggatctgcgccttatcaaccaaattgttttgcctatctaccccgtggtgccaaacccatatactctcctatcctcaatacctccctccacaacccattattctgttctagatctcaaacatgctttgtttgctattcctttgcacccttcatcccagcctctcttcgctttcacttgtactgaccctgacacccatcaggctcagcaaattacttaggctgtactgctgcaaggcttcacagacagcccccattacttcagtcaagcccaaatttcttcctcatctgttacctatctcagcataattctcataaaaacacacgtgctctccctgattatcgtctccggctaatctcccaaaccccaatcccttctacaaaacaacaactcctttccttcctaggcatggttagtaaggtcagaattcttacacaagagctgggaccacgtcctatagcctttctgtccaaacaactggaccttactgttttaacccaaccctcatgtctgcatgcagcggctgccgctgccttaatacttttaaaggccctaaaaatcacaaagtatgctcaactgactctctacagttctcataacttccaaaatctattttcttcctcatacctgatgcatatactctctgctccctggctccttcagctatattcactctttgttgagtctcccacaattaccattgttcctggcacggacttcaacccggcctcccacattattctggataccacacctgaccctcatgactgtatctctctgatccacctgacattcaccccatttccccgtatttccttctttcctgttcctcaccctaatcacatttggtttattgatggcagttccaccaggcctaaatgccactcaccagcaaaggcaggctatgctatagtatcttccacatctatcattgaggctaccgctctgcccccctccactacctctcagcaagccgaactagttgccttaacccaagccctcactcttgcaaaaggactatgcgtcaatatttatactgactctaaatatgcctttcatatcgtgcaccaccatgcaagaagtttcctcactaaacaagggtcctctatcattaatccctctttaataaaaacgcttctcaacgccgcttaacttccaaaggaagctagagtcattcactgcaaggggcatcaaaaggcatcagatcccattgctctaggcgacgcttacgctgattaggtggctagacaagcagctagcattccaacttctgtccctcacagccagtttttctccttcacgtcagtcactcccacctactcccccactgaaacttccacctatcaatctcttcccacagaaggcaaatggttcttagaccaaggaaaatatctccttccagcctcacaggcccattctattctgtcgtcatttcataacctcttccatgtaggttacaagccgctagcccgtctcttagaacctctcatttcctttccatcctggaaatctatcctcaaagaaatcacttctcagtgttccatttgctattctactacccctcagggattgttcaggcctcctccctttcctacatatcaagctcggagatttgcccctgcccaggactggcaagttgactttactcacgtgccccgagtcagaaaactaaaatacctcttagtctaggtagacgctttcactggatgggtagaggcctttcctacagggtctgagaaggccaccgcggtcattttttcccttctgttagacataattcctcggtttggccttcccacctctatacagtctgatagcagaccggcctttattagtcaaatcagccaagcattttttcaggctcttggtattcagtgaaacctttatttcccttacggtcctcagtcttcaggaaaggtagaatggactaacggtcttttaaaaacacacctcaccaagctcagccaccaacttaaaaaggactagacaatacttttaccactttcccttctcagaattcaggcctgtcctcagaatgttacaaggtacagctcatttaagctcctgtatagatgctcctttttattaggccccagtatcattccaagaccaacttggactgtgccccaaaaaacttgtcatccctactatcttctgtctaatcatactcctattcactgttctcaactactcacacatgccctgctcttgtttacactgctggtttacactgtttctccaagccatcacagctgatatctcctggagctatccccaaactgccactcttaactcttgaagtaaataaataatctttgctggcagaactatgctgaacctccttaggcactctctaattaaatgtcctaggtcctcccaattcttagtcctttaatacctgtttttctccttctcttattccatttagtttttcaattcatacaaaaccgtatctaggccatcaccagtaattctaaatgacgaacgtttctcctaacagtcccacaatatcaccccttaccacaaaatcttccttcagcttaatctctcccattctaggttcccacaccgcccctaattccgctcgaagcagccctaagaaacatcgcccattatctctccgtaccatcccccaaaattttcgctgtcccaacacttcaccactattttgttttatttttcttattaatataagaagacaggaatgtcaggcctctgagcccaagctaagccatcatatctcctgtgacctacacgtacacatccagatggccggttcctgccttaactgatgacattccaccacaaaagaaatgaaaatggcctattcttgccttaactgatgacattatcttgtgaaattccttctcctggctcatcctggctcaaaagctcccctactgagcaccttgtgacccccactcctgcccgccagagaacaacccccctttgactgtaattttcctttacctacccaaatcttataaaacagctccaccccatcttccttcactgactcttttcagactcagcccgcctgcacccaggtgaaataaatagccttgttgctcacacaaagcctgtttggtggtctctttacacagacgtgcatgaaacaaaggtcatatatgattcctttttacatgaaatatctataaatccatagaaacagaatgcatactggtggttgccaggggctagggagagagggcaatggagacaaactgtttaatggataagtggttttacttgagagtgatggaaatgctttggaactagatagaggtagtggttgcacaacataacgaatgtacaaaatttctctgaattgctcactttaaagtggttattttgtctgggtgcggtggctcatgcctgtaatcctaacattttggtgggccaaggcgggctgatagcttgagctcaggagtttgagaccagcccaggcaataaggcgaaacccctgtctctataaaaaatacaaaaattagctgggcgtagtggtacgtgcctatagtcccagctacttgggggctgaggcaggaggatcacttgaatccaggaggttgaagctgcagtgagccctgatcacaccactgcactccagcctgggtgacaaagtgagactctatctccccccacaaaaaaagggttaattttatgctatgtgtatttcacctcaataaattgtttttaaaaatcagatgacgggactgattacaggttaaaaggtaaggtcttgtttcagatatgctgaaattgagattttgggaagatatccaggtagagatttctagaagatagctggaaatataagtctggaataaggggagagg

SEQ ID NO: 13 - DNA, 6924 bp, Homo sapiens
tgtcaggcctctgagcccaagctgagccatgatattccctgtgacctgcacgtacacatccagatggccagttcctgccttaactgatgacattccaccacaaaagaagtgaaaatggcctgttcctgccttaactgatgacaatgtcttgtgaaattccttctcctggctcatcctggctcaaaagctcccccactgagtaccttgtgacccccactcctgcccgccagagaacaaccccctttttccttcacctatccaaatcctataaaacggccccacccccatctcccttcgctgactctcttttcggactcagcccgcctgcacccaggtgaaataaacagccatgttgctcacacaaagcctgtttggtggtctcttcactcagacacgcaggaaatttggtgccgtgacttggattgggggacctcccttgagagatcaacccctgtcctcctgtcctttgctccgtgagaaagatccacctacgacctcaggtcctcagacctaccagcccaaggaacatctcaccaattttaaatcgggtgagcggcctcttcttactctcttctccaacctctctcactgtccctcaaccactttctcctttccactcttcaatctctcccttctcttaatttcaattcctttcattttctggtagagacaaaggagacacgttttatccgtggacccagaactctggcaccggtcaaggactagggaaggcagccttcccctggtgttgaatcattgcagggatgcctctctgattatttacccatgtttcagaggtgtcagaccatgcagggacacctgcctttgtccttcatccttagcggcaagttccgcttttctgtgggaggggcaagtaccccaaccccttctctccgtgtctctacaccttctctgcctttctggggggcaagaaacccccaaccccttcttcttcacccttagcagcaagtcccgcttttctaggggagggataattaccccaaccccttatatctctgtgccctgatcccttatttccgtgccccaagctcttatatctctgcaccccaatcccttatttccatgccccaacctcttatatctctgcaccctgatcccttatttcctcgcccaacctcttatatctctgtgccccaatcccttatttccgtgccctgacctcgtatctctgtgccccatcccctttcccacttttctggagggtaagaacccccgaaccccttccctccgtgtctctactctctcttttctctgggcttgcctccttcactatgggcaaccttccaccctccattcctccttcttctcccttagcctgtgttcttaagaacttaaaacctcttcaactctcacctgacctaaaatctaagcatcttattttcttctgcaatgccacttgaccccaatacaaactcgacagtagttccaaatagccagaaaacggcactttcgatttttccatcttacaagatctaaataattcttgttgtaaaatgggcaaatgatctgagatgcctgacgtccaggcattcttttacacatcggtccctctctagtctctgttcccaatgcaactcatcccaaatcttccttctttccctcctgtctgtcccctcagtcccaaccccaagcgtctctgagtctttctaatgttccttttctacagacccatctgacctctcccctcctccccaggctgctcctcgccaggccgagctaggtcccaattcttcctcagcctccactcctccaccctataatccttttatcacacctcccctcctcacacctggtccggcttacagttttgttccatgactagccctcccccacctgcccagcaatttactcttaaaaaggtggctggagctaaaggcatagtcaaggttaatgctcctttttctttatcccaaatcagacagcatttaggctctttttcatcaaatataaaaatccagcccagctcatgactcgtttggcagcaaccctgagatgctttacagccctagaccctaaaaggtcaaaaggccgtcttattctcaaaatgcattttattacccaatctgctcccgacactaaataaaactccaaaaattaaattccggccctcaaaccccacaacaggatttaattaacctcgccttcaaggtgtacaatagtagaaaaaagttgcaattccttgcctccactgtgagacaaaccccagccacatctccagcacacaagaacttccaaatgcctgaaccgcagcggccagacatttctccagaacctccttccccaggagcttgctacaagtgccagaaatctggccacaaggccaaggaatgcctgcagcccaggattcctcctaagccgcgtcccatctgtgcgggactccactggaaatcggactgtccaactcacctggcagccactcccagagcccctggaactctggccgaaggctctctgactccttcccagatcttcttggcttagtggctgaagactgatgctgcccaatcgcctcgaaagccccctagaccatcacggacgctgagcttcaggtaactcacacagtggagggtaagtccgtccccttcttaatcaatacggaggctactcactccgcattaccttattttcaagggcctgtttcccttgcttccataactgtggtgcgtattgacagccaggcttctaaacctcttaaaactccccaaatctggtgccaattagacaatactcttttaagcattccttttagttatccccacctgcccagttcccttattaggctgagacactttaactacattatctgcttccctgactattcctggattacagttacatctcatggctgcccttcttcccaatccaaagcctcctttgcgtcctcctcttgtattcccccaccttaacccacaagtataagatacctctactccctccttggcaaccgatcatgcaccccttaccatctcattaaaacctaatcacccttaccccgattgatgccaatatcccatcccacagcatgctttgaaaggattaaagcctgttatcactcgcctgctacagcatggccttttaaagcctataaactctccttacaattcccccattttacctgtcctaaaaccagacaagcctttcaagttagttcaggatctatgccttatcaaccaaattgttttgcctatctaccccatggtgccaaacccatacactctcctatcctcaatacctccctccacaatccattattctgttctggatctcaaacatgctttcttcactactcctttgcacctgtcatcccagcctctcttcgctttcacttagactgaccctgacacccatcaggctcagcaaattacctgggctgtactgccgcaaggcttcacagacagcccccattacttcagtcaagcccaaatttcatcctcatctgttacctatctcggcataattctcataaaaacacatgtgctttccctgctgattgtgtccgattaatctcccaaacctcaatcccttacaaaacaacaactcctttccttcctaggcatggttagtgcggtcagaattcttatacaagagccaggaccacaccctgtagcctttctgtgcaaacaacttgacctgttttagcctagccatcatgtctccgtgcagtggctgctgccgccctaatacttttagaggccctcaaagtcacaaactatgctcaacttactctctacatgtctcataacttccaaaatctattttcttcctcatacctgacacatatactttctgctccccagctccttcagctgtactcactctttgttaagttccacaattaccattgttcctggcccggacttcaatccggcctcccacattattcctgataccacaactgacacccatgactgtatctctctgatccacctgacattcaccccatttccccgtatttccttctttcctgttcctcatcctgatcatgcttgatttattgatggcggttccatcaggcctaattgccacacaccagcaaaggcaggctatgctatagcacaagccactagcccgcctcttagaacctttcatttcctttccatggtggaaatctatcctcaaggaaataacttctcagtgttccatctgctattctactactcctcagggattattcaggccccctcccttccctacacatgaagctcgaggatttgcccccacccaggactggcaaattagctttactcaatatgccccgagtcagataactaaaatacctcgtagtctaggtagacactttcactggataggtagaggcctttcctacagggtctgagaaggccaccgcagtcatttcttcccttctgtcagacataattcctcagtttagccttcccaactctatacagtctgataacagaccagcctttattagtcaaatcagccaagcagtttttcaggctcttagtattcagtgaaacctttatatcccttatggtcctccatcttcaggaaaagtagaatggactaaaggtcttttaaaaacacacctcaccaagctcagccaccaattcaaaaaggactggacaatacttttatcactttcccttctcagaagtcagacctgtcctcagaatgatacaaggtacagcccatttgagctcctgtatagacactctttttattaggccccagtctcattccagacaccagaccaacttagactctgcccccaaaaaacttgtcatccctactatcttctgtctagtcatactcctattcaccgttctcaactactcatacatgccctgctcttgtttacactgccggtttacactgtttctccaagccatcacagctgatatctcctggtgctatccccaaactgccactcttaactcttgaagtaaataaataatctttgctggcaggactatgctgaatctccttaggcactctctaatcagatgtcctgagtcgtcccaattcttagacctttaatacctgtttttctccttctcttattctatttagtttttcaattcatacaaaaccatatccatgccatcaccaataattctaaatgacaaatgtttcttctaacaatccacaatatcaccccttaccacaaaatcttccttcatcttaatctctcccactctaggttcccacgccacccctaatcccgctcgaagcagccctgagaaacatcgcccattatctctccataccatctcccaaaattttcgctgtcccaacactttaccactattttgttttatttttcttattaatataagaagacaggaatgtcaggcctctgagcccaagctaagccatcatattccctgtgacctgcacgtacacatccagatccccggttcctgcgttaactgatgacattccaccacaaaagaagtgaaaatggcctgttcctgccttaactgagacattgtcttgtgaaattccttctcctggctcatcctggctcacaagctcccccactgagtaccttgtgacccccactcctgcccgccagagaacaaccccctttttcctttacctacccaaatcttataaaacggccccacccctatctcccttcgctgactctcttttcggactcagcccgcctgcacccaggtgaaataaacagccatgttgctcacacaaagcctgtttggtggtctcttcacacagacacgcatgaaaattactacttcagaatgcatcaccctttcccttcaactcagcacatgtctcttacatgttcgttacttgattgttttccccatcctcatatactctcctggatgcctctaccctcaggttcatggttttctcatgagtatatttattattgacacatactcctaaatcacctctcccagcagattaatttaccttcaagcaatatttaattcccaaagagtttctactggaaaaggtatacagtgtcagaaattgcttttggaatcaaaaaaaaaaaaaaaggcttcaatgtaaattctggccctgccatttaataattgcattgttacaaataaattatttaaatgctctgatattcagttccctgccttcaaaatggaaatactaatagcctctgtgagaattatatgagataaataatgaaagaaacctagtataatcctgtccctggaatatggtggtttatcattaaatgtttagtttctcttctttgcctttcttccctgtctgaagtttctgtaatttccttaaaattacccaacattctacatagtggctgatcatgaccccatttcttgaaaaaagtttcctgggaccggttttggattaaagaagagctacactatggatttagaaaaacgattcacttttgtgcagtgccgctcctatcagtactcctgacatgtcctattggtcccttggttctggccagaatgtgacatttaagaattaggtctatgccttgacatgaaaactttggatactttactagttcataatctgtccccgattgcagttgtgtttgccatatactcctccttctctcccccagcccaggagccatgagatactgtagtcagtgagagggccaaaataaccataacaaaagagcattgacctggttgcatattcatattgcaattcactctttgtacttccaatatgccctacgatttgaacacataagacactgcaaactgaaagaaaaactcaccctatttgagaaaagaaaggaatttataccacatttggcttagtttttataaaagggtgtgtgtgtgtctgtgtgtgtgtgtgtgtgtgtgtgtgtgtgtgtaggcatatatggatgcatgtatatacagacatatatagacacatatgtatacatgtagctacatatatagagacggagacagaaagagatggcat

SEQ ID NO: 14 - DNA, 7643 bp, Homo sapiens
gtcttacgccataacgcatagccttccccttcccgcctagatatctgtgttcaattacaaacagcagccaatcgagtcagtttagattgtgcagtccaaccctagccaataggggaaagacacaacagtagggaccagctgttaggaataagaacccctttccctcccttgtccagtgtgctcttgccattgctccatccgcgagacacacccttctacagaagtaaattgccttgatgagaaaacttttgcctgagtatattttcactttgtgacaccaagcatttacttccaacaatttgggggcccacccaggattcccattctcctccggggaaccggtctctggtcacttcttgtggggaggcgcatcccatcgccttgttgcagtggcctcagtgtgagagattggaacccatccagtgcaacaaataaacccagactctcggcaacaagaaaagatacaggccagcagcttggcaaaaggattctcacatgctgcagcaaccaggtaactctgcacagaccaaggtaagaaatgttgcaggggtgacaaagtatttccttggtggttgggatattctggaggatgaaagtgtgtgtgaatgatcacaagcactactgcttgcggtgctgcttgtgtgaatggtaccaagcactactgctgtgcagagtgagtgggtcctatctgcagttctgtggtcacttcatacagcttagggcggatcctgctgtgggtttcataccggcatgccaatgccaagaggggcctaaattcccacgagggaagtagccagagtggacaaagcaaaagaaggatgcaaggatcctccaggaggcggggttaaaggataggcaagaaatctctaatacaagggactgagccttaacaagcctccagagaataggcaagaagtctctaatactaggacctgacatgggaaataccctaagcaagacaaggagtaaaaaggataaaggtagcagtaaagatattgccccgatagtcccctaggtctcatgttaaaagactggaaagataatgagaagactaaacataagcagcagcaattactgttttatttggactcagggacccatcctcaaaccctcaatcttctggccaaagtttaggtcaaatgagagtgcgatgtgtcagcttttgattcaatatgtcaatgataaaagcccagcttcttaagaggaaatggactatgctctttgttggaggcagggacctgtcctcctttttccctttgagacaactaggaaagaacctgatctagcatcacaaaaggaaaaattaggtaagttagttccaatgctcaaagactccagcacatgggatcccctagaccatcttcccccactcagtgaccccaacccctctcctcaggcagccgctgctgccccagatcccactctagatccttcacctactcatgttactcctcctccttacaatcctgacttttagaaattatcatcccaggagcctgtcccctatcagcctaaggacccctccctaaagggactccagtgtgaaatagagcaatgtaaaaaggatatccagaacttccctttcccctctacaactcaagagtcagcccctgctctctttcccttaagagaaatgccataaagagggggaaccattggctccgtgaatgctcccttaatcagttcagaggtccagaatttaaagaaagagcttaagccactgcaagatgacccttatggagtgacagatcaaactgatcaatttttaggacctcagttatacacttgggtagagttaatgtccatcttggacatcctcttttcaggaaaagaagggagtgtgattcgtagggctgctatggtaatttgggaacgtgagtgtcctcccagtcaaaaagttcctactgtgaaccagaaattccccgcccgagacccccagttggacaataaaaacatgcaggacctaagggagatgataataaaaggaattcaggaatcagtaccccaaaccccaaatctctctaaagcatttgatatataacaaaaaaaaaggatgaagggcctatgagattcctaaatagactgaaagagcaaatgagacaatatgcaggcctcaatttagaagatccccttgggcaaggaatattaaaactccaatttgtcactagaagatggccagacatctcaaaaaaaattacaaaagtagaaaattgggaagaccatctcctaagtgaacttctcagggaagctcaaaaagtatatgtgagaagacatgaagaaaagcaaaaacaaaagacaaaacttatgttatccaccttccaacagatgactccaaacccatatacttctaaacagagcttcaaggggccagaaccataaagggtccaaatactcctttaaaggactaaggaccttgtttaccaggccctctaaagagtatggggaagcaaagtcaaagaatcccagaactgagagggggtaagggcaagataggtgctacaaatgtagaagaacaggccacttcaagacagaatgtcctgaatttaaaaaggagaaagaagcccttccactcatgactttcgaggaagaatacgggggtcaggggccctgtctcttttatcttgagtcccaccaggagcccttgataaatctagaagcgggacctaagcatgagcttatcacctttttggtcaattcaggggtggctcattcctgtttgtttccccccatctaatattgcctacagaacttttggtaactggggtaaaaagagaaggatttaaagaaaaattttaaaaaacacagaagtcagataccaggatcgatcagctcatattcagtttttgttaatccctgaggcagggactaatttattagggagggatttaatgctgaagttaggcataggcctacaagtcagcccaagaggattcctcatctctttaacctattcatcactgcagatgaaaaatacattaatcctaatgtctggtccaaagaggagaactgagggaaactccgagtctccccagtccacgtcaaggtaaaaccccccggggaagttgtaaggaggaaacaataccccatatccagaggacatgatagggtcgaaacctataattaaaggtcttattaaagatgggctttttgagccctgtatgtccccttataacaccccaatattgccagtcaagaaatcagacggatcataccggctggtacaggaccttagagctattaatcaaatagtccaaactacccaccccgttgtccccagttcttacaccattctcagcaacattccatttaatcatcaatggtttactgtaatagatttaaaggatgctttttgggcacgtcccctggctgaagacagtcgagatatatttgcttttgagtgggaaggtccccattcagggcggaaacaacattatcgatggacagtcttaccctaagggttcacagactcccctaacctttttggtcaaattttagaacaagtattagaaaaagttgtcatcccaaaacaaatatgcctactccaatatgttgatgatattcttatatctggtgaggacatacagaaagtaactggcttctctacacatattcttaaccatttgcagttcaaggggttacgagtctcaaaggaaaagcttcagtatgtggagcctgaagttaaatatttaggccacttgataagtgcagactagggcccgaacaagttgagagaattgtgtccctacccttgcctcaaactaaacaagaactcaggaaatttttagggttagctggatgttgccacttatggattaactcatatgcacagtaaactttcatatcaaaaacttccccaggggaagcctgaccatctcctgtggacttctgaggaagtcgatcaggtcaaagagctgaacgaaaggctcataactgcccctgtcttagccttaccttccctagaaaagcgtaccacctttttgtgaacatggataatgcggtagctttgggagtgcttactcaagaacacagtggctgtcggcagcccgtggccttcctgtcaaaagtcttagatctagttacttgtggatggcctcaatacatccaatccattacagctacagcagtattggtcaaagaaaccaaaaacttaacctttggagaaaaattgacagtaagcacgccccactaagttagaactatcttaaatcagaaagcagggaggtggcctgctgactcaagaatcttaaaagtatatgaggctattccgttaaaaaaaaaaaagctgatttaacattaaccactgataatttgcttaacccagcaggtttcctaacaggggatccaaatctaaagaaaaaacacacaggtttagatttaatcgattaccacacaaatgtctgaccagacctaggagaaactcccttcaggacaggaggacacttattataaatggttcctcccaggtgattgagggaaaaagacacaatgggtattcagtaattgacagaaaaactctcaaagaaagagagccaaaaaaattgcccagtgattggtctgcccaaacttgcgagctgttcgcactcagccaaaccttaaagtacttgcagaaccagaaaagacccatctgtacagattctaagtacaccttttgagtggctcatacattttgaaaaatttagactgaacgaggcctcattaatagtaaaggtcaagaccttgctcataaggagctaaccactcaagtattgaataaccttcagttgccagaagaaatacctattgtccacatccccagacaccagaaaagcctttctttcgaaagtcgaggaaataacctaacagatcagatagccaaacaggctgccgtttcctctaaaacacctatttttcacttaactccttaccttcctcctcttaccgtgatccccctttttcttctaatgaaaaaaaaaaaccctaataacaataggtgctaaagagaattcagaaggaaaacggatgtcgccaaaccagagagaaatgttatccaaaccccttatgagggaaatcttatcctaactgcatcaagagatccattgggggccccaagccatgtgtgacggagtcctcagtttatgggagcacagaaatttataccctggccaaacaggttacagacagttgcttagtttgtaagaaaactaataaactataaaaagattaccccttatgggaaggagtccaggcttcagtccattccaaagtatccagattgattacacagagatgcctccaacagggcgtctaaaatacatactagtgacagatcacctcagtcactgggtcgaagctatcccttttcaaatgcaacagccaataatgtagttaaagcctttactaaaaatatagtgcctaggtttgggttaatagaaaatgctgactcagacagtggaacccattttaccacacacatcattaaaaagctatcccaaacactagacattagatgggaatatcatactccttgacacccaccttcatcacggagggtaaaaagaatgaatcaaactctgaagaaccacttaaccaagttggttctggagaattgattaccatggaccaaatgtcttcctattgccctgttaagaatccaaactgccccttggaaagatattcatctttccccttacgagatgctctatggaatgccttatttacactccattgcggacattcctacctttgaaacaaaagaccaattccttaaaaattatatacttggtatatcttctactttctctcctcttaaaaccaaaggtctcctagcacaggcactgtccctggagttcccagtacatcaacatcagcctggggatcacgtcctcatcaaaaactaggacgaaaagctcaaactggcctggaaaggaccatacctagtgcacctaactactgaaaccacagtccagacagcaaaaaaaggatggacccatcacacccgagtcaaaaaagtgccgccccctccagagtcatgggccatagtcccaggggaaaaccctaccaaactaaagctaaggaaaatttaactctctttcatctattctattactccttcttctttcctctctattgctgatcacctcattattaatgtaaccgagtcaatttcgcctcaaactattatatttgatgcttgccttgttataccctgtggagacttgacacgtcgaagcagctctccactccaaaaaagtacctctgtccttcctggctctgctcagactggatattagtgaatcgggatcatttagtctggaaaggtttcaataaagaccccaatgtcaactgggagtattgccccccacaccccgccaagacagagcttttatgctgcagttggtccaatgttctgtagaccaataaagagcacagatggactgccccaaccagtagttgtaaacgttctgtagaccactaaagagcacggataaactgccccaaccagtagctgtaatttcctaaagccatacattcactttactaaagaaacagcttcccctagctgtgagctaaaccagtactgtccaatacaggttattatctcaaaccctccaagttcttccccttctataagccggttcccttctttaagccagttttatggcatgggggctgaggtttcaggaacagaacctattggatcctttgaaatatgctgcattgatcccctactgcctacactttcccctaagccttcttccaaaacctctcacaacaaaactattgctcctcctccatctaatgaaaagaccaaggtagctattgtagaagttaaagacctaaaacaaactttggcaactgagacaggatatcaagatgtgaatgctcttaaatttaaaactcgagatcaaatagctgcaggatttgagtcaatatttttgtgagtgacaactaataaaaacgtagattggataaattacatttattataatcagcagtggtttataattacaccacggatgctgtcaaagggtaacagaacaattggggcccactagccagatggcctgagaaaacagaatggccctagatatattagccaaaataggggatgtttgtgttatgattaaaattcactgttgtacctttatcccaaacaacactgaccccactgggaacataataagcgtcttacaaagacttaccgctttatccaatgaactaactaaaaattctggagtcgataaccctttctcaacatggctagagaggtagttcagtaaatgaaaaggaatcatagcctcaatccttctcttacagccattataggtgtgctcattcttacaggatgctgtatcataccctgtactcatagtttagtgcaaagacttataaaaacagctctcaccaaaaccttcctcagctctcctccaccttattcagataaactcttccttctcctagacatgcattgtgtcataatggatagcctttcccttccagcctagacagctgggttcaatttcaaacattagtcaactgggtcactttagattgtgcggtccaaccctagccagtaggggaaagacacaacagtggggaccagctgtgttaagaataagaacctcttcccctcccttgtccatctcacgattgctccatctgca

SEQ ID NO: 15 - DNA, 7744 bp, Homo sapiens
gccagaaacaataagttcctcttcaaagcttgcttggtctttcttgctctgtacacaagcccttcctgcttaatctgtaatgaacacttgtttctctgcttaatctataactagcaaatctctgactctgtaaacaacccttcccaactagttggtaatggacagcctctcccttctcgcctaattgaccttattcaatttcaaacactagccaatcgggtcagcttagactgtgtggtccaactccacccaatgggggaaaggacacaggaactgtgttagggataaaaacccctgccctaccctgctcagtgtgttcttgtgatcggacaggtgcaggtagcacccttctgcagaagtaaatgtgtcttgctgagaaactttctaagtgctggtttttctttgtggcactgagcacttgtctctaacaatttgagggatcgtccaggatcccattctcctctggggaagggtctctgatcatctcttgtgaggagatgtgtcccactgccttgttgcagtggcctcaggggtgagggatcgagacccacctggtgtgacgaataaacccagactctcagcaacgcaggaggaaagggcctactgatactgtggcgacccagtaactgtgcacagaccaatgtaagaaaatccatggggcagtgaagtacttccttggtggtcaggacaccctggaagttgaaagtgtgtgaatgagatgcagaattaagtctgaagcaagtgtggagtccagatttgcagttctgtggtcacctcatacagcttaaggtggggcacgcctttcctgtcgggggtttataccaacccaccaatgctaagagggacctaaattcccatgagggaagcggcccaagaaggatgaagggaaggcaaaggagtgcaagaaacctccagtggggtggttgagcctccagagaaagggtgcaagaaatctctagtaagagaggtttagccccacacatgcaggaaactcagggaaacacctaaaacttccaggatgggaaataacccaagcaggacaggaaatataaaggactagacagacaataaaattccctctaatagccctccaggtctcatgttaaaatactgtaagggtaatgaaaggactaaacattagaaaaagcaacaaatgataaaatattgttgttttatttggaccaaagaacccacccttgaaccctcagtttgcttttttttttggccagtttgggtcaaatgaggattggatttgtcaacttctaatagaatatgtcaatgacaaaagtcctgtctcccaggaggaaatagactatgccctgtgctggcggcaggggcctgtcctcctctaccccctaaaagctacaggaaataagccaaaagctacctcccctgaaaacagaatccctacccccaagcagtctaacaccacatgggaccctttagacaaccttcccccacccaccgctctgccccaagctgaacactcagtccctccaccatataaccctgccctgcgggccccgtcaccccacattcctatggagtagtcgcccaaacatgcccctccctcagagaagctccaacgagaaatagaacaatgccacagggacactcacaacttccctttcctctcctaaaaggagtctgccccaaccctttttcccttaagagaagtgccacgtggaggaatgggaattggctttgtaaatgcccccttaactagtttagaggtcagaaacctgaagagggaacttaaaccactattagatgatccttttggggtcacggatcaaattgaccaatttttaggaccacaagtatacacttgggctgagttaatgtccatcttcagtattctcttttcgagggaggaaagaaccatgatccgcagggctgctatgatagtctgggagcacaaacatcctcccggtcaaaatatccctgcagcagaacaaaaatttctggcccaagacccgcaatgggataataacaatgcagcccaccgagaaaacttgaaagaccttagggaaatgatagttaaagggattcaggaatcagtgccttgaacccaaagtatttcccgagcatttaatatacagcagggaaaagatgaagggcccatggagtttttaaacagactcaaggaacagatgagaaaatatgtaggcttagacacagaggatccccttgggcaggggatgtgaaagctccattttgttactaatagttggccagatatcacaaagaaattacaaaaaatagagaactggaaatggaaagatcggcctatagaggaacctttgagggaggcccaaaaagtatatgtaagaagggataaagaaaagcaaaagcaaaaggcaaaaaatcatgctgtccgctctacaacaaagtacccgagggtccaaaacctgtaaagaacttaagcccccactcactaggccatataaagggtatgtaaaagcaaagcaaggaaacttaaaaacagggagagaaagagggcaaaacaaatgtttcaaatgtggaagaataggtcacttcaaaagagaatgtcccaaatgggaaaaagaaaaagaagtcatcccacttacggcctttgaagaagaatagggaggtcagggattctgtttcttttatctcaagtaccaccaagagccccttataaatttagaggtgggacgtaaatccgaactgctccccggaaagacatcagcttatctccttatgaaatgttttatgggttgccttatttaaattccactacggacctcccgacatttgagacaaaggatcagtttcttaaaaactatgtatttggtctgtcttctaccctttcctttctcaggactcaaggcctcctagcgcaaactccaccccttgaattcgcagttcaccaacaccaacctggagatcatgtccttatcagaagttggaaagagggaaagctcgaacccacctgggaaggaccccttatctagtgctcctaacgactgaaacagcagtctgaaccactgagaaggggttgacccaccatacccgggtcaaaaaggcatcgccctctccaaagtcaaggaccatcatcccaggaccaacccccatcagagtaatgttaaagaaaaaagcctaatctgtctatccttttttttttcctcttctctttcccttagctaccccacatctcattattaatataaacgcatcagagtcaccgcaaatcattacttttgatgcttgtcttgttataccctgtggagacttgcgaagtcaaaggcagctctctactttgcccttcttggaaattctcagactgggcagattctattaactggggagttcccttagacttgggatattatttttaaaattctgttaactgggaatcccgtcctctgcaaacagagcgtctctgccatagctggtccaatgttctatggactacgaaaaatcagggttggacctccccaacaagtctctgtgtatccctaaaactatacaattgtttcactaaaggaagcccccccaccaattgccagcaaaactaatgtaatccagtacaaatttccattactatctcaatttcccaaaattcctcccttcattaagtcgtttctagggtatgggagcagaggtcgcaggggcagactctacaggatttttcaaaattagtttcgttgcctcgtcatcccctccgccctctccttcaaaccttctaatcaaactactagtctctccctacaatgcaatggctcccaaagtagccactgtagaagttaaagatttaaaacccaccctagctattgaaacagggtaccaagatgcaaatgcctggctagcacggattaaatattccgtccgcaaactaaacaaaagcgactgttaacgcttgtgcaacgggcaggccagaaacccaaatcatcccctttctacttggatggtcctccgaccaacagggtatgagctgtatggtatctctcttccaaaaccccacagcctggggcaataaggcatgccaaactctcttgctgttattcccggaagttaaaagccctgcgggtcagcccccaagggccatctgtcctccaggtaccaatgtcaatttcacctcgtgtctctcacagcaaggggaaaacttggcattccttggaaatctagcaagatgaagtaagcctaagcctttctaggagctaaccaatcagtctgcccttgttcatccccaagcagatgtatggtggtactgtggtggaccactattgggtactctgccaaataagtggggcaacacttgcgccctaattcaattggccatcccaccctggcatttcgtcgactaagcaaaaaggacaatcacaaaaaaaggagtactccctacgggtcctctgacccttacatttacatagatgccatcggagttccacgaggagtgttaaatgaatttaaagcccaaaatcaaatagctacaggatttcaatctatattgttctcatgggaaactgtaaacaaaagtgtagactggataaattacatttactataatcaacagcagtttgtcaattatactagggatgccattaaaggaatagctgaacaattaggtcctaacagccaaatggcttgggaaaacaggatagccctggacatgatattagccaagaaaggtgggagtctgtgtcatgattggggtccaatgctgtacttttatccctaacaacacagcccccgatggaacaattacaaaagcctgggccttaccaccctagcaaatgaattagccgaaaattctggaatagattaccccttctctggtctcatggaaaaatggtttagaaaatggaagggactcataacctcaatctttaccccccttgcaattgctataggtgtactcattcttgtaggttgctgcaccatacctcgtatttgtggatcagggcaaaggcttataaaaacagcccccaccaaaacccctctcgattctccccctccctactcggataagttcctactcccagacaaccaagaggagcaacaaagccaagatatgttacaaaaatttgaagaggaagaactataaactcaagagggggaaatctgccagacacaataagttcctcttcaaagcttccttcgtctttctctctgtacacagcccttcctgcttaatctgtaatgaacacttgtttctctgcttaatctataactagcaaatctctgactctgtaaacaacccctcccaactagttggtaatagacagcctctcccttcccgcctaattggccttattccattttaaacactagccaattgggtcagcttagactgtgtggtccaactccagccaatggggaaaggacacagaaacaggaactatatagggatttaaaaccctgctctaccctgctcagtgtgctcttgtgatcagacaggtgcaggcagcaccattctgcagaagtaaatgtgccttgctgagaaattttctaagtgctggtttttctttgtggcaccgagcacttgtctgtaacatttgtgtgtctgtctccttcaatacactgaaaagtccttgatggcaggaactgtatttatcttttatctgtaaacccctgtagagtgcctgtaaatgtgtactgaataaatgaatgccaccaacaaatccagacccaaccctcaatggcacaaatcatatgttataatcaatgcctcccaacaatttgaatctcacagatatactttgcactaaagaagccagatacgaaacaggacattttgtattattccatttgaagttcaataacaggcaaaactaatctttgtgacagaagccagaactaagcggagtagggtagagtgaggggggggtcttatccaggaagggtcacaagagaaccttatggagtgttggaacagtctctatgttgatctgagggtggcagttacacaggtatatacatatctaaaagaataatcaagcagtatacttgagattagtaccatttactgaaatttatcttgtatttcaaaaacccaagttctatatatggccctcatctgcctcaacccccatccaaacatcaatgctcaataaacatttgtgactgaacgcctaaatactttctaaataacaacaatcaactacactattttcatataagggaagaaaaatctagtcaagcaattgcagtcaaagttttgggctggagctaagctaaccaccaccatcacctcacacaaacaagaaacttgcttctgtccagagttgcagtgtgcctacaggtgctgcatgggtagcatttgcccctccctatgactggctggaaacatacccagccccactgttgaggcataggatcccaatggcatttcaagtcactaggagaaaaaagtggaattttacaactgaaggctctatcacatcaaaaatctagacacactggcaataaaatcagaagaaaacctctgcccacctttccaggaattttcacttaatctttctgtgactgttacctgcctgacaaactcctattcatccttcaaatcccaactcagatgttaactcttctgggaagttcttcctaacctcctcaccctccttctatgttccttttactgttctattactttggttcacttcaatttaaatattggtcatgtttatttcccctgagatcacatttgccattctagcacgaagtacatggcagggctctttagaagcatgaaaatgtctgttgaagtgacttgaaacacgactactactggacatgccttacaatttatatgcccaactctagagtcccaaaataagtggtatttcctagataaggcacagtctgtacttatgaagagggagtgaaaaaactataaatattctctaggacagtgttatttttagtattatggtcaccagcctctaagagtgaacttcaaggtagcaacctggagactaaatgactcaaagattatgggatctgccaggaaaggtatgctcctgaagctatggtatagcagatatggtcccagaagcagtgggttcactcgcttcaaggcaggatcttcaatgccctgcatttatataaatgtcagaacaagtaactgtgcaaccccaaacaagttactttacctccctgtgcctcagtttcctcattggtaaaatgaaggtaataacagaacccaaaatttcatgtggtgttaaaggattaaatgagatgatacagtgcctggcatatcgtgagcactcaataaatgtttgctccaattatttcactgctctgggacgggacagggatccctcagttttatttggtcctgtcatattcctgccctacctggcaccggcaccaaatctcttctctgagcctctccaccctggcttccttgcttgcacagctgattaccctcaccacacagggcctccctctggccatgaacacaacccaacaaagcaaagctacactgcattctttagtccctctcctcttccactttcctaatgaaaacttagttgtttcctatttcatttccgtggtgctctatctccttttggttagcagattaatgagagcaaactgatcaaatacccatgtccctacagtcactctctcaaagattctcatgaataaactcagttaaatagagtaacatgaattacaagaatttcaggctctactgtctaatgagacaaagcttcctttccgctaccccctcctctccctctctctttcttcctggcaaagagaagaggggatgctg

SEQ ID NO: 16 - DNA, 9755 bp, Homo sapiens
tggagggcaggaagcatccggcatgggagaaagatgtaggctgggagggtaggccagtctggccttttcacatttctccagtattaaccatcacacctataaatttccccagcctataagcagctatgggctctggagttaagctcgtcccccatctccacaggtttttgcaatatacctgtgttgttgctgttgagcaacaatctctctctctctctctgtctgtctcccccctctctctcctctctctctctctgtgtgtgtgtgtgtgtgtgtgtgtgtttctttagcccttgccctcccttcaaaacctaacattttagtgccaaaacccaggataggaattgggttctaaatgggtaaatgttttctagcaacctggaaagcagcaagcagcaaaaaccagacccaggcctgcttccagatcctgaatggactccctattcccagctccgttcctttattctctcttcttctctggtcctgggctgacttccagatcctgatcaaactctccatcctctttttccttccttcccctttccaggcagctccagcaagtatcaatcccattgctggacatcacatccaacacccgtctccaattagtgggtgagtctctctttttttcctctccagattcctctcatatttctgggggttcaccagaaaattccagtaccaggtgagaggtctccctggtcaccaggtgaccgtggcctaccctctcaggggacgccgtcagaatgctcaccactttggccactgcagcctctgggggtctgcaaagagctgtagggacgccctggctctcctaggtcccttctcccaggaggaatcggggtactcactcccctccggggtattcacttccctctggggtacttccatcctctaaatttctcaccctctggccagcagtatggggcaacactcctcaaaacctcaagacaccactcttggatgtttccatccagaacctccaagcccagggcttggcagactccattaaaactgaacgccttgctggccaagtgtgatagttcatgcctgtaatctcagcactttgggaggccaaggtgggcagatcacaagatcaggagttcgagaccagcctggccaatatggtgaaaccctgtctctactaaaaatacaaaaattagccgggtgtggtggcaggtgcctgtaatcccagctacccaggaggctgaggcaggagaattgcttgaaccggggaggcagaggttgcagtgagccaagatcgttccactgcattccagtctgggtgacagagtgagactctgtctcaaacaaaaacaaaaacaaaaacaaaaaactgaacaccttactttcctctgtaatgttgcccagccccaatgtaaactagacaataatagtcaatagccaaaaaccaaaacattcaatttccacatctgacataatctaaaagacttcctccagtgcaatcgtaaatgatctgaggtgctttgcttatctgtgctcctggctcactctctctctgccaatcccgttcaccttttcaaatcttcctcctcaacaaaaaacccacaaaaacgcctcctcctccagacaaacctttctcctctaatttcaacctagccaacaaactaggcacgtgcccagcccccttccaccaaaaaccaggcacacagccaaaggtcctcctaagttctccctttccaggaggtcacagggactaaaggcataatctgagttcatgttcccttttccctagtcgacctctctcagcttaaaaagagactcagcggccgggcgtggtggctcacacctgtaatcccagcaatttgggaggctgaggcaggctgataacgaggtcatgatattgagaccatcctggctaacatagtgaaaccctgtctctactaaaaatacaaaaaattagctgggcgtggtggcagacgcctgtagtcccagctacttgggaggctgaggcaggagaatggtgtgaacccaggaggtggagcttgcagtgagccaagatcacgccactgtactccagcctgggcgacagagcgagactctgtctcaaaaaaaaaaagagattcagctcgttttgcacagatcccacctccttcctcaaggaatttctgtatgtcactcaattttatgaccttacctggcatgtcatatatgtcatcctctcctgcaccctcacccctgaggacagggaatgcatctggatagctgcccaggcccatgtagacaccctcccatagacaagatgctgcccataacccaatatggaccctaactgtccccagaactgaccccagttgggattatcaggcaacttctgcagacagatagaaataaggccatatgatatgcctcctagctggcataaataaagccattcctggccaggcatggtggctcacatctgtaatcccagcacttcgggaggccaaggcaggcagatcacctgaggtcaggagttcgagaccagcctgaccaacatggagaaactccgtctgtactaaaaaaaaaaaaaaaaaaaaaattaggcgtggtggtgcatgcctgtataaaggggaataagtattaacttacacaatcataaggtcccacaataggctgtctgcaagcttgtggagcaaggagagccagtccgagtctcagctacccgggaggctaaggcaggagaatcacttgaactcaggaggcagaggttgtggtgagtcgagatcacgccattgcactccagcctgggcaacaagagtgaaactccatctcaaaaataaataaataaagctgttcctgctcttttcttctcctgcctttcaaaggccataactaaatatgccacgttgaaccctaatgccaataagggaagaatctacctccatttacacttcattttccagtcagccccagacattctaatgaaacttaaaaaactggagaatagccctcaaacctcccaaaaagacttaatcaaagtggcctttaaggtctttaacaatagagaggaaaaactaaaagtccaaaagctaaaaagagaccaggctaaatgccagatgctggcagctgccattcaacagggttcccaacatgtacagaaatcctcaaccttgcagcaaactctaccagaagcctgttttaagtgcagccaacagagtcactgggcaaaggcctactctcaaaactttgccccatctgtggcatcaaggaacattggaagtgggactgtgctcagcaaaactcttcatcccgcttcaccacctctaactgaagactgatggggccaggggcctaccaccccaactgccatcaccacctcggaacccagggtcagtctctggtaagcccatgtctttcctattggatacagggactagttactcagttttattagaatattctggacccctcctcagttcttctatctgtattgtgggagttgatggaatcccctctaggcacaaacagactggtcctctattatgcaacctattcaacaccccattcacccactccttcctggttatccctcggtgccctgcccctatcttggggcaggacatactaagtaaatcccaggcctccatacaatctgcctcctgcaattccgctccttttattttattctgccaccagatgcttccctctccccctcatcctcgttatccaccctgttaccttctgttaattctgaaatttggaacatttttaaacccacaatagccacacatcacatcccagttaaaataaccctccaaaaccactccattttccatcatcagtctcaatatcccctaacccaggcagcctcaggggcctcaaacctattatctgtaaacttttacaagctaatattctcaagatcctaccacttggtccaggatctctgagttgttaaccaggtggtaataccaattcatccaacactccactctcatcccacatactccactctcccatagtccctcttctaccacacacttccctgtactggatttaaaggacacctttttcactatttccttaaattcggcttcccaaagtatttttgctttctcttggtcagatcctaatacccacatgtccacccaactaacatggaccatactcccacaggggttctgggacagcccccacctattcggacaggccgtcaccaaggacctagctgaacttcccattgctcctagcaccctccctcaataagtcaatgacctacttttctgtagcccctcccttaacctgtccatccaacgcaccactcagcttttaaacttcctccataggtaaagatattgggtctcaccaacaaagactcatgtagcccaaacccaggtcactcacctgagttctaacccctaattctcaggccatcctaacccaacaaaaggagctaattcaagacattgccccttccccacacaaagaaggacctcctgtccttcttgggcctcatgggatacttccggctgtggattcccaacttctgtttgctggccaagctgctctacatgtcctcacttgggcccagcctagagcctctgaacccggctcgtcccatcaattcacactttaaaaaaaactaaaaaatacccttttaatggccccagaactgggactgcccaaccccaccaagccctttactctgcatgtacattctgacaaggccttgctcttgaactgctctgccaaacacaagccattgcatacccctcaaaacaaccagactgtcgtccaaggctggccaccctgcctaaaaatcttgggtgcggccacattgctggcctcggaggcacagaaactcactctctaccaacacattactatttcatcttcccataacctacaggacctcatgagccatcaatctcttctatccctcccatcatcctgcttacaccaggtacacaccttattcataggaaaccttctaatcaccttccagaaaggtaaagctctcaaccctcccactctcctccctgtaaacacctctgactctgagctgtctcactcctgcctggacctcttagactccctttcctcccccttccaacacatttcagaagcccctttgcagggaacaactacatggttcattaacggaagctctttaaaggagccatgtccaccatgtggttacaacatcattgccaaaataaactctcagaatctaatgctctcccaccccatactacctcgcaacaggcagaactacctctcaacagatagagttggttgccctaaccagggccctcaccctaacaaagggaaagagggttaacttttacactgattcctggcccggcgtggtggctcacgcctgtaatcccagcactttgggaggccgaggcgggcggatcacgaggtcgggagatcgagaccatcctggccaacacggtgaaaccccatctctactaaaaatacaaaaattagctgggcatggtggcgggcacctgtagtcacagctactctggaggctgaggcaggagaattgcttgaacccaggaggcgggggttgcagtgagccaagattgtgccacttactccagcctgggtgacagagtgagactccattacaggaaaaaaaaacatttacaccaataccaaatatgcataccacatcctacattctcacaccttaatctggcaggaaaggggatttctagctaaaaagaacccccatagtaaatggcaaactcatacacaagctggtggaggcagctaaactaccactacaggccaccattatccattgtaagggacaccaaaaggctacaaatgccataaccaagggaaatcttttagcaaattaggcagcccggcaggcagcccttaaaccccatcattattgcccagttttcccagcatataccctgtatgtacccaggaggaacaaacctcacttgccctggctggtgccattcaggaaaaaatggttctacctcagtgctaaaattgtcttggccaaattttaaaaaccttctgggccgggcatggtggctcacgcctgtaatcccagcattttgggaggctgaggcgggaggatcacctgaggtcaggagttcaaaaccagcctggccaacatggtgaaaccccatgtctactaaaaatacaaaaattagccggacatggtggcaggcgcctgtaatcccagctactcaggaggctgaggcagagaactgcttgaacccaggatggagaggatgcattgagccgagatcgtgccactgcactccagcctgggtgacagagcaagactctgtctcaaaaaaaaaaaccttctgtacttttatatgtgcacaaccatttccatgctggttgcctccccctacttcagctcttaaaaacatatacattctcccaccatggctgccaatctcaaagatattactaaggcatgttccctttgcactcagacttcccctcagaaagctatcaaatcaccccctttccccacacaccaggcctgaggacacctgccagggcaggactgggaaatcgccttcacctgcatgccccctgtaaaatgagtccagaaccttctgacaatagtagatacactggatggatagaggggtttcctaccaccactactactactactgaaaagccacactgttgcttctattctcctcacacatattatcccccggtttggactcccctctttcatccagtcagacaacgggccaacatatgtttcacaggttagccaacagctggcaaaggctctaaacattaaatgggccttccatattccttattgaccctcatcttcaggtaagattgaatggtccaatgcccttctaaaacaacaattatccaaactctccctagaggttaaaatggcctaaactttactactccccatggccctcatgcatttataagccattcctcacaagcccctcagcataagcccatttgaacatatgtatggatgcccctttatcctccaaaatctccctgtatctccccgcccttctgcatggggtacttggccagcattacacctcactcaccatctaatagacagtacactaacgcttacttgccgccgcctgaaagtccatcctcaaaacactcctccctgtccctacaaccaggggggactgggtctggatcacagacccctcctcctcccctctcctaccaaagtggacgggtcctcaccaggttattctagctactcccacggcagcaaagctaacacccttcccacactggatacacaattccaaactaaaaaaacctccagattcacatccagaaaatttctccccccacaaaaactattcttcctccctcacaggaccaacctcactgcgcttaacaagggtgcagaagttgcctatccagaaggccctggtccgtaacactctctgcctccaatttcaaatattttatctcataccttgtttcagatctttccctccccacgtccctggatactccactcgaattcctcacatcaatccaggagctatggctacagggtacctttcagaatttcactcctactcaaattgccttttttcattttgtcctttgtgggatatgctaagtcctcacccccaacctctggcagtcgggccccttcatcagcctcacacatttctcttaaatcagtcacactcccctctttcttccaactgtaaatttgtttgtccacacaaatccagcagttcacagcccttcctgttaatctaactgcagaaacttggcccaaaataaacctgcatctcacctacttggccaattcattcccaaaacctgtttataatcttgttcggctaaacacctttccccgcaatccatcatatccacccacaccgtcacacacagggctgtcactctcctttgcctcttaacatctaaacatgttacaagttggattccatagaacacctcttatcaacccctcccctctctgccagcactgctctccgtgtaaccaactcaagggcgctccctggaaaaaatgcacacacaattccctcagctgcaacctatatccttctgccctacccgtactgcagtagctacttgttaacgaaaacctatttctgtctctctccaaaaccaaacagccttcacctcctcccccaccaacatcccctatccggccctcacaggggttacccttgttaacagctattcaacctggaaaaacaaaaagttggaacaaaacctttgtccaggattcacccctgatcttctcatagctcgctaccttcacttacaacttttgcctgccaacccccccaaccccccttttctttctgtatgaaacaaacttatctttgtctgccggcaggtgggttacaaacatacaccctggtgtttcaatctccaaacgttgacattttgcctaacaaccaaaccattgaggctctccctatttcctcctcctccgagcacgctaagccagctctacatctccttcttctggtaacaggattaagcctctctgtcgcacttggcaccacaatggcgggtcgggtgtatcagcctcagctgccttatatagatatataaatctctgcagtcctcttgacatgcctacttccatcacaagcctccaaaggcaggtaggttcccctgtgggagttgttctccagaaccgaagggccgtagacctgtcagccactgagaaggggcgcacatgtgtgtatctctaagaaggaggctgtttaaatgttcacgaatacggcactgtttgagacacagcccgcaggctccgagacgggtctgcagaaatccaacatcaagccactaactcttagaggcaggggtcatccctcctaaagtggatgccttgggtaacctcttcttagggcccctaattttcttcttcctaacagttggcctgtgtgtactcaccttcatatcccacttcacctcccaaaggctgaactcccttgtccaggcagccacccagaaagacactgataccatcccactccgccaagtccagtatcagcgccgccaggaaagcaactcagaagtcagacacccactgcttcaaaacccaaaccctgattacagcaccactattcagcaggaagcagccagataatcaacaaccacgctcttccctttatattaaagtagaaggtggccaggcgcggtggctcacgcctgtaatcccagcagtttgggaggctgaggcaggcagatcacttgaggtcaggagtttgagaccagcctggccaacatggtgaaaccccatctctactgaaaatacaaaaattagccgggtgtggtggcggccacctgtagtcccagctactcaggaggctgaggcaagagaatcgcttgaacccgggaggcagaggctgcaatgagccaagattgcaccactgcattccagcctgggcgacagagtgagactctgtctcgaaaaaataaaaaaagtataaagcaagaatgttagtccaacctgcacaattttgtaagtcccccaccatttcgcagaccttggtcaaaatgaaacattccacgggggtttgggtggtgagaaacagcctgcctcttatattctgctgggagaaagtgcaaagaacaccacattctgccggaacaagggccagaaccacctcatcctaagaacacattatcaacattttcccaggaagcaggccatgaccccctgccccgacccctcccactcaggcctataaattgccccagcctgtaagcggcaatgggctctgggactaagctggtcgcccatctccacaggtttttgc

SEQ ID NO: 17 - DNA, 9708 bp, Homo sapiens
gagaggtgatgccagctgggcttcctgggtcgagtaggggcttggaaagctgtaaaactcactcatttcctgcatcagggattacttcggttctggataaataatattgaggtataatatatgcttaaaatattcctaacaccaggatttacttatatgttttcttccccaagaaagctataaacagcgagaattttaggtgtaagttttcctgtgtgccctcccccgaaaccagagttaaagaaaagattaactgcccatttttctgtgatcagtgggccttatctatcctcccaattccttgtaaacactgtttgtaagttctataagatcctgcttttttgctgtgcagctgcaaggccataaatcaggtaagcgtaagtcgcaatttcagtttttctcaaaatctaaagcatgtcacaaaataatttactgcctttgtttctcgctcctgtactggaacatacttcccgcctcacatatctcccgccttaaagagtttaaaaggcaatcacccgagctagcagtggcaacccattcgggaccccttccatgctgtggaagctttgtactttcgctctgctcaataaaacctacagctcattctctctcttggtccaagtatctgtcactcgccatggtcagccgccacaccaattctttggcgtggctaggcaaagaaccttgggtgttacatcttagtgagccagccaggagactccaggaagagcatcccaactgccacgcagtgagtaccctcggacctcttttgcttgctattctgtcccatccttccttagaattcggaggctaaacactgggcacctgtcagccagttaaaggcgattagcaagaccactggactaaaaacacgagtgtcagcctgggaaagggctctctgacaatccctgaccctttggagttgggagcactggtttgcccggaaccagttttaagtctttcactttctgtagtggtcccgaagtacacccgggagtgctcagcaaatgtcatggtctcccagatatccaggttgagaccatggccccaccagaggctcccacagcatgggttactaagcgtgagacagccacatcttctgactcctgcgtcctgggttcaaataactgccggttagatttctttcctcacctggtaagcaagattattcccactagacaggaccaagaatccctatttaggagacttaagtttttaaggtggtgttcagaagttccttgttgatggtgccctctggaatttaggcaggtgttgccatctgatggccactttgaaaggccagttccccaccatcgtgtatggtctcccacatcaggacaatttgaagacagatctgtaattttcatgtggatggtagaggccctaggacattttcttcattgttccccagatgaatttcctttttttggtgcctctcaagtataatctgtggtgtatgggtacggcccttagagcagttgaattgctttttcaaccattcaatcatggatattggaagaaagaaaatatagtcaattgagacacgggatactggtaccaccttaagatgggggcttactcctttgatggaaagtggggacaaaaggctagagtgcagcagttgttctctcagccctggcctagaggacatcaaccatcccctttgagcttactaagcctcctgtcactaattcagagattcctccttgaagggcagttttatggccaggcccacgtaaattgggccttgacatgcaagcatcagtggtgcccccgacccaggccttgccaccccagaacagataggacgcgttggcaaagggaccacaataaatccaacagtcctcatgccccatctagtggtcaatgggtgcacggcagagggcaaggatgatttccattctgccggtaagcgtggttaaatctggtaaatggaaggctcaaggacgatcatgcgctccgagcacaattggactggacccttgggggatgccctaaggggaagatgagtccctaagactaaccaggggtgcgggcatacctgtgtttaaaattccagttgggcaccacgccttcaaaactggacactcccttgagatgtatcctgaataactgggacaagttcgaccctgagaccttaaaaaagaagcgactgattgtcttctgtaccaatgcctggccacagtactccttacaaaatggagaaacttggccccctgagggaagtattaattataacaccattctacaactagatcttttctgtaaacgggaaggtaaatggagtgaaatcccttatgtacaggctttctttgcccttcgtgacaatactgctctatgccaagcctgcaagatttgcccaaatgacaaaaacccacaattgcctccatactcagggcctccttccttagccccactctcttccctcactgactctcctccatccagccccaccaaagtgttagaggcacaccgaaaagaaaacgtaaactccgcgaaccaggcgcccaaactaagtcccttacaagcagtaggaggagaatttaggcccacccatgtgcatgtctctttctcactctcagatttaaaacaaataaaggcagatacagggaaattctcggatgatcccaataactatatagatgtcttacaagggttaggacagtcctttgatctagcatggaggggcatcatgttgctccttgatcagaccttaagtcctactgaaaaggagggagctttagcggcagcccagcaatttagggatttatggtatctcagccaggtaaacagatcaaatggccccagaggagaaggaaaaattcccccacagggcaacaggaggtcaccgctgtagaccctcattgggatactgactcagatcatgaagattggagccgcaggcatttgctaacttgtatcttggaagggttaagaagaagtaggaagaagcctatgaactactcaatgctatccacaattacacagggaaaagaagaaaacccctcagcttttctagaaagggtatgggaggctctaagaaagtatacctccctaactccggattccctggaaggccaacttattctaaaggataaatttatcacccaatcagcggccaatattaggagaaaactccaaaagtctgccttaggcccagaacaaaatttggaggcattattaaacctggtgaccttggtgttctataaaatggaccgagaggaacaggccaaaagggaaaagcaagataagagaaagaccgcagccttggtcatggctctcagacaagcaaacattggaggttcagaaaggacaaaaaatggagcaggacaatcacctggtagggcttgtgatcactgtggtttgcaaagacactttaaaaaagattgtccaacaaaaaacaaactgcccccttgcccacgtccaatatgccaaggaaaccattggaaggcatgctgccccagatgatgaaggctctctgggccagaagcccccagccagatgattcagcaagaggactgagggtgcctggggcaagcgccagctcatatcaccctcacagagccccgggtaagctcaaccattaagaaccaggaaatcgatttcctcctggacaccagcacggtcttctcagtgttaatctcctgccctagacagttatcctcaagatccattaccatccaaggaatcctaggacagcctgtaaccaggtatttctcccacctcctcagctgcaactgggagaccttgctcttttcacgtctttcttatcatgcctgaaagtcccacacccttattaaggagggacatattatccaaagctggagctattaactacacgaatacgggggacaaattacccatttgttgtcccttacttgaggagggaatcgaccctgaagtctgggcaatggaaggacaattcggtagggcaaaaaatgcctgtccagttcaaattaggctaaaagaccccaccacttttccttatcaaaggcaatatcccctatggcctgaagctcataaaggaccagaggatattattaggcatttaaaagctcaaggcttagtgagaaaatgggacagtccctgcaacaccccaatcctacgagtacaaaaaccaaatggtcagtggagaccagtgcaagacctcagaatcatcaatgaggcagtaattcctttatatgctgctgtacccaacccctaagccccgctctctcagataccagaggaagcagaacggttcactgttctggacctcaaggatgccttctcctgcattccccagcacactgactcccagttcctctttgcctttgaggatcctacagaccacacatcccgactttcgtggatggtcctgccccaggggtttagggatagccctcatctgtttggtcaggcactggcccaagacctaggccaattctcaagtccaggcactctagtcctccaatacgcagatgacttactttgggctaccagtttggaagcctcacatcaacagactactctagatctcttgaattttctagctaatcgagggtacaaggtatttaagtcagaggcccagctctgccaacaacaaattaaatatctaggcttaaacctagccgaaagaactagggccctcagcaaagaacaaattgagcctatactggcttatcctcgccctaagacattgaaacagttgcagggattccttggaatcgccggcttttgccaactgtgaatccctggatacagtgagaaggccaagccactctatattctgataaaggagacccagagggcaaataactcatctagtagaatgggaatcagaggcggaaacagccttcaaaactttataacagaccctagtacatgctccagccctaagccttcccacgggacaaaatttatctttatatgtcacagagagaccaggaatagctcttggagttctaagtcagacccgtgggatagccctacaaccaggggcatacctaagtaaggaaactaatgtagtagcaaaaggctggcctcactgtttatgggtggttgcagcagcggccatcttagtatcagagactatcaaaataatacaaggaaaggatctcactgtctggactactcatgatgtaagtggcatattaaatgctaaaggaagtttgtggctctcagataaccacctactcaaataccaggcactaatccttgaaggatcagtgtttcaaatatgcacatgtgcagccctcaactctgccacttttctcccagaggatggggagccaattgagcataactgccaccaaattattgcccagacttatgccgcctgggaggatctcttagaagttcctttaactaaccctgaccttaacctgtatactgatagaagttcatttaggtacaaagggcaggctatgccatagttagcaatgcaacagtacttgagagtaagcctcttcccccagggaccagcacccagttagcagaactcgtggcacttacctgagccttagaactgggagaaggaaaaagaataaatgtgtatacagatagcagatatgcttatctagttctacatgcccatgctgcaatatggaaagagagggagtttataacctctcaggggacacccattaagtaccacaaggaaatcatgaaattactgcacgcagtgcagaaacccaagaaggcggcagtcttacactgccggggtcatcaaaaagatgaaggagaagcagcagaaggaaactgccgaggagatgctgaggccaaaactgctgctaagcaggacttccctttagaagtgcccatggaaggacccttagtatggagcaaccccctccaggaggttaagccccagtattccccaagcgaaacagaatggggactctcatgggggcatagttttctcccctcagggtggttagcgacagaagagggaaaggtgctcatacctgaagccagccagtggaaaatacttaagaccctccaacaaacctttcatacaggttttgaaagtacccgtaagatggccaaatccctatttacagggccaaaccttctccaaactatgcggcaggtagtcaaggcctgggagatgtgccaaagaaataatcccttggtccatcataaggcccctctgggggaacaaagaatagggcactatcctgtagaggactggcagttaaacttcacccacatgcctaagtcaagaggatttcaatacttgttggtctatgttgatacctttacaaagtgggtggaagccttcccctgcacaacagagaaggcccaagaagtagttaaaatcttacttcatgaaataattcctatattcggacttcccccaaagcttacagagcaacaatggtccagcttttaaagctacaataactcaaggaatttccaaggcactaggaatacaatatcaccttcactgtgcctggagaccacaatcctcagggaaagtcgaaaaggcaaatgaaacactaaagaggcatttgagaaagtatctcccatggccactctcttgcccatggccttgttaagaatccgaaattcccctggaaatttgatccaaaatcaaagggggctcagtccatatgaaatgctgtatggatggccttttctcacaaatgacctcctgctcaatcaggaaacggccaatttggtcaaagatataataacttctctagcaaagtatcaacaaaaccttaaaactttacccaaagggtatgacaggagaaaagggatagagctgttccaaccagaagatctagtagtggtcaagtccctcccctctaccttcccatctatggatcccttgtgggagggaccatactcagtaatcctctctatccccactgaggttaaggtggcaggagtggaatcctggattcaccacacccgagttaaaccttggacaccccttgaggaacttacaggactatcagctcaggagtctgaagatcagccagaccagccttgatacacctgtgacccacttgaggccctgcttctcctatttcggaaggaagcatcccaggctaaaaagactcctgcagttaatcctaaagaagaaaaactcatctctacctaatagaggataagcagaaagcctacatggatctttgacatctctccttgctctctttaatggagtccttatactgtttcatcatattaaacagtatactaaccataccctttgcagtaggattatatactgtagctcctgccaggacaaaaatcctgaccacatcaaccttttttctatcgtccttccttttaacaatttactccttcttccctcctcctttctactaccgctccacctacagagcaccatgactccctttataaggatctcctaagcttcttttaactctcctaagtattctttctgccacctcttcatccctccccaactgcacttgcttctctagtgcatactctcctccccttcccagaaacactgatgtagtctacttcgaaaggatattgtttaaaactaaatcagggtttactacccacacctatatgagaaaggaatgttatagtgctgcttctctctgctcccacaatggccatacatatcaccaaggacaaatgacccagtccaactgtcccgatgccctagggactacccaatgttggacatattacacccatgtgggtataactgatgagagaggtgtccaggataaagccaaaaacaacatgtccaacaagtaattaaaaacttgatccaaccatctaacactccaagtccatataagaaactagacctttccgggttacaaaagactcttgactctcattcccatctctagagtctatttaacaccacattcacaggaatgcaggaggcctctcctaacaatccaactaactactggatgtgtcttcccttgcgtttccaaccacatgtcccagtagtccctgtcccaggacattggaacctatccacctcagtcctaaacaccaccgggataattggctccccagtcaccaatctgccagccacacaggcctcaaatctcacatgtataaattttagcatgactcccaatagaaacatctcccaaagtcaatcctggataccagtgacctcaggtttcacctgtctaactccagacatctttttcatccgtgctaacatagcttattgatgtctaaagggcaccccaaaagagttatgctttctctcatttctagcacccccatgtccatttataccgaacaagagttggaaagtctccttataccccagtcccgccacgcccgagcgcctattctcccttttatggtaggagccagaatactgggtgggcttgggacaggaattggaggtataacctccttcacccaattctattataaaatatcacaagaattaaatgatgatatggaatgggttgccaattccctgatgaccctacaaagccagcttaattctctgactggggtggccctccaaaaacgaagggccctagacttactaacagctaaaagaagaagaacctgcctcttcttaggagaagaatgttgctactttgtcaaccagtcaggaattattgccgaaaaagtccaggagctaagggaatgaagagaacgtagaaagagtgaactccaactctcaggaccctggagtatatttaaccaatgagtaccttggcttctcccctttctaggccctgtaacagccatcttgctatcactcgccttcggtccctgtatttttaacctccttgtcaaatttatttcctctaggataaaggccatcaagctacaaatggccttacaaatggaacctcaaatgaatttaactcaagcttctaccgaggaccccaggatcagcccactggtctcttaactggcctagaaagttcccctctggaggacaatacaacagcagggccccatcgtcgcccctaaccagcaggaagtagctagagcagtcatcgcccagttcccaacagcagttggggtgtcctgtttagaggggggactgagaggtgatgccagctgagcttcctgggttgagtaggggcttggaaagctgtaaaactcactcatttcctgcatcaggacttacttcagttctggataaataatactgaggatatatgcttaaaatattcctaacaccaggatttgcttatatgttttcttcccaagaaagctataaacagcgagaattttagctgtaagttttcctgtatgccccactcctcccctgccaaaaccagagttaaagaaaagattaactgcccatttttctgtgatcagcggaccttatctatcctcccaattccttatgaacatagttcgttaagttctataagatcctctttttcttgctgtacagctccaaggccacaaaacgagtaagcataagtcgcaatttcagattttctcaaaatctaaggcatgtcacaaaataatttactgcctttgtttcttgctcctgtaacattcttcccgcctcacgtatctcccgccttaaagagtttaaaaggcaatcacccaagctagcagtggcaacccatttgggaccccttccacactgtagaagctttgtactttcactctgctcaataaaacctacagctcactctctctctcagtccaagtctctgtcactcgccgcagtcagcctccacaccaattctttggcgtggctaggcacagaaccttgggtgttacaaaaggata